European Patent Application EP 4 509 606 A1, published February 19, 2025. Title: Nucleic Acid Construct for Treating Hereditary Coagulation Factor Deficiency and Use Thereof. Applicant: KANGLIN BIOTECHNOLOGY (HANGZHOU) CO., LTD. The sequence listing filed with the application follows.

SEQUENCE LISTING (37 sequences)

SEQ ID NO: 1 - DNA, 3985 bp, synthetic construct
  source 1..3985: mol_type = other DNA
acatgtgagcaaaaggccagcaaaaggccaggaaccgtaaaaaggccgcgttgctggcgtttttccataggctccgcccccctgacgagcatcacaaaaatcgacgctcaagtcagaggtggcgaaacccgacaggactataaagataccaggcgtttccccctggaagctccctcgtgcgctctcctgttccgaccctgccgcttaccggatacctgtccgcctttctcccttcgggaagcgtggcgctttctcatagctcacgctgtaggtatctcagttcggtgtaggtcgttcgctccaagctgggctgtgtgcacgaaccccccgttcagcccgaccgctgcgccttatccggtaactatcgtcttgagtccaacccggtaagacacgacttatcgccactggcagcagccactggtaacaggattagcagagcgaggtatgtaggcggtgctacagagttcttgaagtggtggcctaactacggctacactagaaggacagtatttggtatctgcgctctgctgaagccagttaccttcggaaaaagagttggtagctcttgatccggcaaacaaaccaccgctggtagcggtggtttttttgtttgcaagcagcagattacgcgcagaaaaaaaggatctcaagaagatcctttgatcttttctacggggtctgacgctcagtggaacgaaaactcacgttaagggattttggtcatgagattatcaaaaaggatcttcacctagatccttttaaattaaaaatgaagttttaaatcaatctaaagtatatatgagtaaacttggtctgacagttaccaatgcttaatcagtgaggcacctatctcagcgatctgtctatttcgttcatccatagttgcctgactccccgtcgtgtagataactacgatacgggagggcttaccatctggccccagtgctgcaatgataccgcgagacccacgctcaccggctccagatttatcagcaataaaccagccagccggaagggccgagcgcagaagtggtcctgcaactttatccgcctccatccagtctattaattgttgccgggaagctagagtaagtagttcgccagttaatagtttgcgcaacgttgttgccattgctacaggcatcgtggtgtcacgctcgtcgtttggtatggcttcattcagctccggttcccaacgatcaaggcgagttacatgatcccccatgttgtgcaaaaaagcggttagctccttcggtcctccgatcgttgtcagaagtaagttggccgcagtgttatcactcatggttatggcagcactgcataattctcttactgtcatgccatccgtaagatgcttttctgtgactggtgagtactcaaccaagtcattctgagaatagtgtatgcggcgaccgagttgctcttgcccggcgtcaatacgggataataccgcgccacatagcagaactttaaaagtgctcatcattggaaaacgttcttcggggcgaaaactctcaaggatcttaccgctgttgagatccagttcgatgtaacccactcgtgcacccaactgatcttcagcatcttttactttcaccagcgtttctgggtgagcaaaaacaggaaggcaaaatgccgcaaaaaagggaataagggcgacacggaaatgttgaatactcatactcttcctttttcaatattattgaagcatttatcagggttattgtctcatgagcggatacatatttgaatgtatttagaaaaataaacaaataggggttccgcgcacatttccccgaaaagtgccacctgacgtctaagaaaccattattatcatgacattaacctataaaaataggcgtatcacgaggccctttcgtctcgcgcgtttcggtgatgacggtgaaaacctctgacacatgcagctcccggagacggtcacagcttgtctgtaagcggatgccgggagcagacaagcccgtcagggcgcgtcagcgggtgttggcgggtgtcggggctggcttaactatgcggcatcagagcagattgtactgagagtgcaccataaaattgtaaacgttaatattttgttaaaattcgcgttaaatttttgttaaatcagctcattttttaaccaataggccgaaatcggcaaaatcccttataaatcaaaagaatagcccgagatagggttgagtgttgttccagtttggaacaagagtccactattaaagaacgtggactccaacgtcaaagggcgaaaaaccgtctatcagggcgatggcccactacgtgaaccatcacccaaatcaagttttttggggtcgaggtgccgtaaagcactaaatcggaaccctaaagggagcccccgatttagagcttgacggggaaagccggcgaacgtggcgagaaaggaagggaagaaagcgaaaggagcgggcgctagggcgctggcaagtgtagcggtcacgctgcgcgtaaccaccacacccgccgcgcttaatgcgccgctacagggcgcgtactatggttgctttgacgtatgcggtgtgaaataccgcacagatgcgtaaggagaaaataccgcatcaggcgcccctgcaggcagctgcgcgctcgctcgctcactgaggccgcccgggcgtcgggcgacctttggtcgcccggcctcagtgagcgagcgagcgcgcagagagggagtggccaactccatcactaggggttcctacgcgtccattgacgtcaataatgacgtatgttcccatagtaacgccaatagggactttccattgacgtcaatgggtggagtatttacggtaaactgcccacttggcagtacatcaagtgtatcatatgccaagtacgccccctattgacgtcaatgacggtaaatggcccgcctggcattatgcccagtacatgaccttatgggactttcctacttggcagtacatctacgtattagtcatcgctattaccatggtcgaggtgagccccacgttctgcttcactctccccatctcccccccctccccacccccaattttgtatttatttattttttaattattttgtgcagcgatgggggcggggggggggggggggcgcgcgccaggcggggcggggcggggcgaggggcggggcggggcgaggcggagaggtgcggcggcagccaatcagagcggcgcgctccgaaagtttccttttatggcgaggcggcggcggcggcggccctataaaaagcgaagcgcgcggcgggcgggagtcgctgcgcgctgccttcgccccgtgccccgctccgccgccgcctcgcgccgcccgccccggctctgactgaccgcgttactcccacaggtgagcgggcgggacggcccttctcctccgggctgtaattagcgcttggtttaatgacggcttgtttcttttctgtggctgcgtgaaagccttgaggggctccgggagggccctttgtgcggggggagcggctcggggctgtccgcggggggacggctgccttcgggggggacggggcagggcggggttcggcttctggcgtgtgaccggcggctctagagcctctgctaaccatgttcatgccttcttctttttcctacagctcctgggcaacgtctcctgggcaacgtaccggtgtcgacgtttatttgtgaaatttgtgatgctattgctttatttgtaaccatctagctttatttgtgaaatttgtgatgctattgctttatttgtaaccattataagctgcaataaacaagttaacaacaacaattgcattcattttatgtttcaggttcagggggagatgtgggaggttttttaaagtttaaacaggaacccctagtgatggagttggccactccctctctgcgcgctcgctcgctcactgaggccgggcgaccaaaggtcgcccgacgcccgggctttgcccgggcggcctcagtgagcgagcgagcgcgcagctgcctgcagg

SEQ ID NO: 2 - DNA, 141 bp, synthetic construct
  source 1..141: mol_type = other DNA
cctgcaggcagctgcgcgctcgctcgctcactgaggccgcccgggcaaagcccgggcgtcgggcgacctttggtcgcccggcctcagtgagcgagcgagcgcgcagagagggagtggccaactccatcactaggggttcct

SEQ ID NO: 3 - DNA, 5388 bp, synthetic construct
  source 1..5388: mol_type = other DNA
acatgtgagcaaaaggccagcaaaaggccaggaaccgtaaaaaggccgcgttgctggcgtttttccataggctccgcccccctgacgagcatcacaaaaatcgacgctcaagtcagaggtggcgaaacccgacaggactataaagataccaggcgtttccccctggaagctccctcgtgcgctctcctgttccgaccctgccgcttaccggatacctgtccgcctttctcccttcgggaagcgtggcgctttctcatagctcacgctgtaggtatctcagttcggtgtaggtcgttcgctccaagctgggctgtgtgcacgaaccccccgttcagcccgaccgctgcgccttatccggtaactatcgtcttgagtccaacccggtaagacacgacttatcgccactggcagcagccactggtaacaggattagcagagcgaggtatgtaggcggtgctacagagttcttgaagtggtggcctaactacggctacactagaaggacagtatttggtatctgcgctctgctgaagccagttaccttcggaaaaagagttggtagctcttgatccggcaaacaaaccaccgctggtagcggtggtttttttgtttgcaagcagcagattacgcgcagaaaaaaaggatctcaagaagatcctttgatcttttctacggggtctgacgctcagtggaacgaaaactcacgttaagggattttggtcatgagattatcaaaaaggatcttcacctagatccttttaaattaaaaatgaagttttaaatcaatctaaagtatatatgagtaaacttggtctgacagttaccaatgcttaatcagtgaggcacctatctcagcgatctgtctatttcgttcatccatagttgcctgactccccgtcgtgtagataactacgatacgggagggcttaccatctggccccagtgctgcaatgataccgcgagacccacgctcaccggctccagatttatcagcaataaaccagccagccggaagggccgagcgcagaagtggtcctgcaactttatccgcctccatccagtctattaattgttgccgggaagctagagtaagtagttcgccagttaatagtttgcgcaacgttgttgccattgctacaggcatcgtggtgtcacgctcgtcgtttggtatggcttcattcagctccggttcccaacgatcaaggcgagttacatgatcccccatgttgtgcaaaaaagcggttagctccttcggtcctccgatcgttgtcagaagtaagttggccgcagtgttatcactcatggttatggcagcactgcataattctcttactgtcatgccatccgtaagatgcttttctgtgactggtgagtactcaaccaagtcattctgagaatagtgtatgcggcgaccgagttgctcttgcccggcgtcaatacgggataataccgcgccacatagcagaactttaaaagtgctcatcattggaaaacgttcttcggggcgaaaactctcaaggatcttaccgctgttgagatccagttcgatgtaacccactcgtgcacccaactgatcttcagcatcttttactttcaccagcgtttctgggtgagcaaaaacaggaaggcaaaatgccgcaaaaaagggaataagggcgacacggaaatgttgaatactcatactcttcctttttcaatattattgaagcatttatcagggttattgtctcatgagcggatacatatttgaatgtatttagaaaaataaacaaataggggttccgcgcacatttccccgaaaagtgccacctgacgtctaagaaaccattattatcatgacattaacctataaaaataggcgtatcacgaggccctttcgtctcgcgcgtttcggtgatgacggtgaaaacctctgacacatgcagctcccggagacggtcacagcttgtctgtaagcggatgccgggagcagacaagcccgtcagggcgcgtcagcgggtgttggcgggtgtcggggctggcttaactatgcggcatcagagcagattgtactgagagtgcaccataaaattgtaaacgttaatattttgttaaaattcgcgttaaatttttgttaaatcagctcattttttaaccaataggccgaaatcggcaaaatcccttataaatcaaaagaatagcccgagatagggttgagtgttgttccagtttggaacaagagtccactattaaagaacgtggactccaacgtcaaagggcgaaaaaccgtctatcagggcgatggcccactacgtgaaccatcacccaaatcaagttttttggggtcgaggtgccgtaaagcactaaatcggaaccctaaagggagcccccgatttagagcttgacggggaaagccggcgaacgtggcgagaaaggaagggaagaaagcgaaaggagcgggcgctagggcgctggcaagtgtagcggtcacgctgcgcgtaaccaccacacccgccgcgcttaatgcgccgctacagggcgcgtactatggttgctttgacgtatgcggtgtgaaataccgcacagatgcgtaaggagaaaataccgcatcaggcgcccctgcaggcagctgcgcgctcgctcgctcactgaggccgcccgggcaaagcccgggcgtcgggcgacctttggtcgcccggcctcagtgagcgagcgagcgcgcagagagggagtggccaactccatcactaggggttcctacgcgtccattgacgtcaataatgacgtatgttcccatagtaacgccaatagggactttccattgacgtcaatgggtggagtatttacggtaaactgcccacttggcagtacatcaagtgtatcatatgccaagtacgccccctattgacgtcaatgacggtaaatggcccgcctggcattatgcccagtacatgaccttatgggactttcctacttggcagtacatctacgtattagtcatcgctattaccatggtcgaggtgagccccacgttctgcttcactctccccatctcccccccctccccacccccaattttgtatttatttattttttaattattttgtgcagcgatgggggcggggggggggggggggcgcgcgccaggcggggcggggcggggcgaggggcggggcggggcgaggcggagaggtgcggcggcagccaatcagagcggcgcgctccgaaagtttccttttatggcgaggcggcggcggcggcggccctataaaaagcgaagcgcgcggcgggcgggagtcgctgcgcgctgccttcgccccgtgccccgctccgccgccgcctcgcgccgcccgccccggctctgactgaccgcgttactcccacaggtgagcgggcgggacggcccttctcctccgggctgtaattagcgcttggtttaatgacggcttgtttcttttctgtggctgcgtgaaagccttgaggggctccgggagggccctttgtgcggggggagcggctcggggctgtccgcggggggacggctgccttcgggggggacggggcagggcggggttcggcttctggcgtgtgaccggcggctctagagcctctgctaaccatgttcatgccttcttctttttcctacagctcctgggcaacgtctcctgggcaacgtaccggtgccaccatgcagcgggtaaatatgatcatggccgagagtcccggactcatcactatatgcctcttgggttacttgcttagcgcagaatgtacagtgtttctggaccatgagaatgccaacaaaatactgaatcggcccaaaaggtacaacagtggtaagctggaagagtttgtccaagggaatctcgagcgggaatgcatggaagaaaaatgcagcttcgaagaggcaagggaggtatttgagaataccgaacgcactactgagttttggaaacaatacgttgacggagaccaatgtgagtctaatccgtgccttaatggaggttcatgtaaagacgatataaacagttacgaatgttggtgccctttcggctttgagggtaaaaactgtgagttggatgtcacctgcaacataaaaaacggacgatgtgaacaattttgcaagaactctgctgataacaaagtagtgtgttcatgtactgaagggtatcgcttggcggaaaaccaaaagagttgcgaaccagcggttccatttccttgcggcagggtctcagtttcccaaacctctaagttgacaagggccgagacggtgtttccggatgtagactatgtgaatagcacggaggcagagactatactcgacaatattacccaaagcacacagtcatttaatgatttcacccgagtggtaggaggggaagacgctaaaccaggacaattcccttggcaggtggttttgaacggcaaggtagatgctttttgtgggggctcaatcgttaacgagaaatggatagtaacggccgcgcattgtgtagaaacgggtgtgaagatcacagtggtagctggtgaacacaacatcgaagagacggagcacacagaacaaaagaggaatgttatccgcattatccctcatcataactacaatgctgctataaacaagtataatcacgacatagcacttcttgaactggacgaacctcttgtcttgaattcctatgtgacacccatctgtatcgctgataaagaatatacaaacatcttccttaaatttggtagtggttacgtatcaggctggggtcgggtcttccacaaaggcagaagtgcattggtattgcagtatcttagagtacccttggtggatagagcgacttgtcttctgagtacgaaatttaccatttacaataatatgttttgcgctggcttccatgagggtggacgggacagttgccaaggagattcaggcggacctcacgtaacggaagtggagggcacgtcattcctgacgggcattattagctggggtgaagagtgtgcaatgaagggaaagtatgggatctatacgaaggtctccaggtatgtgaattggataaaggagaagaccaagctcacgtgagtcgacgtttatttgtgaaatttgtgatgctattgctttatttgtaaccatctagctttatttgtgaaatttgtgatgctattgctttatttgtaaccattataagctgcaataaacaagttaacaacaacaattgcattcattttatgtttcaggttcagggggagatgtgggaggttttttaaagtttaaacaggaacccctagtgatggagttggccactccctctctgcgcgctcgctcgctcactgaggccgggcgaccaaaggtcgcccgacgcccgggctttgcccgggcggcctcagtgagcgagcgagcgcgcagctgcctgcagg

SEQ ID NO: 4 - DNA, 145 bp, synthetic construct
  source 1..145: mol_type = other DNA
ttggccactccctctctgcgcgctcgctcgctcactgaggccgcccgggcaaagcccgggcgtcgggcgacctttggtcgcccggcctcagtgagcgagcgagcgcgcagagagggagtggccaactccatcactaggggttcct

SEQ ID NO: 5 - DNA, 5397 bp, synthetic construct
  source 1..5397: mol_type = other DNA
acatgtgagcaaaaggccagcaaaaggccaggaaccgtaaaaaggccgcgttgctggcgtttttccataggctccgcccccctgacgagcatcacaaaaatcgacgctcaagtcagaggtggcgaaacccgacaggactataaagataccaggcgtttccccctggaagctccctcgtgcgctctcctgttccgaccctgccgcttaccggatacctgtccgcctttctcccttcgggaagcgtggcgctttctcatagctcacgctgtaggtatctcagttcggtgtaggtcgttcgctccaagctgggctgtgtgcacgaaccccccgttcagcccgaccgctgcgccttatccggtaactatcgtcttgagtccaacccggtaagacacgacttatcgccactggcagcagccactggtaacaggattagcagagcgaggtatgtaggcggtgctacagagttcttgaagtggtggcctaactacggctacactagaaggacagtatttggtatctgcgctctgctgaagccagttaccttcggaaaaagagttggtagctcttgatccggcaaacaaaccaccgctggtagcggtggtttttttgtttgcaagcagcagattacgcgcagaaaaaaaggatctcaagaagatcctttgatcttttctacggggtctgacgctcagtggaacgaaaactcacgttaagggattttggtcatgagattatcaaaaaggatcttcacctagatccttttaaattaaaaatgaagttttaaatcaatctaaagtatatatgagtaaacttggtctgacagttaccaatgcttaatcagtgaggcacctatctcagcgatctgtctatttcgttcatccatagttgcctgactccccgtcgtgtagataactacgatacgggagggcttaccatctggccccagtgctgcaatgataccgcgagacccacgctcaccggctccagatttatcagcaataaaccagccagccggaagggccgagcgcagaagtggtcctgcaactttatccgcctccatccagtctattaattgttgccgggaagctagagtaagtagttcgccagttaatagtttgcgcaacgttgttgccattgctacaggcatcgtggtgtcacgctcgtcgtttggtatggcttcattcagctccggttcccaacgatcaaggcgagttacatgatcccccatgttgtgcaaaaaagcggttagctccttcggtcctccgatcgttgtcagaagtaagttggccgcagtgttatcactcatggttatggcagcactgcataattctcttactgtcatgccatccgtaagatgcttttctgtgactggtgagtactcaaccaagtcattctgagaatagtgtatgcggcgaccgagttgctcttgcccggcgtcaatacgggataataccgcgccacatagcagaactttaaaagtgctcatcattggaaaacgttcttcggggcgaaaactctcaaggatcttaccgctgttgagatccagttcgatgtaacccactcgtgcacccaactgatcttcagcatcttttactttcaccagcgtttctgggtgagcaaaaacaggaaggcaaaatgccgcaaaaaagggaataagggcgacacggaaatgttgaatactcatactcttcctttttcaatattattgaagcatttatcagggttattgtctcatgagcggatacatatttgaatgtatttagaaaaataaacaaataggggttccgcgcacatttccccgaaaagtgccacctgacgtctaagaaaccattattatcatgacattaacctataaaaataggcgtatcacgaggccctttcgtctcgcgcgtttcggtgatgacggtgaaaacctctgacacatgcagctcccggagacggtcacagcttgtctgtaagcggatgccgggagcagacaagcccgtcagggcgcgtcagcgggtgttggcgggtgtcggggctggcttaactatgcggcatcagagcagattgtactgagagtgcaccataaaattgtaaacgttaatattttgttaaaattcgcgttaaatttttgttaaatcagctcattttttaaccaataggccgaaatcggcaaaatcccttataaatcaaaagaatagcccgagatagggttgagtgttgttccagtttggaacaagagtccactattaaagaacgtggactccaacgtcaaagggcgaaaaaccgtctatcagggcgatggcccactacgtgaaccatcacccaaatcaagttttttggggtcgaggtgccgtaaagcactaaatcggaaccctaaagggagcccccgatttagagcttgacggggaaagccggcgaacgtggcgagaaaggaagggaagaaagcgaaaggagcgggcgctagggcgctggcaagtgtagcggtcacgctgcgcgtaaccaccacacccgccgcgcttaatgcgccgctacagggcgcgtactatggttgctttgacgtatgcggtgtgaaataccgcacagatgcgtaaggagaaaataccgcatcaggcgccttggccactccctctctgcgcgctcgctcgctcactgaggccgcccgggcaaagcccgggcgtcgggcgacctttggtcgcccggcctcagtgagcgagcgagcgcgcagagagggagtggccaactccatcactaggggttcctacgcgtccattgacgtcaataatgacgtatgttcccatagtaacgccaatagggactttccattgacgtcaatgggtggagtatttacggtaaactgcccacttggcagtacatcaagtgtatcatatgccaagtacgccccctattgacgtcaatgacggtaaatggcccgcctggcattatgcccagtacatgaccttatgggactttcctacttggcagtacatctacgtattagtcatcgctattaccatggtcgaggtgagccccacgttctgcttcactctccccatctcccccccctccccacccccaattttgtatttatttattttttaattattttgtgcagcgatgggggcggggggggggggggggcgcgcgccaggcggggcggggcggggcgaggggcggggcggggcgaggcggagaggtgcggcggcagccaatcagagcggcgcgctccgaaagtttccttttatggcgaggcggcggcggcggcggccctataaaaagcgaagcgcgcggcgggcgggagtcgctgcgcgctgccttcgccccgtgccccgctccgccgccgcctcgcgccgcccgccccggctctgactgaccgcgttactcccacaggtgagcgggcgggacggcccttctcctccgggctgtaattagcgcttggtttaatgacggcttgtttcttttctgtggctgcgtgaaagccttgaggggctccgggagggccctttgtgcggggggagcggctcggggctgtccgcggggggacggctgccttcgggggggacggggcagggcggggttcggcttctggcgtgtgaccggcggctctagagcctctgctaaccatgttcatgccttcttctttttcctacagctcctgggcaacgtctcctgggcaacgtaccggtcgccaccatgcagcgggtaaatatgatcatggccgagagtcccggactcatcactatatgcctcttgggttacttgcttagcgcagaatgtacagtgtttctggaccatgagaatgccaacaaaatactgaatcggcccaaaaggtacaacagtggtaagctggaagagtttgtccaagggaatctcgagcgggaatgcatggaagaaaaatgcagcttcgaagaggcaagggaggtatttgagaataccgaacgcactactgagttttggaaacaatacgttgacggagaccaatgtgagtctaatccgtgccttaatggaggttcatgtaaagacgatataaacagttacgaatgttggtgccctttcggctttgagggtaaaaactgtgagttggatgtcacctgcaacataaaaaacggacgatgtgaacaattttgcaagaactctgctgataacaaagtagtgtgttcatgtactgaagggtatcgcttggcggaaaaccaaaagagttgcgaaccagcggttccatttccttgcggcagggtctcagtttcccaaacctctaagttgacaagggccgagacggtgtttccggatgtagactatgtgaatagcacggaggcagagactatactcgacaatattacccaaagcacacagtcatttaatgatttcacccgagtggtaggaggggaagacgctaaaccaggacaattcccttggcaggtggttttgaacggcaaggtagatgctttttgtgggggctcaatcgttaacgagaaatggatagtaacggccgcgcattgtgtagaaacgggtgtgaagatcacagtggtagctggtgaacacaacatcgaagagacggagcacacagaacaaaagaggaatgttatccgcattatccctcatcataactacaatgctgctataaacaagtataatcacgacatagcacttcttgaactggacgaacctcttgtcttgaattcctatgtgacacccatctgtatcgctgataaagaatatacaaacatcttccttaaatttggtagtggttacgtatcaggctggggtcgggtcttccacaaaggcagaagtgcattggtattgcagtatcttagagtacccttggtggatagagcgacttgtcttctgagtacgaaatttaccatttacaataatatgttttgcgctggcttccatgagggtggacgggacagttgccaaggagattcaggcggacctcacgtaacggaagtggagggcacgtcattcctgacgggcattattagctggggtgaagagtgtgcaatgaagggaaagtatgggatctatacgaaggtctccaggtatgtgaattggataaaggagaagaccaagctcacgtgagtcgacgtttatttgtgaaatttgtgatgctattgctttatttgtaaccatctagctttatttgtgaaatttgtgatgctattgctttatttgtaaccattataagctgcaataaacaagttaacaacaacaattgcattcattttatgtttcaggttcagggggagatgtgggaggttttttaaagtttaaacaggaacccctagtgatggagttggccactccctctctgcgcgctcgctcgctcactgaggccgggcgaccaaaggtcgcccgacgcccgggctttgcccgggcggcctcagtgagcgagcgagcgcgcagagagggagtggccaa

SEQ ID NO: 6 - DNA, 592 bp, synthetic construct
  source 1..592: mol_type = other DNA
aatcaacctctggattacaaaatttgtgaaagattgactggtattcttaactatgttgctccttttacgctatgtggatacgctgctttaatgcctttgtatcatgctattgcttcccgtatggctttcattttctcctccttgtataaatcctggttgctgtctctttatgaggagttgtggcccgttgtcaggcaacgtggcgtggtgtgcactgtgtttgctgacgcaacccccactggttggggcattgccaccacctgtcagctcctttccgggactttcgctttccccctccctattgccacggcggaactcatcgccgcctgccttgcccgctgctggacaggggctcggctgttgggcactgacaattccgtggtgttgtcggggaagctgacgtcctttccatggctgctcgcctgtgttgccacctggattctgcgcgggacgtccttctgctacgtcccttcggccctcaatccagcggaccttccttcccgcggcctgctgccggctctgcggcctcttccgcgtcttcgccttcgccctcagacgagtcggatctccctttgggccgcctccccgcctg

SEQ ID NO: 7 - DNA, 27 bp, synthetic construct
  source 1..27: mol_type = other DNA
acacccaagctgtctagagccgccacc

SEQ ID NO: 8 - DNA, 5998 bp, synthetic construct
  source 1..5998: mol_type = other DNA
acatgtgagcaaaaggccagcaaaaggccaggaaccgtaaaaaggccgcgttgctggcgtttttccataggctccgcccccctgacgagcatcacaaaaatcgacgctcaagtcagaggtggcgaaacccgacaggactataaagataccaggcgtttccccctggaagctccctcgtgcgctctcctgttccgaccctgccgcttaccggatacctgtccgcctttctcccttcgggaagcgtggcgctttctcatagctcacgctgtaggtatctcagttcggtgtaggtcgttcgctccaagctgggctgtgtgcacgaaccccccgttcagcccgaccgctgcgccttatccggtaactatcgtcttgagtccaacccggtaagacacgacttatcgccactggcagcagccactggtaacaggattagcagagcgaggtatgtaggcggtgctacagagttcttgaagtggtggcctaactacggctacactagaaggacagtatttggtatctgcgctctgctgaagccagttaccttcggaaaaagagttggtagctcttgatccggcaaacaaaccaccgctggtagcggtggtttttttgtttgcaagcagcagattacgcgcagaaaaaaaggatctcaagaagatcctttgatcttttctacggggtctgacgctcagtggaacgaaaactcacgttaagggattttggtcatgagattatcaaaaaggatcttcacctagatccttttaaattaaaaatgaagttttaaatcaatctaaagtatatatgagtaaacttggtctgacagttaccaatgcttaatcagtgaggcacctatctcagcgatctgtctatttcgttcatccatagttgcctgactccccgtcgtgtagataactacgatacgggagggcttaccatctggccccagtgctgcaatgataccgcgagacccacgctcaccggctccagatttatcagcaataaaccagccagccggaagggccgagcgcagaagtggtcctgcaactttatccgcctccatccagtctattaattgttgccgggaagctagagtaagtagttcgccagttaatagtttgcgcaacgttgttgccattgctacaggcatcgtggtgtcacgctcgtcgtttggtatggcttcattcagctccggttcccaacgatcaaggcgagttacatgatcccccatgttgtgcaaaaaagcggttagctccttcggtcctccgatcgttgtcagaagtaagttggccgcagtgttatcactcatggttatggcagcactgcataattctcttactgtcatgccatccgtaagatgcttttctgtgactggtgagtactcaaccaagtcattctgagaatagtgtatgcggcgaccgagttgctcttgcccggcgtcaatacgggataataccgcgccacatagcagaactttaaaagtgctcatcattggaaaacgttcttcggggcgaaaactctcaaggatcttaccgctgttgagatccagttcgatgtaacccactcgtgcacccaactgatcttcagcatcttttactttcaccagcgtttctgggtgagcaaaaacaggaaggcaaaatgccgcaaaaaagggaataagggcgacacggaaatgttgaatactcatactcttcctttttcaatattattgaagcatttatcagggttattgtctcatgagcggatacatatttgaatgtatttagaaaaataaacaaataggggttccgcgcacatttccccgaaaagtgccacctgacgtctaagaaaccattattatcatgacattaacctataaaaataggcgtatcacgaggccctttcgtctcgcgcgtttcggtgatgacggtgaaaacctctgacacatgcagctcccggagacggtcacagcttgtctgtaagcggatgccgggagcagacaagcccgtcagggcgcgtcagcgggtgttggcgggtgtcggggctggcttaactatgcggcatcagagcagattgtactgagagtgcaccataaaattgtaaacgttaatattttgttaaaattcgcgttaaatttttgttaaatcagctcattttttaaccaataggccgaaatcggcaaaatcccttataaatcaaaagaatagcccgagatagggttgagtgttgttccagtttggaacaagagtccactattaaagaacgtggactccaacgtcaaagggcgaaaaaccgtctatcagggcgatggcccactacgtgaaccatcacccaaatcaagttttttggggtcgaggtgccgtaaagcactaaatcggaaccctaaagggagcccccgatttagagcttgacggggaaagccggcgaacgtggcgagaaaggaagggaagaaagcgaaaggagcgggcgctagggcgctggcaagtgtagcggtcacgctgcgcgtaaccaccacacccgccgcgcttaatgcgccgctacagggcgcgtactatggttgctttgacgtatgcggtgtgaaataccgcacagatgcgtaaggagaaaataccgcatcaggcgcccctgcaggcagctgcgcgctcgctcgctcactgaggccgcccgggcaaagcccgggcgtcgggcgacctttggtcgcccggcctcagtgagcgagcgagcgcgcagagagggagtggccaactccatcactaggggttcctacgcgtccattgacgtcaataatgacgtatgttcccatagtaacgccaatagggactttccattgacgtcaatgggtggagtatttacggtaaactgcccacttggcagtacatcaagtgtatcatatgccaagtacgccccctattgacgtcaatgacggtaaatggcccgcctggcattatgcccagtacatgaccttatgggactttcctacttggcagtacatctacgtattagtcatcgctattaccatggtcgaggtgagccccacgttctgcttcactctccccatctcccccccctccccacccccaattttgtatttatttattttttaattattttgtgcagcgatgggggcgggggggggggggggcgcgcgccaggcggggcggggcggggcgaggggcggggcggggcgaggcggagaggtgcggcggcagccaatcagagcggcgcgctccgaaagtttccttttatggcgaggcggcggcggcggcggccctataaaaagcgaagcgcgcggcgggcgggagtcgctgcgcgctgccttcgccccgtgccccgctccgccgccgcctcgcgccgcccgccccggctctgactgaccgcgttactcccacaggtgagcgggcgggacggcccttctcctccgggctgtaattagcgcttggtttaatgacggcttgtttcttttctgtggctgcgtgaaagccttgaggggctccgggagggccctttgtgcggggggagcggctcggggctgtccgcggggggacggctgccttcgggggggacggggcagggcggggttcggcttctggcgtgtgaccggcggctctagagcctctgctaaccatgttcatgccttcttctttttcctacagctcctgggcaacgtacacccaagctgtctagagccgccaccaccggtgccaccatgcagcgggtaaatatgatcatggccgagagtcccggactcatcactatatgcctcttgggttacttgcttagcgcagaatgtacagtgtttctggaccatgagaatgccaacaaaatactgaatcggcccaaaaggtacaacagtggtaagctggaagagtttgtccaagggaatctcgagcgggaatgcatggaagaaaaatgcagcttcgaagaggcaagggaggtatttgagaataccgaacgcactactgagttttggaaacaatacgttgacggagaccaatgtgagtctaatccgtgccttaatggaggttcatgtaaagacgatataaacagttacgaatgttggtgccctttcggctttgagggtaaaaactgtgagttggatgtcacctgcaacataaaaaacggacgatgtgaacaattttgcaagaactctgctgataacaaagtagtgtgttcatgtactgaagggtatcgcttggcggaaaaccaaaagagttgcgaaccagcggttccatttccttgcggcagggtctcagtttcccaaacctctaagttgacaagggccgagacggtgtttccggatgtagactatgtgaatagcacggaggcagagactatactcgacaatattacccaaagcacacagtcatttaatgatttcacccgagtggtaggaggggaagacgctaaaccaggacaattcccttggcaggtggttttgaacggcaaggtagatgctttttgtgggggctcaatcgttaacgagaaatggatagtaacggccgcgcattgtgtagaaacgggtgtgaagatcacagtggtagctggtgaacacaacatcgaagagacggagcacacagaacaaaagaggaatgttatccgcattatccctcatcataactacaatgctgctataaacaagtataatcacgacatagcacttcttgaactggacgaacctcttgtcttgaattcctatgtgacacccatctgtatcgctgataaagaatatacaaacatcttccttaaatttggtagtggttacgtatcaggctggggtcgggtcttccacaaaggcagaagtgcattggtattgcagtatcttagagtacccttggtggatagagcgacttgtcttctgagtacgaaatttaccatttacaataatatgttttgcgctggcttccatgagggtggacgggacagttgccaaggagattcaggcggacctcacgtaacggaagtggagggcacgtcattcctgacgggcattattagctggggtgaagagtgtgcaatgaagggaaagtatgggatctatacgaaggtctccaggtatgtgaattggataaaggagaagaccaagctcacgtaggtcgacaatcaacctctggattacaaaatttgtgaaagattgactggtattcttaactatgttgctccttttacgctatgtggatacgctgctttaatgcctttgtatcatgctattgcttcccgtatggctttcattttctcctccttgtataaatcctggttgctgtctctttatgaggagttgtggcccgttgtcaggcaacgtggcgtggtgtgcactgtgtttgctgacgcaacccccactggttggggcattgccaccacctgtcagctcctttccgggactttcgctttccccctccctattgccacggcggaactcatcgccgcctgccttgcccgctgctggacaggggctcggctgttgggcactgacaattccgtggtgttgtcggggaagctgacgtcctttccatggctgctcgcctgtgttgccacctggattctgcgcgggacgtccttctgctacgtcccttcggccctcaatccagcggaccttccttcccgcggcctgctgccggctctgcggcctcttccgcgtcttcgccttcgccctcagacgagtcggatctccctttgggccgcctccccgcctggtcgacgtttatttgtgaaatttgtgatgctattgctttatttgtaaccatctagctttatttgtgaaatttgtgatgctattgctttatttgtaaccattataagctgcaataaacaagttaacaacaacaattgcattcattttatgtttcaggttcagggggagatgtgggaggttttttaaagtttaaacaggaacccctagtgatggagttggccactccctctctgcgcgctcgctcgctcactgaggccgggcgaccaaaggtcgcccgacgcccgggctttgcccgggcggcctcagtgagcgagcgagcgcgcagctgcctgcagg

SEQ ID NO: 9 - DNA, 7330 bp, synthetic construct
  source 1..7330: mol_type = other DNA
atgccggggttttacgagattgtgattaaggtccccagcgaccttgacgagcatctgcccggcatttctgacagctttgtgaactgggtggccgagaaggaatgggagttgccgccagattctgacatggatctgaatctgattgagcaggcacccctgaccgtggccgagaagctgcagcgcgactttctgacggaatggcgccgtgtgagtaaggccccggaggcccttttctttgtgcaatttgagaagggagagagctacttccacatgcacgtgctcgtggaaaccaccggggtgaaatccatggttttgggacgtttcctgagtcagattcgcgaaaaactgattcagagaatttaccgcgggatcgagccgactttgccaaactggttcgcggtcacaaagaccagaaatggcgccggaggcgggaacaaggtggtggatgagtgctacatccccaattacttgctccccaaaacccagcctgagctccagtgggcgtggactaatatggaacagtatttaagcgcctgtttgaatctcacggagcgtaaacggttggtggcgcagcatctgacgcacgtgtcgcagacgcaggagcagaacaaagagaatcagaatcccaattctgatgcgccggtgatcagatcaaaaacttcagccaggtacatggagctggtcgggtggctcgtggacaaggggattacctcggagaagcagtggatccaggaggaccaggcctcatacatctccttcaatgcggcctccaactcgcggtcccaaatcaaggctgccttggacaatgcgggaaagattatgagcctgactaaaaccgcccccgactacctggtgggccagcagcccgtggaggacatttccagcaatcggatttataaaattttggaactaaacgggtacgatccccaatatgcggcttccgtctttctgggatgggccacgaaaaagttcggcaagaggaacaccatctggctgtttgggcctgcaactaccgggaagaccaacatcgcggaggccatagcccacactgtgcccttctacgggtgcgtaaactggaccaatgagaactttcccttcaacgactgtgtcgacaagatggtgatctggtgggaggaggggaagatgaccgccaaggtcgtggagtcggccaaagccattctcggaggaagcaaggtgcgcgtggaccagaaatgcaagtcctcggcccagatagacccgactcccgtgatcgtcacctccaacaccaacatgtgcgccgtgattgacgggaactcaacgaccttcgaacaccagcagccgttgcaagaccggatgttcaaatttgaactcacccgccgtctggatcatgactttgggaaggtcaccaagcaggaagtcaaagactttttccggtgggcaaaggatcacgtggttgaggtggagcatgaattctacgtcaaaaagggtggagccaagaaaagacccgcccccagtgacgcagatataagtgagcccaaacgggtgcgcgagtcagttgcgcagccatcgacgtcagacgcggaagcttcgatcaactacgcagacaggtaccaaaacaaatgttctcgtcacgtgggcatgaatctgatgctgtttccctgcagacaatgcgagagaatgaatcagaattcaaatatctgcttcactcacggacagaaagactgtttagagtgctttcccgtgtcagaatctcaacccgtttctgtcgtcaaaaaggcgtatcagaaactgtgctacattcatcatatcatgggaaaggtgccagacgcttgcactgcctgcgatctggtcaatgtggatttggatgactgcatctttgaacaataaatgatttaaatcaggtatggctgccgatggttatcttccagattggctcgaggacaacctctctgagggcattcgcgagtggtgggacttgaaacctggagccccgaaacccaaagccaaccagcaaaagcaggacgacggccggggtctggtgcttcctggctacaagtacctcggacccttcaacggactcgacaagggggagcccgtcaacgcggcggatgcagcggccctcgagcacgacaaggcctacgaccagcagctcaaagcgggtgacaatccgtacctgcggtataaccacgccgacgccgagtttcaggagcgtctgcaagaagatacgtcttttgggggcaacctcgggcgagcagtcttccaggccaagaagagggttctcgaacctcttggtctggttgaggaaggtgctaagacggctcctggaaagaaacgtccggtagagcagtcgccacaagagccagactcctcctcgggcattggcaagacaggccagcagcccgctaaaaagagactcaattttggtcagactggcgactcagagtcagtccccgacccacaacctctcggagaacctccagcaacccccgctgctgtgggacctactacaatggcttcaggcggtggcgcaccaatggcagacaataacgaaggcgccgacggagtgggtaatgcctcaggaaattggcattgcgattccacatggctgggcgacagagtcatcaccaccagcacccgaacatgggccttgcccacctataacaaccacctctacaagcaaatctccagtgcttcaacgggggccagcaacgacaaccactacttcggctacagcaccccctgggggtattttgatttcaacagattccactgccatttctcaccacgtgactggcagcgactcatcaacaacaattggggattccggcccaagagactcaacttcaagctcttcaacatccaagtcaaggaggtcacgacgaatgatggcgtcacgaccatcgctaataaccttaccagcacggttcaagtcttctcggactcggagtaccagttgccgtacgtcctcggctctgcgcaccagggctgcctccctccgttcccggcggacgtgttcatgattccgcagtacggctacctaacgctcaacaatggcagccaggcagtgggacggtcatccttttactgcctggaatatttcccatcgcagatgctgagaacgggcaataactttaccttcagctacaccttcgaggacgtgcctttccacagcagctacgcgcacagccagagcctggaccggctgatgaatcctctcatcgaccagtacctgtatttcctgaacagaactcagaatcagtccggaagtgcccaaaacaaggacttgctgtttagccgggggtctccagctggcatgtctgttcagcccaaaaactggctacctggaccctgttaccggcagcagcgcgtttctaaaacaaaaacagacaacaacaacagcaactttacctggactggtgcttcaaaatataaccttaatgggcgtgaatctataatcaaccctggcactgctatggcctcacacaaagacgacaaagacaagttctttcccatgagcggtgtcatgatttttggaaaggagagcgccggagcttcaaacactgcattggacaatgtcatgatcacagacgaagaggaaatcaaagccactaaccccgtggccaccgaaagatttgggactgtggcagtcaatctccagagcagcagcacagaccctgcgaccggagatgtgcatgttatgggagccttacctggaatggtgtggcaagacagagacgtatacctgcagggtcctatttgggccaaaattcctcacacggatggacactttcacccgtctcctctcatgggcggctttggacttaagcacccgcctcctcagatcctcatcaaaaacacgcctgttcctgcgaatcctccggcagagttttcggctacaaagtttgcttcattcatcacccagtattccacaggacaagtgagcgtggagattgaatgggagctgcagaaagaaaacagcaaacgctggaatcccgaagtgcagtatacatctaactatgcaaaatctgccaacgttgatttcactgtggacaacaatggactttatactgagcctcgccccattggcacccgtttcctcacccgtcccctgtaattgtctgttaatcaataaaccggttgattcgtttcagttgaactttggtctctgcgaagggcgaattcgtttaaacctgcaggactagaggtcctgtattagaggtcacgtgagtgttttgcgacattttgcgacaccatgtggtcacgctgggtatttaagcccgagtgagcacgcagggtctccattttgaagcgggaggtttgaacgcgcagccgccaagccgaattctgcagatatccatcacactggcggccgctcgactagagcggccgccaccgcggtggagctccagcttttgttccctttagtgagggttaattgcgcgcttggcgtaatcatggtcatagctgtttcctgtgtgaaattgttatccgctcacaattccacacaacatacgagccggaagcataaagtgtaaagcctggggtgcctaatgagtgagctaactcacattaattgcgttgcgctcactgcccgctttccagtcgggaaacctgtcgtgccagctgcattaatgaatcggccaacgcgcggggagaggcggtttgcgtattgggcgctcttccgcttcctcgctcactgactcgctgcgctcggtcgttcggctgcggcgagcggtatcagctcactcaaaggcggtaatacggttatccacagaatcaggggataacgcaggaaagaacatgtgagcaaaaggccagcaaaaggccaggaaccgtaaaaaggccgcgttgctggcgtttttccataggctccgcccccctgacgagcatcacaaaaatcgacgctcaagtcagaggtggcgaaacccgacaggactataaagataccaggcgtttccccctggaagctccctcgtgcgctctcctgttccgaccctgccgcttaccggatacctgtccgcctttctcccttcgggaagcgtggcgctttctcatagctcacgctgtaggtatctcagttcggtgtaggtcgttcgctccaagctgggctgtgtgcacgaaccccccgttcagcccgaccgctgcgccttatccggtaactatcgtcttgagtccaacccggtaagacacgacttatcgccactggcagcagccactggtaacaggattagcagagcgaggtatgtaggcggtgctacagagttcttgaagtggtggcctaactacggctacactagaagaacagtatttggtatctgcgctctgctgaagccagttaccttcggaaaaagagttggtagctcttgatccggcaaacaaaccaccgctggtagcggtggtttttttgtttgcaagcagcagattacgcgcagaaaaaaaggatctcaagaagatcctttgatcttttctacggggtctgacgctcagtggaacgaaaactcacgttaagggattttggtcatgagattatcaaaaaggatcttcacctagatccttttaaattaaaaatgaagttttaaatcaatctaaagtatatatgagtaaacttggtctgacagttaccaatgcttaatcagtgaggcacctatctcagcgatctgtctatttcgttcatccatagttgcctgactccccgtcgtgtagataactacgatacgggagggcttaccatctggccccagtgctgcaatgataccgcgagacccacgctcaccggctccagatttatcagcaataaaccagccagccggaagggccgagcgcagaagtggtcctgcaactttatccgcctccatccagtctattaattgttgccgggaagctagagtaagtagttcgccagttaatagtttgcgcaacgttgttgccattgctacaggcatcgtggtgtcacgctcgtcgtttggtatggcttcattcagctccggttcccaacgatcaaggcgagttacatgatcccccatgttgtgcaaaaaagcggttagctccttcggtcctccgatcgttgtcagaagtaagttggccgcagtgttatcactcatggttatggcagcactgcataattctcttactgtcatgccatccgtaagatgcttttctgtgactggtgagtactcaaccaagtcattctgagaatagtgtatgcggcgaccgagttgctcttgcccggcgtcaatacgggataataccgcgccacatagcagaactttaaaagtgctcatcattggaaaacgttcttcggggcgaaaactctcaaggatcttaccgctgttgagatccagttcgatgtaacccactcgtgcacccaactgatcttcagcatcttttactttcaccagcgtttctgggtgagcaaaaacaggaaggcaaaatgccgcaaaaaagggaataagggcgacacggaaatgttgaatactcatactcttcctttttcaatattattgaagcatttatcagggttattgtctcatgagcggatacatatttgaatgtatttagaaaaataaacaaataggggttccgcgcacatttccccgaaaagtgccacctaaattgtaagcgttaatattttgttaaaattcgcgttaaatttttgttaaatcagctcattttttaaccaataggccgaaatcggcaaaatcccttataaatcaaaagaatagaccgagatagggttgagtgttgttccagtttggaacaagagtccactattaaagaacgtggactccaacgtcaaagggcgaaaaaccgtctatcagggcgatggcccactacgtgaaccatcaccctaatcaagttttttggggtcgaggtgccgtaaagcactaaatcggaaccctaaagggagcccccgatttagagcttgacggggaaagccggcgaacgtggcgagaaaggaagggaagaaagcgaaaggagcgggcgctagggcgctggcaagtgtagcggtcacgctgcgcgtaaccaccacacccgccgcgcttaatgcgccgctacagggcgcgtcccattcgccattcaggctgcgcaactgttgggaagggcgatcggtgcgggcctcttcgctattacgccagctggcgaaagggggatgtgctgcaaggcgattaagttgggtaacgccagggttttcccagtcacgacgttgtaaaacgacggccagtgagcgcgcgtaatacgactcactatagggcgaattgggtaccgggccccccctcgatcgaggtcgacggtatcgggggagctcgcagggtctccattttgaagcgggaggtttgaacgcgcagccgcc

SEQ ID NO: 10 - DNA, 11635 bp, synthetic construct
  source 1..11635: mol_type = other DNA
ggtacccaactccatgcttaacagtccccaggtacagcccaccctgcgtcgcaaccaggaacagctctacagcttcctggagcgccactcgccctacttccgcagccacagtgcgcagattaggagcgccacttctttttgtcacttgaaaaacatgtaaaaataatgtactaggagacactttcaataaaggcaaatgtttttatttgtacactctcgggtgattatttaccccccacccttgccgtctgcgccgtttaaaaatcaaaggggttctgccgcgcatcgctatgcgccactggcagggacacgttgcgatactggtgtttagtgctccacttaaactcaggcacaaccatccgcggcagctcggtgaagttttcactccacaggctgcgcaccatcaccaacgcgtttagcaggtcgggcgccgatatcttgaagtcgcagttggggcctccgccctgcgcgcgcgagttgcgatacacagggttgcagcactggaacactatcagcgccgggtggtgcacgctggccagcacgctcttgtcggagatcagatccgcgtccaggtcctccgcgttgctcagggcgaacggagtcaactttggtagctgccttcccaaaaagggtgcatgcccaggctttgagttgcactcgcaccgtagtggcatcagaaggtgaccgtgcccggtctgggcgttaggatacagcgcctgcatgaaagccttgatctgcttaaaagccacctgagcctttgcgccttcagagaagaacatgccgcaagacttgccggaaaactgattggccggacaggccgcgtcatgcacgcagcaccttgcgtcggtgttggagatctgcaccacatttcggccccaccggttcttcacgatcttggccttgctagactgctccttcagcgcgcgctgcccgttttcgctcgtcacatccatttcaatcacgtgctccttatttatcataatgctcccgtgtagacacttaagctcgccttcgatctcagcgcagcggtgcagccacaacgcgcagcccgtgggctcgtggtgcttgtaggttacctctgcaaacgactgcaggtacgcctgcaggaatcgccccatcatcgtcacaaaggtcttgttgctggtgaaggtcagctgcaacccgcggtgctcctcgtttagccaggtcttgcatacggccgccagagcttccacttggtcaggcagtagcttgaagtttgcctttagatcgttatccacgtggtacttgtccatcaacgcgcgcgcagcctccatgcccttctcccacgcagacacgatcggcaggctcagcgggtttatcaccgtgctttcactttccgcttcactggactcttccttttcctcttgcgtccgcataccccgcgccactgggtcgtcttcattcagccgccgcaccgtgcgcttacctcccttgccgtgcttgattagcaccggtgggttgctgaaacccaccatttgtagcgccacatcttctctttcttcctcgctgtccacgatcacctctggggatggcgggcgctcgggcttgggagaggggcgcttctttttctttttggacgcaatggccaaatccgccgtcgaggtcgatggccgcgggctgggtgtgcgcggcaccagcgcatcttgtgacgagtcttcttcgtcctcggactcgagacgccgcctcagccgcttttttgggggcgcgcggggaggcggcggcgacggcgacggggacgacacgtcctccatggttggtggacgtcgcgccgcaccgcgtccgcgctcgggggtggtttcgcgctgctcctcttcccgactggccatttccttctcctataggcagaaaaagatcatggagtcagtcgagaaggaggacagcctaaccgccccctttgagttcgccaccaccgcctccaccgatgccgccaacgcgcctaccaccttccccgtcgaggcacccccgcttgaggaggaggaagtgattatcgagcaggacccaggttttgtaagcgaagacgacgaggatcgctcagtaccaacagaggataaaaagcaagaccaggacgacgcagaggcaaacgaggaacaagtcgggcggggggaccaaaggcatggcgactacctagatgtgggagacgacgtgctgttgaagcatctgcagcgccagtgcgccattatctgcgacgcgttgcaagagcgcagcgatgtgcccctcgccatagcggatgtcagccttgcctacgaacgccacctgttctcaccgcgcgtaccccccaaacgccaagaaaacggcacatgcgagcccaacccgcgcctcaacttctaccccgtatttgccgtgccagaggtgcttgccacctatcacatctttttccaaaactgcaagatacccctatcctgccgtgccaaccgcagccgagcggacaagcagctggccttgcggcagggcgctgtcatacctgatatcgcctcgctcgacgaagtgccaaaaatctttgagggtcttggacgcgacgagaaacgcgcggcaaacgctctgcaacaagaaaacagcgaaaatgaaagtcactgtggagtgctggtggaacttgagggtgacaacgcgcgcctagccgtgctgaaacgcagcatcgaggtcacccactttgcctacccggcacttaacctaccccccaaggttatgagcacagtcatgagcgagctgatcgtgcgccgtgcacgacccctggagagggatgcaaacttgcaagaacaaaccgaggagggcctacccgcagttggcgatgagcagctggcgcgctggcttgagacgcgcgagcctgccgacttggaggagcgacgcaagctaatgatggccgcagtgcttgttaccgtggagcttgagtgcatgcagcggttctttgctgacccggagatgcagcgcaagctagaggaaacgttgcactacacctttcgccagggctacgtgcgccaggcctgcaaaatttccaacgtggagctctgcaacctggtctcctaccttggaattttgcacgaaaaccgcctcgggcaaaacgtgcttcattccacgctcaagggcgaggcgcgccgcgactacgtccgcgactgcgtttacttatttctgtgctacacctggcaaacggccatgggcgtgtggcagcaatgcctggaggagcgcaacctaaaggagctgcagaagctgctaaagcaaaacttgaaggacctatggacggccttcaacgagcgctccgtggccgcgcacctggcggacattatcttccccgaacgcctgcttaaaaccctgcaacagggtctgccagacttcaccagtcaaagcatgttgcaaaactttaggaactttatcctagagcgttcaggaattctgcccgccacctgctgtgcgcttcctagcgactttgtgcccattaagtaccgtgaatgccctccgccgctttggggtcactgctaccttctgcagctagccaactaccttgcctaccactccgacatcatggaagacgtgagcggtgacggcctactggagtgtcactgtcgctgcaacctatgcaccccgcaccgctccctggtctgcaattcgcaactgcttagcgaaagtcaaattatcggtacctttgagctgcagggtccctcgcctgacgaaaagtccgcggctccggggttgaaactcactccggggctgtggacgtcggcttaccttcgcaaatttgtacctgaggactaccacgcccacgagattaggttctacgaagaccaatcccgcccgccaaatgcggagcttaccgcctgcgtcattacccagggccacatccttggccaattgcaagccatcaacaaagcccgccaagagtttctgctacgaaagggacggggggtttacctggacccccagtccggcgaggagctcaacccaatccccccgccgccgcagccctatcagcagccgcgggcccttgcttcccaggatggcacccaaaaagaagctgcagctgccgccgccgccacccacggacgaggaggaatactgggacagtcaggcagaggaggttttggacgaggaggaggagatgatggaagactgggacagcctagacgaagcttccgaggccgaagaggtgtcagacgaaacaccgtcaccctcggtcgcattcccctcgccggcgccccagaaattggcaaccgttcccagcatcgctacaacctccgctcctcaggcgccgccggcactgcctgttcgccgacccaaccgtagatgggacaccactggaaccagggccggtaagtctaagcagccgccgccgttagcccaagagcaacaacagcgccaaggctaccgctcgtggcgcgggcacaagaacgccatagttgcttgcttgcaagactgtgggggcaacatctccttcgcccgccgctttcttctctaccatcacggcgtggccttcccccgtaacatcctgcattactaccgtcatctctacagcccctactgcaccggcggcagcggcagcggcagcaacagcagcggtcacacagaagcaaaggcgaccggatagcaagactctgacaaagcccaagaaatccacagcggcggcagcagcaggaggaggagcgctgcgtctggcgcccaacgaacccgtatcgacccgcgagcttagaaataggatttttcccactctgtatgctatatttcaacaaagcaggggccaagaacaagagctgaaaataaaaaacaggtctctgcgctccctcacccgcagctgcctgtatcacaaaagcgaagatcagcttcggcgcacgctggaagacgcggaggctctcttcagcaaatactgcgcgctgactcttaaggactagtttcgcgccctttctcaaatttaagcgcgaaaactacgtcatctccagcggccacacccggcgccagcacctgtcgtcagcgccattatgagcaaggaaattcccacgccctacatgtggagttaccagccacaaatgggacttgcggctggagctgcccaagactactcaacccgaataaactacatgagcgcgggaccccacatgatatcccgggtcaacggaatccgcgcccaccgaaaccgaattctcctcgaacaggcggctattaccaccacacctcgtaataaccttaatccccgtagttggcccgctgccctggtgtaccaggaaagtcccgctcccaccactgtggtacttcccagagacgcccaggccgaagttcagatgactaactcaggggcgcagcttgcgggcggctttcgtcacagggtgcggtcgcccgggcgttttagggcggagtaacttgcatgtattgggaattgtagtttttttaaaatgggaagtgacgtatcgtgggaaaacggaagtgaagatttgaggaagttgtgggttttttggctttcgtttctgggcgtaggttcgcgtgcggttttctgggtgttttttgtggactttaaccgttacgtcattttttagtcctatatatactcgctctgtacttggccctttttacactgtgactgattgagctggtgccgtgtcgagtggtgttttttaataggtttttttactggtaaggctgactgttatggctgccgctgtggaagcgctgtatgttgttctggagcgggagggtgctattttgcctaggcaggagggtttttcaggtgtttatgtgtttttctctcctattaattttgttatacctcctatgggggctgtaatgttgtctctacgcctgcgggtatgtattcccccgggctatttcggtcgctttttagcactgaccgatgttaaccaacctgatgtgtttaccgagtcttacattatgactccggacatgaccgaggaactgtcggtggtgctttttaatcacggtgaccagtttttttacggtcacgccggcatggccgtagtccgtcttatgcttataagggttgtttttcctgttgtaagacaggcttctaatgtttaaatgtttttttttttgttattttattttgtgtttaatgcaggaacccgcagacatgtttgagagaaaaatggtgtctttttctgtggtggttccggaacttacctgcctttatctgcatgagcatgactacgatgtgcttgcttttttgcgcgaggctttgcctgattttttgagcagcaccttgcattttatatcgccgcccatgcaacaagcttacataggggctacgctggttagcatagctccgagtatgcgtgtcataatcagtgtgggttcttttgtcatggttcctggcggggaagtggccgcgctggtccgtgcagacctgcacgattatgttcagctggccctgcgaagggacctacgggatcgcggtatttttgttaatgttccgcttttgaatcttatacaggtctgtgaggaacctgaatttttgcaatcatgattcgctgcttgaggctgaaggtggagggcgctctggagcagatttttacaatggccggacttaatattcgggatttgcttagagacatattgataaggtggcgagatgaaaattatttgggcatggttgaaggtgctggaatgtttatagaggagattcaccctgaagggtttagcctttacgtccacttggacgtgagggcagtttgccttttggaagccattgtgcaacatcttacaaatgccattatctgttctttggctgtagagtttgaccacgccaccggaggggagcgcgttcacttaatagatcttcattttgaggttttggataatcttttggaataaaaaaaaaaaaacatggttcttccagctcttcccgctcctcccgtgtgtgactcgcagaacgaatgtgtaggttggctgggtgtggcttattctgcggtggtggatgttatcagggcagcggcgcatgaaggagtttacatagaacccgaagccagggggcgcctggatgctttgagagagtggatatactacaactactacacagagcgagctaagcgacgagaccggagacgcagatctgtttgtcacgcccgcacctggttttgcttcaggaaatatgactacgtccggcgttccatttggcatgacactacgaccaacacgatctcggttgtctcggcgcactccgtacagtagggatcgcctacctccttttgagacagagacccgcgctaccatactggaggatcatccgctgctgcccgaatgtaacactttgacaatgcacaacgtgagttacgtgcgaggtcttccctgcagtgtgggatttacgctgattcaggaatgggttgttccctgggatatggttctgacgcgggaggagcttgtaatcctgaggaagtgtatgcacgtgtgcctgtgttgtgccaacattgatatcatgacgagcatgatgatccatggttacgagtcctgggctctccactgtcattgttccagtcccggttccctgcagtgcatagccggcgggcaggttttggccagctggtttaggatggtggtggatggcgccatgtttaatcagaggtttatatggtaccgggaggtggtgaattacaacatgccaaaagaggtaatgtttatgtccagcgtgtttatgaggggtcgccacttaatctacctgcgcttgtggtatgatggccacgtgggttctgtggtccccgccatgagctttggatacagcgccttgcactgtgggattttgaacaatattgtggtgctgtgctgcagttactgtgctgatttaagtgagatcagggtgcgctgctgtgcccggaggacaaggcgtctcatgctgcgggcggtgcgaatcatcgctgaggagaccactgccatgttgtattcctgcaggacggagcggcggcggcagcagtttattcgcgcgctgctgcagcaccaccgccctatcctgatgcacgattatgactctacccccatgtaggcgtggacttccccttcgccgcccgttgagcaaccgcaagttggacagcagcctgtggctcagcagctggacagcgacatgaacttaagcgagctgcccggggagtttattaatatcactgatgagcgtttggctcgacaggaaaccgtgtggaatataacacctaagaatatgtctgttacccatgatatgatgctttttaaggccagccggggagaaaggactgtgtactctgtgtgttgggagggaggtggcaggttgaatactagggttctgtgagtttgattaaggtacggtgatcaatataagctatgtggtggtggggctatactactgaatgaaaaatgacttgaaattttctgcaattgaaaaataaacacgttgaaacataacatgcaacaggttcacgattctttattcctgggcaatgtaggagaaggtgtaagagttggtagcaaaagtttcagtggtgtattttccactttcccaggaccatgtaaaagacatagagtaagtgcttacctcgctagtttctgtggattcactagaatcgatgtaggatgttgcccctcctgacgcggtaggagaaggggagggtgccctgcatgtctgccgctgctcttgctcttgccgctgctgaggaggggggcgcatctgccgcagcaccggatgcatctgggaaaagcaaaaaaggggctcgtccctgtttccggaggaatttgcaagcggggtcttgcatgacggggaggcaaacccccgttcgccgcagtccggccggcccgagactcgaaccgggggtcctgcgactcaacccttggaaaataaccctccggctacagggagcgagccacttaatgctttcgctttccagcctaaccgcttacgccgcgcgcggccagtggccaaaaaagctagcgcagcagccgccgcgcctggaaggaagccaaaaggagcgctcccccgttgtctgacgtcgcacacctgggttcgacacgcgggcggtaaccgcatggatcacggcggacggccggatccggggttcgaaccccggtcgtccgccatgatacccttgcgaatttatccaccagaccacggaagagtgcccgcttacaggctctccttttgcacggtctagagcgtcaacgactgcgcacgcctcaccggccagagcgtcccgaccatggagcactttttgccgctgcgcaacatctggaaccgcgtccgcgactttccgcgcgcctccaccaccgccgccggcatcacctggatgtccaggtacatctacggattacgtcgacgtttaaaccatatgatcagctcactcaaaggcggtaatacggttatccacagaatcaggggataacgcaggaaagaacatgtgagcaaaaggccagcaaaaggccaggaaccgtaaaaaggccgcgttgctggcgtttttccataggctccgcccccctgacgagcatcacaaaaatcgacgctcaagtcagaggtggcgaaacccgacaggactataaagataccaggcgtttccccctggaagctccctcgtgcgctctcctgttccgaccctgccgcttaccggatacctgtccgcctttctcccttcgggaagcgtggcgctttctcatagctcacgctgtaggtatctcagttcggtgtaggtcgttcgctccaagctgggctgtgtgcacgaaccccccgttcagcccgaccgctgcgccttatccggtaactatcgtcttgagtccaacccggtaagacacgacttatcgccactggcagcagccactggtaacaggattagcagagcgaggtatgtaggcggtgctacagagttcttgaagtggtggcctaactacggctacactagaagaacagtatttggtatctgcgctctgctgaagccagttaccttcggaaaaagagttggtagctcttgatccggcaaacaaaccaccgctggtagcggtggtttttttgtttgcaagcagcagattacgcgcagaaaaaaaggatctcaagaagatcctttgatcttttctacggggtctgacgctcagtggaacgaaaactcacgttaagggattttggtcatgagattatcaaaaaggatcttcacctagatccttttaaattaaaaatgaagttttaaatcaatctaaagtatatatgagtaaacttggtctgacagttaccaatgcttaatcagtgaggcacctatctcagcgatctgtctatttcgttcatccatagttgcctgactccccgtcgtgtagataactacgatacgggagggcttaccatctggccccagtgctgcaatgataccgcgagacccacgctcaccggctccagatttatcagcaataaaccagccagccggaagggccgagcgcagaagtggtcctgcaactttatccgcctccatccagtctattaattgttgccgggaagctagagtaagtagttcgccagttaatagtttgcgcaacgttgttgccattgctacaggcatcgtggtgtcacgctcgtcgtttggtatggcttcattcagctccggttcccaacgatcaaggcgagttacatgatcccccatgttgtgcaaaaaagcggttagctccttcggtcctccgatcgttgtcagaagtaagttggccgcagtgttatcactcatggttatggcagcactgcataattctcttactgtcatgccatccgtaagatgcttttctgtgactggtgagtactcaaccaagtcattctgagaatagtgtatgcggcgaccgagttgctcttgcccggcgtcaatacgggataataccgcgccacatagcagaactttaaaagtgctcatcattggaaaacgttcttcggggcgaaaactctcaaggatcttaccgctgttgagatccagttcgatgtaacccactcgtgcacccaactgatcttcagcatcttttactttcaccagcgtttctgggtgagcaaaaacaggaaggcaaaatgccgcaaaaaagggaataagggcgacacggaaatgttgaatactcatactcttcctttttcaatattattgaagcatttatcagggttattgtctcatgagcggatacatatttgaatgtatttagaaaaataaacaaataggggttccgcgcacatttccccgaaaagtgccacctaaattgtaagcgttaatattttgttaaaattcgcgttaaatttttgttaaatcagctcattttttaaccaataggccgaaatcggcaaaatcccttataaatcaaaagaatagaccgagatagggttgagtgttgttccagtttggaacaagagtccactattaaagaacgtggactccaacgtcaaagggcgaaaaaccgtctatcagggcgatggcccactacgtgaaccatcaccctaatcaagttttttggggtcgaggtgccgtaaagcactaaatcggaaccctaaagggagcccccgatttagagcttgacggggaaagccggcgaacgtggcgagaaaggaagggaagaaagcgaaaggagcgggcgctagggcgctggcaagtgtagcggtcacgctgcgcgtaaccaccacacccgccgcgcttaatgcgccgctacagggcgcgatggatcc

SEQ ID NO: 11 - DNA, 21 bp, synthetic construct
  source 1..21: mol_type = other DNA
ggaacccctagtgatggagtt

SEQ ID NO: 12 - DNA, 18 bp, synthetic construct
  source 1..18: mol_type = other DNA
cactccctctctgcgcgc

SEQ ID NO: 13 - DNA, 16 bp, synthetic construct
  source 1..16: mol_type = other DNA
cggcctcagtgagcga

SEQ ID NO: 14 - DNA, 568 bp, synthetic construct
  source 1..568: mol_type = other DNA
tagttattaatagtaatcaattacggggtcattagttcatagcccatatatggagttccgcgttacataacttacggtaaatggcccgcctggctgaccgcccaacgacccccgcccattgacgtcaataatgacgtatgttcccatagtaacgccaatagggactttccattgacgtcaatgggtggagtatttacggtaaactgcccacttggcagtacatcaagtgtatcatatgccaagtacgccccctattgacgtcaatgacggtaaatggcccgcctggcattatgcccagtacatgaccttatgggactttcctacttggcagtacatctacgtattagtcatcgctattaccatggtgatgcggttttggcagtacatcaatgggcgtggatagcggtttgactcacggggatttccaagtctccaccccattgacgtcaatgggagtttgttttggcaccaaaatcaacgggactttccaaaatgtcgtaacaactccgccccattgacgcaaatgggcggtaggcgtgtacggtgggaggtctatataagcagagct

SEQ ID NO: 15 - DNA, 5670 bp, synthetic construct
  source 1..5670: mol_type = other DNA
acatgtgagcaaaaggccagcaaaaggccaggaaccgtaaaaaggccgcgttgctggcgtttttccataggctccgcccccctgacgagcatcacaaaaatcgacgctcaagtcagaggtggcgaaacccgacaggactataaagataccaggcgtttccccctggaagctccctcgtgcgctctcctgttccgaccctgccgcttaccggatacctgtccgcctttctcccttcgggaagcgtggcgctttctcatagctcacgctgtaggtatctcagttcggtgtaggtcgttcgctccaagctgggctgtgtgcacgaaccccccgttcagcccgaccgctgcgccttatccggtaactatcgtcttgagtccaacccggtaagacacgacttatcgccactggcagcagccactggtaacaggattagcagagcgaggtatgtaggcggtgctacagagttcttgaagtggtggcctaactacggctacactagaaggacagtatttggtatctgcgctctgctgaagccagttaccttcggaaaaagagttggtagctcttgatccggcaaacaaaccaccgctggtagcggtggtttttttgtttgcaagcagcagattacgcgcagaaaaaaaggatctcaagaagatcctttgatcttttctacggggtctgacgctcagtggaacgaaaactcacgttaagggattttggtcatgagattatcaaaaaggatcttcacctagatccttttaaattaaaaatgaagttttaaatcaatctaaagtatatatgagtaaacttggtctgacagttaccaatgcttaatcagtgaggcacctatctcagcgatctgtctatttcgttcatccatagttgcctgactccccgtcgtgtagataactacgatacgggagggcttaccatctggccccagtgctgcaatgataccgcgagacccacgctcaccggctccagatttatcagcaataaaccagccagccggaagggccgagcgcagaagtggtcctgcaactttatccgcctccatccagtctattaattgttgccgggaagctagagtaagtagttcgccagttaatagtttgcgcaacgttgttgccattgctacaggcatcgtggtgtcacgctcgtcgtttggtatggcttcattcagctccggttcccaacgatcaaggcgagttacatgatcccccatgttgtgcaaaaaagcggttagctccttcggtcctccgatcgttgtcagaagtaagttggccgcagtgttatcactcatggttatggcagcactgcataattctcttactgtcatgccatccgtaagatgcttttctgtgactggtgagtactcaaccaagtcattctgagaatagtgtatgcggcgaccgagttgctcttgcccggcgtcaatacgggataataccgcgccacatagcagaactttaaaagtgctcatcattggaaaacgttcttcggggcgaaaactctcaaggatcttaccgctgttgagatccagttcgatgtaacccactcgtgcacccaactgatcttcagcatcttttactttcaccagcgtttctgggtgagcaaaaacaggaaggcaaaatgccgcaaaaaagggaataagggcgacacggaaatgttgaatactcatactcttcctttttcaatattattgaagcatttatcagggttattgtctcatgagcggatacatatttgaatgtatttagaaaaataaacaaataggggttccgcgcacatttccccgaaaagtgccacctgacgtctaagaaaccattattatcatgacattaacctataaaaataggcgtatcacgaggccctttcgtctcgcgcgtttcggtgatgacggtgaaaacctctgacacatgcagctcccggagacggtcacagcttgtctgtaagcggatgccgggagcagacaagcccgtcagggcgcgtcagcgggtgttggcgggtgtcggggctggcttaactatgcggcatcagagcagattgtactgagagtgcaccataaaattgtaaacgttaatattttgttaaaattcgcgttaaatttttgttaaatcagctcattttttaaccaataggccgaaatcggcaaaatcccttataaatcaaaagaatagcccgagatagggttgagtgttgttccagtttggaacaagagtccactattaaagaacgtggactccaacgtcaaagggcgaaaaaccgtctatcagggcgatggcccactacgtgaaccatcacccaaatcaagttttttggggtcgaggtgccgtaaagcactaaatcggaaccctaaagggagcccccgatttagagcttgacggggaaagccggcgaacgtggcgagaaaggaagggaagaaagcgaaaggagcgggcgctagggcgctggcaagtgtagcggtcacgctgcgcgtaaccaccacacccgccgcgcttaatgcgccgctacagggcgcgtactatggttgctttgacgtatgcggtgtgaaataccgcacagatgcgtaaggagaaaataccgcatcaggcgcccctgcaggcagctgcgcgctcgctcgctcactgaggccgcccgggcaaagcccgggcgtcgggcgacctttggtcgcccggcctcagtgagcgagcgagcgcgcagagagggagtggccaactccatcactaggggttcctacgcgttagttattaatagtaatcaattacggggtcattagttcatagcccatatatggagttccgcgttacataacttacggtaaatggcccgcctggctgaccgcccaacgacccccgcccattgacgtcaataatgacgtatgttcccatagtaacgccaatagggactttccattgacgtcaatgggtggagtatttacggtaaactgcccacttggcagtacatcaagtgtatcatatgccaagtacgccccctattgacgtcaatgacggtaaatggcccgcctggcattatgcccagtacatgaccttatgggactttcctacttggcagtacatctacgtattagtcatcgctattaccatggtgatgcggttttggcagtacatcaatgggcgtggatagcggtttgactcacggggatttccaagtctccaccccattgacgtcaatgggagtttgttttggcaccaaaatcaacgggactttccaaaatgtcgtaacaactccgccccattgacgcaaatgggcggtaggcgtgtacggtgggaggtctatataagcagagctacacccaagctgtctagagccgccaccaccggtgccaccatgcagcgggtaaatatgatcatggccgagagtcccggactcatcactatatgcctcttgggttacttgcttagcgcagaatgtacagtgtttctggaccatgagaatgccaacaaaatactgaatcggcccaaaaggtacaacagtggtaagctggaagagtttgtccaagggaatctcgagcgggaatgcatggaagaaaaatgcagcttcgaagaggcaagggaggtatttgagaataccgaacgcactactgagttttggaaacaatacgttgacggagaccaatgtgagtctaatccgtgccttaatggaggttcatgtaaagacgatataaacagttacgaatgttggtgccctttcggctttgagggtaaaaactgtgagttggatgtcacctgcaacataaaaaacggacgatgtgaacaattttgcaagaactctgctgataacaaagtagtgtgttcatgtactgaagggtatcgcttggcggaaaaccaaaagagttgcgaaccagcggttccatttccttgcggcagggtctcagtttcccaaacctctaagttgacaagggccgagacggtgtttccggatgtagactatgtgaatagcacggaggcagagactatactcgacaatattacccaaagcacacagtcatttaatgatttcacccgagtggtaggaggggaagacgctaaaccaggacaattcccttggcaggtggttttgaacggcaaggtagatgctttttgtgggggctcaatcgttaacgagaaatggatagtaacggccgcgcattgtgtagaaacgggtgtgaagatcacagtggtagctggtgaacacaacatcgaagagacggagcacacagaacaaaagaggaatgttatccgcattatccctcatcataactacaatgctgctataaacaagtataatcacgacatagcacttcttgaactggacgaacctcttgtcttgaattcctatgtgacacccatctgtatcgctgataaagaatatacaaacatcttccttaaatttggtagtggttacgtatcaggctggggtcgggtcttccacaaaggcagaagtgcattggtattgcagtatcttagagtacccttggtggatagagcgacttgtcttctgagtacgaaatttaccatttacaataatatgttttgcgctggcttccatgagggtggacgggacagttgccaaggagattcaggcggacctcacgtaacggaagtggagggcacgtcattcctgacgggcattattagctggggtgaagagtgtgcaatgaagggaaagtatgggatctatacgaaggtctccaggtatgtgaattggataaaggagaagaccaagctcacgtaggtcgacaatcaacctctggattacaaaatttgtgaaagattgactggtattcttaactatgttgctccttttacgctatgtggatacgctgctttaatgcctttgtatcatgctattgcttcccgtatggctttcattttctcctccttgtataaatcctggttgctgtctctttatgaggagttgtggcccgttgtcaggcaacgtggcgtggtgtgcactgtgtttgctgacgcaacccccactggttggggcattgccaccacctgtcagctcctttccgggactttcgctttccccctccctattgccacggcggaactcatcgccgcctgccttgcccgctgctggacaggggctcggctgttgggcactgacaattccgtggtgttgtcggggaagctgacgtcctttccatggctgctcgcctgtgttgccacctggattctgcgcgggacgtccttctgctacgtcccttcggccctcaatccagcggaccttccttcccgcggcctgctgccggctctgcggcctcttccgcgtcttcgccttcgccctcagacgagtcggatctccctttgggccgcctccccgcctggtcgacgtttatttgtgaaatttgtgatgctattgctttatttgtaaccatctagctttatttgtgaaatttgtgatgctattgctttatttgtaaccattataagctgcaataaacaagttaacaacaacaattgcattcattttatgtttcaggttcagggggagatgtgggaggttttttaaagtttaaacaggaacccctagtgatggagttggccactccctctctgcgcgctcgctcgctcactgaggccgggcgaccaaaggtcgcccgacgcccgggctttgcccgggcggcctcagtgagcgagcgagcgcgcagctgcctgcagg

SEQ ID NO: 16 - DNA, 872 bp, synthetic construct
  source 1..872: mol_type = other DNA
tagttattaatagtaatcaattacggggtcattagttcatagcccatatatggagttccgcgttacataacttacggtaaatggcccgcctggctgaccgcccaacgacccccgcccattgacgtcaataatgacgtatgttcccatagtaacgccaatagggactttccattgacgtcaatgggtggagtatttacggtaaactgcccacttggcagtacatcaagtgtatcatatgccaagtacgccccctattgacgtcaatgacggtaaatggcccgcctggcattatgcccagtacatgaccttatgggactttcctacttggcagtacatctacgtattagtcatcgctattaccatggtcgaggtgagccccacgttctgcttcactctccccatctcccccccctccccacccccaattttgtatttatttattttttaattattttgtgcagcgatgggggcggggggggggggggggcgcgcgccaggcggggcggggcggggcgaggggcggggcggggcgaggcggagaggtgcggcggcagccaatcagagcggcgcgctccgaaagtttccttttatggcgaggcggcggcggcggcggccctataaaaagcgaagcgcgcggcgggcgggagtcgctgcgacgctgccttcgccccgtgccccgctccgccgccgcctcgcgccgcccgccccggctctgactgaccgcgttactcccacaggtgagcgggcgggacggcccttctcctccgggctgtaattagctgagcaagaggtaagggtttaagggatggttggttggtggggtattaatgtttaattacctggagcacctgcctgaaatcactttttttcag

SEQ ID NO: 17 - DNA, 5974 bp, synthetic construct
  source 1..5974: mol_type = other DNA
acatgtgagcaaaaggccagcaaaaggccaggaaccgtaaaaaggccgcgttgctggcgtttttccataggctccgcccccctgacgagcatcacaaaaatcgacgctcaagtcagaggtggcgaaacccgacaggactataaagataccaggcgtttccccctggaagctccctcgtgcgctctcctgttccgaccctgccgcttaccggatacctgtccgcctttctcccttcgggaagcgtggcgctttctcatagctcacgctgtaggtatctcagttcggtgtaggtcgttcgctccaagctgggctgtgtgcacgaaccccccgttcagcccgaccgctgcgccttatccggtaactatcgtcttgagtccaacccggtaagacacgacttatcgccactggcagcagccactggtaacaggattagcagagcgaggtatgtaggcggtgctacagagttcttgaagtggtggcctaactacggctacactagaaggacagtatttggtatctgcgctctgctgaagccagttaccttcggaaaaagagttggtagctcttgatccggcaaacaaaccaccgctggtagcggtggtttttttgtttgcaagcagcagattacgcgcagaaaaaaaggatctcaagaagatcctttgatcttttctacggggtctgacgctcagtggaacgaaaactcacgttaagggattttggtcatgagattatcaaaaaggatcttcacctagatccttttaaattaaaaatgaagttttaaatcaatctaaagtatatatgagtaaacttggtctgacagttaccaatgcttaatcagtgaggcacctatctcagcgatctgtctatttcgttcatccatagttgcctgactccccgtcgtgtagataactacgatacgggagggcttaccatctggccccagtgctgcaatgataccgcgagacccacgctcaccggctccagatttatcagcaataaaccagccagccggaagggccgagcgcagaagtggtcctgcaactttatccgcctccatccagtctattaattgttgccgggaagctagagtaagtagttcgccagttaatagtttgcgcaacgttgttgccattgctacaggcatcgtggtgtcacgctcgtcgtttggtatggcttcattcagctccggttcccaacgatcaaggcgagttacatgatcccccatgttgtgcaaaaaagcggttagctccttcggtcctccgatcgttgtcagaagtaagttggccgcagtgttatcactcatggttatggcagcactgcataattctcttactgtcatgccatccgtaagatgcttttctgtgactggtgagtactcaaccaagtcattctgagaatagtgtatgcggcgaccgagttgctcttgcccggcgtcaatacgggataataccgcgccacatagcagaactttaaaagtgctcatcattggaaaacgttcttcggggcgaaaactctcaaggatcttaccgctgttgagatccagttcgatgtaacccactcgtgcacccaactgatcttcagcatcttttactttcaccagcgtttctgggtgagcaaaaacaggaaggcaaaatgccgcaaaaaagggaataagggcgacacggaaatgttgaatactcatactcttcctttttcaatattattgaagcatttatcagggttattgtctcatgagcggatacatatttgaatgtatttagaaaaataaacaaataggggttccgcgcacatttccccgaaaagtgccacctgacgtctaagaaaccattattatcatgacattaacctataaaaataggcgtatcacgaggccctttcgtctcgcgcgtttcggtgatgacggtgaaaacctctgacacatgcagctcccggagacggtcacagcttgtctgtaagcggatgccgggagcagacaagcccgtcagggcgcgtcagcgggtgttggcgggtgtcggggctggcttaactatgcggcatcagagcagattgtactgagagtgcaccataaaattgtaaacgttaatattttgttaaaattcgcgttaaatttttgttaaatcagctcattttttaaccaataggccgaaatcggcaaaatcccttataaatcaaaagaatagcccgagatagggttgagtgttgttccagtttggaacaagagtccactattaaagaacgtggactccaacgtcaaagggcgaaaaaccgtctatcagggcgatggcccactacgtgaaccatcacccaaatcaagttttttggggtcgaggtgccgtaaagcactaaatcggaaccctaaagggagcccccgatttagagcttgacggggaaagccggcgaacgtggcgagaaaggaagggaagaaagcgaaaggagcgggcgctagggcgctggcaagtgtagcggtcacgctgcgcgtaaccaccacacccgccgcgcttaatgcgccgctacagggcgcgtactatggttgctttgacgtatgcggtgtgaaataccgcacagatgcgtaaggagaaaataccgcatcaggcgcccctgcaggcagctgcgcgctcgctcgctcactgaggccgcccgggcaaagcccgggcgtcgggcgacctttggtcgcccggcctcagtgagcgagcgagcgcgcagagagggagtggccaactccatcactaggggttcctacgcgttagttattaatagtaatcaattacggggtcattagttcatagcccatatatggagttccgcgttacataacttacggtaaatggcccgcctggctgaccgcccaacgacccccgcccattgacgtcaataatgacgtatgttcccatagtaacgccaatagggactttccattgacgtcaatgggtggagtatttacggtaaactgcccacttggcagtacatcaagtgtatcatatgccaagtacgccccctattgacgtcaatgacggtaaatggcccgcctggcattatgcccagtacatgaccttatgggactttcctacttggcagtacatctacgtattagtcatcgctattaccatggtcgaggtgagccccacgttctgcttcactctccccatctcccccccctccccacccccaattttgtatttatttattttttaattattttgtgcagcgatgggggcggggggggggggggggcgcgcgccaggcggggcggggcggggcgaggggcggggcggggcgaggcggagaggtgcggcggcagccaatcagagcggcgcgctccgaaagtttccttttatggcgaggcggcggcggcggcggccctataaaaagcgaagcgcgcggcgggcgggagtcgctgcgacgctgccttcgccccgtgccccgctccgccgccgcctcgcgccgcccgccccggctctgactgaccgcgttactcccacaggtgagcgggcgggacggcccttctcctccgggctgtaattagctgagcaagaggtaagggtttaagggatggttggttggtggggtattaatgtttaattacctggagcacctgcctgaaatcactttttttcagacacccaagctgtctagagccgccaccaccggtgccaccatgcagcgggtaaatatgatcatggccgagagtcccggactcatcactatatgcctcttgggttacttgcttagcgcagaatgtacagtgtttctggaccatgagaatgccaacaaaatactgaatcggcccaaaaggtacaacagtggtaagctggaagagtttgtccaagggaatctcgagcgggaatgcatggaagaaaaatgcagcttcgaagaggcaagggaggtatttgagaataccgaacgcactactgagttttggaaacaatacgttgacggagaccaatgtgagtctaatccgtgccttaatggaggttcatgtaaagacgatataaacagttacgaatgttggtgccctttcggctttgagggtaaaaactgtgagttggatgtcacctgcaacataaaaaacggacgatgtgaacaattttgcaagaactctgctgataacaaagtagtgtgttcatgtactgaagggtatcgcttggcggaaaaccaaaagagttgcgaaccagcggttccatttccttgcggcagggtctcagtttcccaaacctctaagttgacaagggccgagacggtgtttccggatgtagactatgtgaatagcacggaggcagagactatactcgacaatattacccaaagcacacagtcatttaatgatttcacccgagtggtaggaggggaagacgctaaaccaggacaattcccttggcaggtggttttgaacggcaaggtagatgctttttgtgggggctcaatcgttaacgagaaatggatagtaacggccgcgcattgtgtagaaacgggtgtgaagatcacagtggtagctggtgaacacaacatcgaagagacggagcacacagaacaaaagaggaatgttatccgcattatccctcatcataactacaatgctgctataaacaagtataatcacgacatagcacttcttgaactggacgaacctcttgtcttgaattcctatgtgacacccatctgtatcgctgataaagaatatacaaacatcttccttaaatttggtagtggttacgtatcaggctggggtcgggtcttccacaaaggcagaagtgcattggtattgcagtatcttagagtacccttggtggatagagcgacttgtcttctgagtacgaaatttaccatttacaataatatgttttgcgctggcttccatgagggtggacgggacagttgccaaggagattcaggcggacctcacgtaacggaagtggagggcacgtcattcctgacgggcattattagctggggtgaagagtgtgcaatgaagggaaagtatgggatctatacgaaggtctccaggtatgtgaattggataaaggagaagaccaagctcacgtaggtcgacaatcaacctctggattacaaaatttgtgaaagattgactggtattcttaactatgttgctccttttacgctatgtggatacgctgctttaatgcctttgtatcatgctattgcttcccgtatggctttcattttctcctccttgtataaatcctggttgctgtctctttatgaggagttgtggcccgttgtcaggcaacgtggcgtggtgtgcactgtgtttgctgacgcaacccccactggttggggcattgccaccacctgtcagctcctttccgggactttcgctttccccctccctattgccacggcggaactcatcgccgcctgccttgcccgctgctggacaggggctcggctgttgggcactgacaattccgtggtgttgtcggggaagctgacgtcctttccatggctgctcgcctgtgttgccacctggattctgcgcgggacgtccttctgctacgtcccttcggccctcaatccagcggaccttccttcccgcggcctgctgccggctctgcggcctcttccgcgtcttcgccttcgccctcagacgagtcggatctccctttgggccgcctccccgcctggtcgacgtttatttgtgaaatttgtgatgctattgctttatttgtaaccatctagctttatttgtgaaatttgtgatgctattgctttatttgtaaccattataagctgcaataaacaagttaacaacaacaattgcattcattttatgtttcaggttcagggggagatgtgggaggttttttaaagtttaaacaggaacccctagtgatggagttggccactccctctctgcgcgctcgctcgctcactgaggccgggcgaccaaaggtcgcccgacgcccgggctttgcccgggcggcctcagtgagcgagcgagcgcgcagctgcctgcagg

SEQ ID NO: 18 - DNA, 1602 bp, synthetic construct
  source 1..1602: mol_type = other DNA
cgttacataacttacggtaaatggcccgcctggctgaccgcccaacgacccccgcccattgacgtcaataatgacgtatgttcccatagtaacgccaatagggactttccattgacgtcaatgggtggagtatttacggtaaactgcccacttggcagtacatcaagtgtatcatatgccaagtacgccccctattgacgtcaatgacggtaaatggcccgcctggcattatgcccagtacatgaccttatgggactttcctacttggcagtacatctacgtattagtcatcgctattaccatggtcgaggtgagccccacgttctgcttcactctccccatctcccccccctccccacccccaattttgtatttatttattttttaattattttgtgcagcgatgggggcggggggggggggggggcgcgcgccaggcggggcggggcggggcgaggggcggggcggggcgaggcggagaggtgcggcggcagccaatcagagcggcgcgctccgaaagtttccttttatggcgaggcggcggcggcggcggccctataaaaagcgaagcgcgcggcgggcggggagtcgctgcgacgctgccttcgccccgtgccccgctccgccgccgcctcgcgccgcccgccccggctctgactgaccgcgttactcccacaggtgagcgggcgggacggcccttctcctccgggctgtaattagcgcttggtttaatgacggcttgtttcttttctgtggctgcgtgaaagccttgaggggctccgggagggccctttgtgcggggggagcggctcggggggtgcgtgcgtgtgtgtgtgcgtggggagcgccgcgtgcggctccgcgctgcccggcggctgtgagcgctgcgggcgcggcgcggggctttgtgcgctccgcagtgtgcgcgaggggagcgcggccgggggcggtgccccgcggtgcggggggggctgcgaggggaacaaaggctgcgtgcggggtgtgtgcgtgggggggtgagcagggggtgtgggcgcgtcggtcgggctgcaaccccccctgcacccccctccccgagttgctgagcacggcccggcttcgggtgcggggctccgtacggggcgtggcgcggggctcgccgtgccgggcggggggtggcggcaggtgggggtgccgggcggggcggggccgcctcgggccggggagggctcgggggaggggcgcggcggcccccggagcgccggcggctgtcgaggcgcggcgagccgcagccattgccttttatggtaatcgtgcgagagggcgcagggacttcctttgtcccaaatctgtgcggagccgaaatctgggaggcgccgccgcaccccctctagcgggcgcggggcgaagcggtgcggcgccggcaggaaggaaatgggcggggagggccttcgtgcgtcgccgcgccgccgtccccttctccctctccagcctcggggctgtccgcggggggacggctgccttcgggggggacggggcagggcggggttcggcttctggcgtgtgaccggcggctctagagcctctgctaaccatgttcatgccttcttctttttcctacag

SEQ ID NO: 19 - DNA, 6704 bp, synthetic construct
  source 1..6704: mol_type = other DNA
acatgtgagcaaaaggccagcaaaaggccaggaaccgtaaaaaggccgcgttgctggcgtttttccataggctccgcccccctgacgagcatcacaaaaatcgacgctcaagtcagaggtggcgaaacccgacaggactataaagataccaggcgtttccccctggaagctccctcgtgcgctctcctgttccgaccctgccgcttaccggatacctgtccgcctttctcccttcgggaagcgtggcgctttctcatagctcacgctgtaggtatctcagttcggtgtaggtcgttcgctccaagctgggctgtgtgcacgaaccccccgttcagcccgaccgctgcgccttatccggtaactatcgtcttgagtccaacccggtaagacacgacttatcgccactggcagcagccactggtaacaggattagcagagcgaggtatgtaggcggtgctacagagttcttgaagtggtggcctaactacggctacactagaaggacagtatttggtatctgcgctctgctgaagccagttaccttcggaaaaagagttggtagctcttgatccggcaaacaaaccaccgctggtagcggtggtttttttgtttgcaagcagcagattacgcgcagaaaaaaaggatctcaagaagatcctttgatcttttctacggggtctgacgctcagtggaacgaaaactcacgttaagggattttggtcatgagattatcaaaaaggatcttcacctagatccttttaaattaaaaatgaagttttaaatcaatctaaagtatatatgagtaaacttggtctgacagttaccaatgcttaatcagtgaggcacctatctcagcgatctgtctatttcgttcatccatagttgcctgactccccgtcgtgtagataactacgatacgggagggcttaccatctggccccagtgctgcaatgataccgcgagacccacgctcaccggctccagatttatcagcaataaaccagccagccggaagggccgagcgcagaagtggtcctgcaactttatccgcctccatccagtctattaattgttgccgggaagctagagtaagtagttcgccagttaatagtttgcgcaacgttgttgccattgctacaggcatcgtggtgtcacgctcgtcgtttggtatggcttcattcagctccggttcccaacgatcaaggcgagttacatgatcccccatgttgtgcaaaaaagcggttagctccttcggtcctccgatcgttgtcagaagtaagttggccgcagtgttatcactcatggttatggcagcactgcataattctcttactgtcatgccatccgtaagatgcttttctgtgactggtgagtactcaaccaagtcattctgagaatagtgtatgcggcgaccgagttgctcttgcccggcgtcaatacgggataataccgcgccacatagcagaactttaaaagtgctcatcattggaaaacgttcttcggggcgaaaactctcaaggatcttaccgctgttgagatccagttcgatgtaacccactcgtgcacccaactgatcttcagcatcttttactttcaccagcgtttctgggtgagcaaaaacaggaaggcaaaatgccgcaaaaaagggaataagggcgacacggaaatgttgaatactcatactcttcctttttcaatattattgaagcatttatcagggttattgtctcatgagcggatacatatttgaatgtatttagaaaaataaacaaataggggttccgcgcacatttccccgaaaagtgccacctgacgtctaagaaaccattattatcatgacattaacctataaaaataggcgtatcacgaggccctttcgtctcgcgcgtttcggtgatgacggtgaaaacctctgacacatgcagctcccggagacggtcacagcttgtctgtaagcggatgccgggagcagacaagcccgtcagggcgcgtcagcgggtgttggcgggtgtcggggctggcttaactatgcggcatcagagcagattgtactgagagtgcaccataaaattgtaaacgttaatattttgttaaaattcgcgttaaatttttgttaaatcagctcattttttaaccaataggccgaaatcggcaaaatcccttataaatcaaaagaatagcccgagatagggttgagtgttgttccagtttggaacaagagtccactattaaagaacgtggactccaacgtcaaagggcgaaaaaccgtctatcagggcgatggcccactacgtgaaccatcacccaaatcaagttttttggggtcgaggtgccgtaaagcactaaatcggaaccctaaagggagcccccgatttagagcttgacggggaaagccggcgaacgtggcgagaaaggaagggaagaaagcgaaaggagcgggcgctagggcgctggcaagtgtagcggtcacgctgcgcgtaaccaccacacccgccgcgcttaatgcgccgctacagggcgcgtactatggttgctttgacgtatgcggtgtgaaataccgcacagatgcgtaaggagaaaataccgcatcaggcgcccctgcaggcagctgcgcgctcgctcgctcactgaggccgcccgggcaaagcccgggcgtcgggcgacctttggtcgcccggcctcagtgagcgagcgagcgcgcagagagggagtggccaactccatcactaggggttcctacgcgtcgttacataacttacggtaaatggcccgcctggctgaccgcccaacgacccccgcccattgacgtcaataatgacgtatgttcccatagtaacgccaatagggactttccattgacgtcaatgggtggagtatttacggtaaactgcccacttggcagtacatcaagtgtatcatatgccaagtacgccccctattgacgtcaatgacggtaaatggcccgcctggcattatgcccagtacatgaccttatgggactttcctacttggcagtacatctacgtattagtcatcgctattaccatggtcgaggtgagccccacgttctgcttcactctccccatctcccccccctccccacccccaattttgtatttatttattttttaattattttgtgcagcgatgggggcggggggggggggggggcgcgcgccaggcggggcggggcggggcgaggggcggggcggggcgaggcggagaggtgcggcggcagccaatcagagcggcgcgctccgaaagtttccttttatggcgaggcggcggcggcggcggccctataaaaagcgaagcgcgcggcgggcggggagtcgctgcgacgctgccttcgccccgtgccccgctccgccgccgcctcgcgccgcccgccccggctctgactgaccgcgttactcccacaggtgagcgggcgggacggcccttctcctccgggctgtaattagcgcttggtttaatgacggcttgtttcttttctgtggctgcgtgaaagccttgaggggctccgggagggccctttgtgcggggggagcggctcggggggtgcgtgcgtgtgtgtgtgcgtggggagcgccgcgtgcggctccgcgctgcccggcggctgtgagcgctgcgggcgcggcgcggggctttgtgcgctccgcagtgtgcgcgaggggagcgcggccgggggcggtgccccgcggtgcggggggggctgcgaggggaacaaaggctgcgtgcggggtgtgtgcgtgggggggtgagcagggggtgtgggcgcgtcggtcgggctgcaaccccccctgcacccccctccccgagttgctgagcacggcccggcttcgggtgcggggctccgtacggggcgtggcgcggggctcgccgtgccgggcggggggtggcggcaggtgggggtgccgggcggggcggggccgcctcgggccggggagggctcgggggaggggcgcggcggcccccggagcgccggcggctgtcgaggcgcggcgagccgcagccattgccttttatggtaatcgtgcgagagggcgcagggacttcctttgtcccaaatctgtgcggagccgaaatctgggaggcgccgccgcaccccctctagcgggcgcggggcgaagcggtgcggcgccggcaggaaggaaatgggcggggagggccttcgtgcgtcgccgcgccgccgtccccttctccctctccagcctcggggctgtccgcggggggacggctgccttcgggggggacggggcagggcggggttcggcttctggcgtgtgaccggcggctctagagcctctgctaaccatgttcatgccttcttctttttcctacagacacccaagctgtctagagccgccaccaccggtgccaccatgcagcgggtaaatatgatcatggccgagagtcccggactcatcactatatgcctcttgggttacttgcttagcgcagaatgtacagtgtttctggaccatgagaatgccaacaaaatactgaatcggcccaaaaggtacaacagtggtaagctggaagagtttgtccaagggaatctcgagcgggaatgcatggaagaaaaatgcagcttcgaagaggcaagggaggtatttgagaataccgaacgcactactgagttttggaaacaatacgttgacggagaccaatgtgagtctaatccgtgccttaatggaggttcatgtaaagacgatataaacagttacgaatgttggtgccctttcggctttgagggtaaaaactgtgagttggatgtcacctgcaacataaaaaacggacgatgtgaacaattttgcaagaactctgctgataacaaagtagtgtgttcatgtactgaagggtatcgcttggcggaaaaccaaaagagttgcgaaccagcggttccatttccttgcggcagggtctcagtttcccaaacctctaagttgacaagggccgagacggtgtttccggatgtagactatgtgaatagcacggaggcagagactatactcgacaatattacccaaagcacacagtcatttaatgatttcacccgagtggtaggaggggaagacgctaaaccaggacaattcccttggcaggtggttttgaacggcaaggtagatgctttttgtgggggctcaatcgttaacgagaaatggatagtaacggccgcgcattgtgtagaaacgggtgtgaagatcacagtggtagctggtgaacacaacatcgaagagacggagcacacagaacaaaagaggaatgttatccgcattatccctcatcataactacaatgctgctataaacaagtataatcacgacatagcacttcttgaactggacgaacctcttgtcttgaattcctatgtgacacccatctgtatcgctgataaagaatatacaaacatcttccttaaatttggtagtggttacgtatcaggctggggtcgggtcttccacaaaggcagaagtgcattggtattgcagtatcttagagtacccttggtggatagagcgacttgtcttctgagtacgaaatttaccatttacaataatatgttttgcgctggcttccatgagggtggacgggacagttgccaaggagattcaggcggacctcacgtaacggaagtggagggcacgtcattcctgacgggcattattagctggggtgaagagtgtgcaatgaagggaaagtatgggatctatacgaaggtctccaggtatgtgaattggataaaggagaagaccaagctcacgtaggtcgacaatcaacctctggattacaaaatttgtgaaagattgactggtattcttaactatgttgctccttttacgctatgtggatacgctgctttaatgcctttgtatcatgctattgcttcccgtatggctttcattttctcctccttgtataaatcctggttgctgtctctttatgaggagttgtggcccgttgtcaggcaacgtggcgtggtgtgcactgtgtttgctgacgcaacccccactggttggggcattgccaccacctgtcagctcctttccgggactttcgctttccccctccctattgccacggcggaactcatcgccgcctgccttgcccgctgctggacaggggctcggctgttgggcactgacaattccgtggtgttgtcggggaagctgacgtcctttccatggctgctcgcctgtgttgccacctggattctgcgcgggacgtccttctgctacgtcccttcggccctcaatccagcggaccttccttcccgcggcctgctgccggctctgcggcctcttccgcgtcttcgccttcgccctcagacgagtcggatctccctttgggccgcctccccgcctggtcgacgtttatttgtgaaatttgtgatgctattgctttatttgtaaccatctagctttatttgtgaaatttgtgatgctattgctttatttgtaaccattataagctgcaataaacaagttaacaacaacaattgcattcattttatgtttcaggttcagggggagatgtgggaggttttttaaagtttaaacaggaacccctagtgatggagttggccactccctctctgcgcgctcgctcgctcactgaggccgggcgaccaaaggtcgcccgacgcccgggctttgcccgggcggcctcagtgagcgagcgagcgcgcagctgcctgcagg

SEQ ID NO: 20 - DNA, 842 bp, synthetic construct
  source 1..842: mol_type = other DNA
tctaagctagacccttcagattaaaaataactgaggtaagggcctgggtaggggaggtggtgtgagacgctcctgtctctcctctatctgcccatcggccctttggggaggaggaatgtgcccaaggactaaaaaaaggccatggagccagaggggcgagggcaacagacctttcatgggcaaaccttggggccctgctgtctagcatgccccactacgggtctaggctgcccatgtaaggaggcaaggcctggggacacccgagatgcctggttataattaacccagacatgtggctgcccccccccccccaacacctgctgcctctaaaaataaccctgtccctggtggatcccctgcatgcgaagatcttcgaacaaggctgtgggggactgagggcaggctgtaacaggcttgggggccagggcttatacgtgcctgggactcccaaagtattactgttccatgttcccggcgaagggccagctgtcccccgccagctagactcagcacttagtttaggaaccagtgagcaagtcagcccttggggcagcccatacaaggccatggggctgggcaagctgcacgcctgggtccggggtgggcacggtgcccgggcaacgagctgaaagctcatctgctctcaggggcccctccctggggacagcccctcctggctagtcacaccctgtaggctcctctatataacccaggcaggggcacaggggctgccctcattctaccaccacctccacagcacagacagacactcaggagcagccagcggcgcgcccaggtaagtttagtctttttgtcttttatttcaggtcccggatccggtg

SEQ ID NO: 21 - DNA, 5933 bp, synthetic construct
  source 1..5933: mol_type = other DNA
acatgtgagcaaaaggccagcaaaaggccaggaaccgtaaaaaggccgcgttgctggcgtttttccataggctccgcccccctgacgagcatcacaaaaatcgacgctcaagtcagaggtggcgaaacccgacaggactataaagataccaggcgtttccccctggaagctccctcgtgcgctctcctgttccgaccctgccgcttaccggatacctgtccgcctttctcccttcgggaagcgtggcgctttctcatagctcacgctgtaggtatctcagttcggtgtaggtcgttcgctccaagctgggctgtgtgcacgaaccccccgttcagcccgaccgctgcgccttatccggtaactatcgtcttgagtccaacccggtaagacacgacttatcgccactggcagcagccactggtaacaggattagcagagcgaggtatgtaggcggtgctacagagttcttgaagtggtggcctaactacggctacactagaaggacagtatttggtatctgcgctctgctgaagccagttaccttcggaaaaagagttggtagctcttgatccggcaaacaaaccaccgctggtagcggtggtttttttgtttgcaagcagcagattacgcgcagaaaaaaaggatctcaagaagatcctttgatcttttctacggggtctgacgctcagtggaacgaaaactcacgttaagggattttggtcatgagattatcaaaaaggatcttcacctagatccttttaaattaaaaatgaagttttaaatcaatctaaagtatatatgagtaaacttggtctgacagttaccaatgcttaatcagtgaggcacctatctcagcgatctgtctatttcgttcatccatagttgcctgactccccgtcgtgtagataactacgatacgggagggcttaccatctggccccagtgctgcaatgataccgcgagacccacgctcaccggctccagatttatcagcaataaaccagccagccggaagggccgagcgcagaagtggtcctgcaactttatccgcctccatccagtctattaattgttgccgggaagctagagtaagtagttcgccagttaatagtttgcgcaacgttgttgccattgctacaggcatcgtggtgtcacgctcgtcgtttggtatggcttcattcagctccggttcccaacgatcaaggcgagttacatgatcccccatgttgtgcaaaaaagcggttagctccttcggtcctccgatcgttgtcagaagtaagttggccgcagtgttatcactcatggttatggcagcactgcataattctcttactgtcatgccatccgtaagatgcttttctgtgactggtgagtactcaaccaagtcattctgagaatagtgtatgcggcgaccgagttgctcttgcccggcgtcaatacgggataataccgcgccacatagcagaactttaaaagtgctcatcattggaaaacgttcttcggggcgaaaactctcaaggatcttaccgctgttgagatccagttcgatgtaacccactcgtgcacccaactgatcttcagcatcttttactttcaccagcgtttctgggtgagcaaaaacaggaaggcaaaatgccgcaaaaaagggaataagggcgacacggaaatgttgaatactcatactcttcctttttcaatattattgaagcatttatcagggttattgtctcatgagcggatacatatttgaatgtatttagaaaaataaacaaataggggttccgcgcacatttccccgaaaagtgccacctgacgtctaagaaaccattattatcatgacattaacctataaaaataggcgtatcacgaggccctttcgtctcgcgcgtttcggtgatgacggtgaaaacctctgacacatgcagctcccggagacggtcacagcttgtctgtaagcggatgccgggagcagacaagcccgtcagggcgcgtcagcgggtgttggcgggtgtcggggctggcttaactatgcggcatcagagcagattgtactgagagtgcaccataaaattgtaaacgttaatattttgttaaaattcgcgttaaatttttgttaaatcagctcattttttaaccaataggccgaaatcggcaaaatcccttataaatcaaaagaatagcccgagatagggttgagtgttgttccagtttggaacaagagtccactattaaagaacgtggactccaacgtcaaagggcgaaaaaccgtctatcagggcgatggcccactacgtgaaccatcacccaaatcaagttttttggggtcgaggtgccgtaaagcactaaatcggaaccctaaagggagcccccgatttagagcttgacggggaaagccggcgaacgtggcgagaaaggaagggaagaaagcgaaaggagcgggcgctagggcgctggcaagtgtagcggtcacgctgcgcgtaaccaccacacccgccgcgcttaatgcgccgctacagggcgcgtactatggttgctttgacgtatgcggtgtgaaataccgcacagatgcgtaaggagaaaataccgcatcaggcgcccctgcaggcagctgcgcgctcgctcgctcactgaggccgcccgggcaaagcccgggcgtcgggcgacctttggtcgcccggcctcagtgagcgagcgagcgcgcagagagggagtggccaactccatcactaggggttcctacgcgttctaagctagacccttcagattaaaaataactgaggtaagggcctgggtaggggaggtggtgtgagacgctcctgtctctcctctatctgcccatcggccctttggggaggaggaatgtgcccaaggactaaaaaaaggccatggagccagaggggcgagggcaacagacctttcatgggcaaaccttggggccctgctgtctagcatgccccactacgggtctaggctgcccatgtaaggaggcaaggcctggggacacccgagatgcctggttataattaacccagacatgtggctgcccccccccccccaacacctgctgcctctaaaaataaccctgtccctggtggatcccctgcatgcgaagatcttcgaacaaggctgtgggggactgagggcaggctgtaacaggcttgggggccagggcttatacgtgcctgggactcccaaagtattactgttccatgttcccggcgaagggccagctgtcccccgccagctagactcagcacttagtttaggaaccagtgagcaagtcagcccttggggcagcccatacaaggccatggggctgggcaagctgcacgcctgggtccggggtgggcacggtgcccgggcaacgagctgaaagctcatctgctctcaggggcccctccctggggacagcccctcctggctagtcacaccctgtaggctcctctatataacccaggcaggggcacaggggctgccctcattctaccaccacctccacagcacagacagacactcaggagcagccagcggcgcgcccaggtaagtttagtctttttgtcttttatttcaggtcccggatccggtgacacccaagctgtctagagccgccaccaccggtgccaccatgcagcgggtaaatatgatcatggccgagagtcccggactcatcactatatgcctcttgggttacttgcttagcgcagaatgtacagtgtttctggaccatgagaatgccaacaaaatactgaatcggcccaaaaggtacaacagtggtaagctggaagagtttgtccaagggaatctcgagcgggaatgcatggaagaaaaatgcagcttcgaagaggcaagggaggtatttgagaataccgaacgcactactgagttttggaaacaatacgttgacggagaccaatgtgagtctaatccgtgccttaatggaggttcatgtaaagacgatataaacagttacgaatgttggtgccctttcggctttgagggtaaaaactgtgagttggatgtcacctgcaacataaaaaacggacgatgtgaacaattttgcaagaactctgctgataacaaagtagtgtgttcatgtactgaagggtatcgcttggcggaaaaccaaaagagttgcgaaccagcggttccatttccttgcggcagggtctcagtttcccaaacctctaagttgacaagggccgagacggtgtttccggatgtagactatgtgaatagcacggaggcagagactatactcgacaatattacccaaagcacacagtcatttaatgatttcacccgagtggtaggaggggaagacgctaaaccaggacaattcccttggcaggtggttttgaacggcaaggtagatgctttttgtgggggctcaatcgttaacgagaaatggatagtaacggccgcgcattgtgtagaaacgggtgtgaagatcacagtggtagctggtgaacacaacatcgaagagacggagcacacagaacaaaagaggaatgttatccgcattatccctcatcataactacaatgctgctataaacaagtataatcacgacatagcacttcttgaactggacgaacctcttgtcttgaattcctatgtgacacccatctgtatcgctgataaagaatatacaaacatcttccttaaatttggtagtggttacgtatcaggctggggtcgggtcttccacaaaggcagaagtgcattggtattgcagtatcttagagtacccttggtggatagagcgacttgtcttctgagtacgaaatttaccatttacaataatatgttttgcgctggcttccatgagggtggacgggacagttgccaaggagattcaggcggacctcacgtaacggaagtggagggcacgtcattcctgacgggcattattagctggggtgaagagtgtgcaatgaagggaaagtatgggatctatacgaaggtctccaggtatgtgaattggataaaggagaagaccaagctcacgtgagtcgacaatcaacctctggattacaaaatttgtgaaagattgactggtattcttaactatgttgctccttttacgctatgtggatacgctgctttaatgcctttgtatcatgctattgcttcccgtatggctttcattttctcctccttgtataaatcctggttgctgtctctttatgaggagttgtggcccgttgtcaggcaacgtggcgtggtgtgcactgtgtttgctgacgcaacccccactggttggggcattgccaccacctgtcagctcctttccgggactttcgctttccccctccctattgccacggcggaactcatcgccgcctgccttgcccgctgctggacaggggctcggctgttgggcactgacaattccgtggtgttgtcggggaagctgacgtcctttccatggctgctcgcctgtgttgccacctggattctgcgcgggacgtccttctgctacgtcccttcggccctcaatccagcggaccttccttcccgcggcctgctgccggctctgcggcctcttccgcgtcttcgccttcgccctcagacgagtcggatctccctttgggccgcctccccgcctggtcgacgtttatttgtgaaatttgtgatgctattgctttatttgtaaccatctagctttatttgtgaaatttgtgatgctattgctttatttgtaaccattataagctgcaataaacaagttaacaacaacaattgcattcattttatgtttcaggttcagggggagatgtgggaggttttttaaagtttaaacaggaacccctagtgatggagttggccactccctctctgcgcgctcgctcgctcactgaggccgggcgaccaaaggtcgcccgacgcccgggcggcctcagtgagcgagcgagcgcgcagctgcctgcagg

SEQ ID NO: 22 - DNA, 5377 bp, synthetic construct
  source 1..5377: mol_type = other DNA
acatgtgagcaaaaggccagcaaaaggccaggaaccgtaaaaaggccgcgttgctggcgtttttccataggctccgcccccctgacgagcatcacaaaaatcgacgctcaagtcagaggtggcgaaacccgacaggactataaagataccaggcgtttccccctggaagctccctcgtgcgctctcctgttccgaccctgccgcttaccggatacctgtccgcctttctcccttcgggaagcgtggcgctttctcatagctcacgctgtaggtatctcagttcggtgtaggtcgttcgctccaagctgggctgtgtgcacgaaccccccgttcagcccgaccgctgcgccttatccggtaactatcgtcttgagtccaacccggtaagacacgacttatcgccactggcagcagccactggtaacaggattagcagagcgaggtatgtaggcggtgctacagagttcttgaagtggtggcctaactacggctacactagaaggacagtatttggtatctgcgctctgctgaagccagttaccttcggaaaaagagttggtagctcttgatccggcaaacaaaccaccgctggtagcggtggtttttttgtttgcaagcagcagattacgcgcagaaaaaaaggatctcaagaagatcctttgatcttttctacggggtctgacgctcagtggaacgaaaactcacgttaagggattttggtcatgagattatcaaaaaggatcttcacctagatccttttaaattaaaaatgaagttttaaatcaatctaaagtatatatgagtaaacttggtctgacagttaccaatgcttaatcagtgaggcacctatctcagcgatctgtctatttcgttcatccatagttgcctgactccccgtcgtgtagataactacgatacgggagggcttaccatctggccccagtgctgcaatgataccgcgagacccacgctcaccggctccagatttatcagcaataaaccagccagccggaagggccgagcgcagaagtggtcctgcaactttatccgcctccatccagtctattaattgttgccgggaagctagagtaagtagttcgccagttaatagtttgcgcaacgttgttgccattgctacaggcatcgtggtgtcacgctcgtcgtttggtatggcttcattcagctccggttcccaacgatcaaggcgagttacatgatcccccatgttgtgcaaaaaagcggttagctccttcggtcctccgatcgttgtcagaagtaagttggccgcagtgttatcactcatggttatggcagcactgcataattctcttactgtcatgccatccgtaagatgcttttctgtgactggtgagtactcaaccaagtcattctgagaatagtgtatgcggcgaccgagttgctcttgcccggcgtcaatacgggataataccgcgccacatagcagaactttaaaagtgctcatcattggaaaacgttcttcggggcgaaaactctcaaggatcttaccgctgttgagatccagttcgatgtaacccactcgtgcacccaactgatcttcagcatcttttactttcaccagcgtttctgggtgagcaaaaacaggaaggcaaaatgccgcaaaaaagggaataagggcgacacggaaatgttgaatactcatactcttcctttttcaatattattgaagcatttatcagggttattgtctcatgagcggatacatatttgaatgtatttagaaaaataaacaaataggggttccgcgcacatttccccgaaaagtgccacctgacgtctaagaaaccattattatcatgacattaacctataaaaataggcgtatcacgaggccctttcgtctcgcgcgtttcggtgatgacggtgaaaacctctgacacatgcagctcccggagacggtcacagcttgtctgtaagcggatgccgggagcagacaagcccgtcagggcgcgtcagcgggtgttggcgggtgtcggggctggcttaactatgcggcatcagagcagattgtactgagagtgcaccataaaattgtaaacgttaatattttgttaaaattcgcgttaaatttttgttaaatcagctcattttttaaccaataggccgaaatcggcaaaatcccttataaatcaaaagaatagcccgagatagggttgagtgttgttccagtttggaacaagagtccactattaaagaacgtggactccaacgtcaaagggcgaaaaaccgtctatcagggcgatggcccactacgtgaaccatcacccaaatcaagttttttggggtcgaggtgccgtaaagcactaaatcggaaccctaaagggagcccccgatttagagcttgacggggaaagccggcgaacgtggcgagaaaggaagggaagaaagcgaaaggagcgggcgctagggcgctggcaagtgtagcggtcacgctgcgcgtaaccaccacacccgccgcgcttaatgcgccgctacagggcgcgtactatggttgctttgacgtatgcggtgtgaaataccgcacagatgcgtaaggagaaaataccgcatcaggcgcccctgcaggcagctgcgcgctcgctcgctcactgaggccgcccgggcgtcgggcgacctttggtcgcccggcctcagtgagcgagcgagcgcgcagagagggagtggccaactccatcactaggggttcctacgcgtccattgacgtcaataatgacgtatgttcccatagtaacgccaatagggactttccattgacgtcaatgggtggagtatttacggtaaactgcccacttggcagtacatcaagtgtatcatatgccaagtacgccccctattgacgtcaatgacggtaaatggcccgcctggcattatgcccagtacatgaccttatgggactttcctacttggcagtacatctacgtattagtcatcgctattaccatggtcgaggtgagccccacgttctgcttcactctccccatctcccccccctccccacccccaattttgtatttatttattttttaattattttgtgcagcgatgggggcggggggggggggggggcgcgcgccaggcggggcggggcggggcgaggggcggggcggggcgaggcggagaggtgcggcggcagccaatcagagcggcgcgctccgaaagtttccttttatggcgaggcggcggcggcggcggccctataaaaagcgaagcgcgcggcgggcgggagtcgctgcgcgctgccttcgccccgtgccccgctccgccgccgcctcgcgccgcccgccccggctctgactgaccgcgttactcccacaggtgagcgggcgggacggcccttctcctccgggctgtaattagcgcttggtttaatgacggcttgtttcttttctgtggctgcgtgaaagccttgaggggctccgggagggccctttgtgcggggggagcggctcggggctgtccgcggggggacggctgccttcgggggggacggggcagggcggggttcggcttctggcgtgtgaccggcggctctagagcctctgctaaccatgttcatgccttcttctttttcctacagctcctgggcaacgtctcctgggcaacgtaccggtgccaccatgcagcgggtaaatatgatcatggccgagagtcccggactcatcactatatgcctcttgggttacttgcttagcgcagaatgtacagtgtttctggaccatgagaatgccaacaaaatactgaatcggcccaaaaggtacaacagtggtaagctggaagagtttgtccaagggaatctcgagcgggaatgcatggaagaaaaatgcagcttcgaagaggcaagggaggtatttgagaataccgaacgcactactgagttttggaaacaatacgttgacggagaccaatgtgagtctaatccgtgccttaatggaggttcatgtaaagacgatataaacagttacgaatgttggtgccctttcggctttgagggtaaaaactgtgagttggatgtcacctgcaacataaaaaacggacgatgtgaacaattttgcaagaactctgctgataacaaagtagtgtgttcatgtactgaagggtatcgcttggcggaaaaccaaaagagttgcgaaccagcggttccatttccttgcggcagggtctcagtttcccaaacctctaagttgacaagggccgagacggtgtttccggatgtagactatgtgaatagcacggaggcagagactatactcgacaatattacccaaagcacacagtcatttaatgatttcacccgagtggtaggaggggaagacgctaaaccaggacaattcccttggcaggtggttttgaacggcaaggtagatgctttttgtgggggctcaatcgttaacgagaaatggatagtaacggccgcgcattgtgtagaaacgggtgtgaagatcacagtggtagctggtgaacacaacatcgaagagacggagcacacagaacaaaagaggaatgttatccgcattatccctcatcataactacaatgctgctataaacaagtataatcacgacatagcacttcttgaactggacgaacctcttgtcttgaattcctatgtgacacccatctgtatcgctgataaagaatatacaaacatcttccttaaatttggtagtggttacgtatcaggctggggtcgggtcttccacaaaggcagaagtgcattggtattgcagtatcttagagtacccttggtggatagagcgacttgtcttctgagtacgaaatttaccatttacaataatatgttttgcgctggcttccatgagggtggacgggacagttgccaaggagattcaggcggacctcacgtaacggaagtggagggcacgtcattcctgacgggcattattagctggggtgaagagtgtgcaatgaagggaaagtatgggatctatacgaaggtctccaggtatgtgaattggataaaggagaagaccaagctcacgtgagtcgacgtttatttgtgaaatttgtgatgctattgctttatttgtaaccatctagctttatttgtgaaatttgtgatgctattgctttatttgtaaccattataagctgcaataaacaagttaacaacaacaattgcattcattttatgtttcaggttcagggggagatgtgggaggttttttaaagtttaaacaggaacccctagtgatggagttggccactccctctctgcgcgctcgctcgctcactgaggccgggcgaccaaaggtcgcccgacgcccgggctttgcccgggcggcctcagtgagcgagcgagcgcgcagctgcctgcagg

SEQ ID NO: 23 - DNA, 1386 bp, synthetic construct
  source 1..1386: mol_type = other DNA
atgcagcgggtaaatatgatcatggccgagagtcccggactcatcactatatgcctcttgggttacttgcttagcgcagaatgtacagtgtttctggaccatgagaatgccaacaaaatactgaatcggcccaaaaggtacaacagtggtaagctggaagagtttgtccaagggaatctcgagcgggaatgcatggaagaaaaatgcagcttcgaagaggcaagggaggtatttgagaataccgaacgcactactgagttttggaaacaatacgttgacggagaccaatgtgagtctaatccgtgccttaatggaggttcatgtaaagacgatataaacagttacgaatgttggtgccctttcggctttgagggtaaaaactgtgagttggatgtcacctgcaacataaaaaacggacgatgtgaacaattttgcaagaactctgctgataacaaagtagtgtgttcatgtactgaagggtatcgcttggcggaaaaccaaaagagttgcgaaccagcggttccatttccttgcggcagggtctcagtttcccaaacctctaagttgacaagggccgagacggtgtttccggatgtagactatgtgaatagcacggaggcagagactatactcgacaatattacccaaagcacacagtcatttaatgatttcacccgagtggtaggaggggaagacgctaaaccaggacaattcccttggcaggtggttttgaacggcaaggtagatgctttttgtgggggctcaatcgttaacgagaaatggatagtaacggccgcgcattgtgtagaaacgggtgtgaagatcacagtggtagctggtgaacacaacatcgaagagacggagcacacagaacaaaagaggaatgttatccgcattatccctcatcataactacaatgctgctataaacaagtataatcacgacatagcacttcttgaactggacgaacctcttgtcttgaattcctatgtgacacccatctgtatcgctgataaagaatatacaaacatcttccttaaatttggtagtggttacgtatcaggctggggtcgggtcttccacaaaggcagaagtgcattggtattgcagtatcttagagtacccttggtggatagagcgacttgtcttctgagtacgaaatttaccatttacaataatatgttttgcgctggcttccatgagggtggacgggacagttgccaaggagattcaggcggacctcacgtaacggaagtggagggcacgtcattcctgacgggcattattagctggggtgaagagtgtgcaatgaagggaaagtatgggatctatacgaaggtctccaggtatgtgaattggataaaggagaagaccaagctcacgtag

SEQ ID NO: 24 - protein, 461 aa, synthetic construct
MQRVNMIMAESPGLITICLLGYLLSAECTVFLDHENANKILNRPKRYNSGKLEEFVQGNLERECMEEKCSFEEAREVFENTERTTEFWKQYVDGDQCESNPCLNGGSCKDDINSYECWCPFGFEGKNCELDVTCNIKNGRCEQFCKNSADNKVVCSCTEGYRLAENQKSCEPAVPFPCGRVSVSQTSKLTRAETVFPDVDYVNSTEAETILDNITQSTQSFNDFTRVVGGEDAKPGQFPWQVVLNGKVDAFCGGSIVNEKWIVTAAHCVETGVKITVVAGEHNIEETEHTEQKRNVIRIIPHHNYNAAINKYNHDIALLELDEPLVLNSYVTPICIADKEYTNIFLKFGSGYVSGWGRVFHKGRSALVLQYLRVPLVDRATCLLSTKFTIYNNMFCAGFHEGGRDSCQGDSGGPHVTEVEGTSFLTGIISWGEECAMKGKYGIYTKVSRYVNWIKEKTKLT

SEQ ID NO: 25 - DNA, 7409 bp, synthetic construct
  source 1..7409: mol_type = other DNA
gctgcgcaactgttgggaagggcgatcggtgcgggcctcttcgctattacgccagctggcgaaagggggatgtgctgcaaggcgattaagttgggtaacgccagggttttcccagtcacgacgttgtaaaacgacggccagtgagcgcgcgtaatacgactcactatagggcgaattgggtaccgggccccccctcgaggtcgacggtatcgggggagctcgcagggtctccattttgaagcgggaggtttgaacgcgcagccgccatgccggggttttacgagattgtgattaaggtccccagcgaccttgacgagcatctgcccggcatttctgacagctttgtgaactgggtggccgagaaggaatgggagttgccgccagattctgacatggatctgaatctgattgagcaggcacccctgaccgtggccgagaagctgcagcgcgactttctgacggaatggcgccgtgtgagtaaggccccggaggctcttttctttgtgcaatttgagaagggagagagctacttccacatgcacgtgctcgtggaaaccaccggggtgaaatccatggttttgggacgtttcctgagtcagattcgcgaaaaactgattcagagaatttaccgcgggatcgagccgactttgccaaactggttcgcggtcacaaagaccagaaatggcgccggaggcgggaacaaggtggtggatgagtgctacatccccaattacttgctccccaaaacccagcctgagctccagtgggcgtggactaatatggaacagtatttaagcgcctgtttgaatctcacggagcgtaaacggttggtggcgcagcatctgacgcacgtgtcgcagacgcaggagcagaacaaagagaatcagaatcccaattctgatgcgccggtgatcagatcaaaaacttcagccaggtacatggagctggtcgggtggctcgtggacaaggggattacctcggagaagcagtggatccaggaggaccaggcctcatacatctccttcaatgcggcctccaactcgcggtcccaaatcaaggctgccttggacaatgcgggaaagattatgagcctgactaaaaccgcccccgactacctggtgggccagcagcccgtggaggacatttccagcaatcggatttataaaattttggaactaaacgggtacgatccccaatatgcggcttccgtctttctgggatgggccacgaaaaagttcggcaagaggaacaccatctggctgtttgggcctgcaactaccgggaagaccaacatcgcggaggccatagcccacactgtgcccttctacgggtgcgtaaactggaccaatgagaactttcccttcaacgactgtgtcgacaagatggtgatctggtgggaggaggggaagatgaccgccaaggtcgtggagtcggccaaagccattctcggaggaagcaaggtgcgcgtggaccagaaatgcaagtcctcggcccagatagacccgactcccgtgatcgtcacctccaacaccaacatgtgcgccgtgattgacgggaactcaacgaccttcgaacaccagcagccgttgcaagaccggatgttcaaatttgaactcacccgccgtctggatcatgactttgggaaggtcaccaagcaggaagtcaaagactttttccggtgggcaaaggatcacgtggttgaggtggagcatgaattctacgtcaaaaagggtggagccaagaaaagacccgcccccagtgacgcagatataagtgagcccaaacgggtgcgcgagtcagttgcgcagccatcgacgtcagacgcggaagcttcgatcaactacgcagacaggtaccaaaacaaatgttctcgtcacgtgggcatgaatctgatgctgtttccctgcagacaatgcgagagaatgaatcagaattcaaatatctgcttcactcacggacagaaagactgtttagagtgctttcccgtgtcagaatctcaacccgtttctgtcgtcaaaaaggcgtatcagaaactgtgctacattcatcatatcatgggaaaggtgccagacgcttgcactgcctgcgatctggtcaatgtggatttggatgactgcatctttgaacaataaatgatttaaatcaggtatggctgccgatggttatcttccagattggctcgaggacaacctctctgagggcattcgcgagtggtgggacttgaaacctggagccccgaagcccaaagccaaccagcaaaagcaggacgacggccggggtctggtgcttcctggctacaagtacctcggacccttcaacggactcgacaagggggagcccgtcaacgcggcggacgcagcggccctcgagcacgacaaggcctacgaccagcagctcaaagcgggtgacaatccgtacctgcggtataaccacgccgacgccgagtttcaggagcgtctgcaagaagatacgtcttttgggggcaacctcgggcgagcagtcttccaggccaagaagcgggttctcgaacctctcggtctggttgaggaaggcgctaagacggctcctggaaagaaacgtccggtagagcagtcgccacaagagccagactcctcctcgggcatcggcaagacaggccagcagcccgctaaaaagagactcaattttggtcagactggcgactcagagtcagtccccgatccacaacctctcggagaacctccagcaacccccgctgctgtgggacctactacaatggcttcaggcggtggcgcaccaatggcagacaataacgaaggcgccgacggagtgggtaatgcctcaggaaattggcattgcgattccacatggctgggcgacagagtcatcaccaccagcacccgcacctgggccttgcccacctacaataaccacctctacaagcaaatctccagtgcttcaacgggggccagcaacgacaaccactacttcggctacagcaccccctgggggtattttgatttcaacagattccactgccacttttcaccacgtgactggcagcgactcatcaacaacaattggggattccggcccaagagactcaacttcaaactcttcaacatccaagtcaaggaggtcacgacgaatgatggcgtcacaaccatcgctaataaccttaccagcacggttcaagtcttctcggactcggagtaccagcttccgtacgtcctcggctctgcgcaccagggctgcctccctccgttcccggcggacgtgttcatgattccgcaatacggctacctgacgctcaacaatggcagccaagccgtgggacgttcatccttttactgcctggaatatttcccttctcagatgctgagaacgggcaacaactttaccttcagctacacctttgaggaagtgcctttccacagcagctacgcgcacagccagagcctggaccggctgatgaatcctctcatcgaccaatacctgtattacctgaacagaactcaaaatcagtccggaagtgcccaaaacaaggacttgctgtttagccgtgggtctccagctggcatgtctgttcagcccaaaaactggctacctggaccctgttatcggcagcagcgcgtttctaaaacaaaaacagacaacaacaacagcaattttacctggactggtgcttcaaaatataacctcaatgggcgtgaatccatcatcaaccctggcactgctatggcctcacacaaagacgacgaagacaagttctttcccatgagcggtgtcatgatttttggaaaagagagcgccggagcttcaaacactgcattggacaatgtcatgattacagacgaagaggaaattaaagccactaaccctgtggccaccgaaagatttgggaccgtggcagtcaatttccagagcagcagcacagaccctgcgaccggagatgtgcatgctatgggagcattacctggcatggtgtggcaagatagagacgtgtacctgcagggtcccatttgggccaaaattcctcacacagatggacactttcacccgtctcctcttatgggcggctttggactcaagaacccgcctcctcagatcctcatcaaaaacacgcctgttcctgcgaatcctccggcggagttttcagctacaaagtttgcttcattcatcacccaatactccacaggacaagtgagtgtggaaattgaatgggagctgcagaaagaaaacagcaagcgctggaatcccgaagtgcagtacacatccaattatgcaaaatctgccaacgttgattttactgtggacaacaatggactttatactgagcctcgccccattggcacccgttaccttacccgtcccctgtaattacgtgttaatcaataaaccggttgattcgtttcagttgaactttggtctcctgtccttcttatcttatcggttaccatggttatagcttacacattaactgcttggttgcgcttcgcgataaaagacttacgtcatcgggttacccctagggggatccactagttctagaggtcctgtattagaggtcacgtgagtgttttgcgacattttgcgacaccatgtggtcacgctgggtatttaagcccgagtgagcacgcagggtctccattttgaagcgggaggtttgaacgcgcagccgccaagccgaattctgcagatatccatcacactggcggccgctcgactagagcggccgccaccgcggtggagctccagcttttgttccctttagtgagggttaattgcgcgcttggcgtaatcatggtcatagctgtttcctgtgtgaaattgttatccgctcacaattccacacaacatacgagccggaagcataaagtgtaaagcctggggtgcctaatgagtgagctaactcacattaattgcgttgcgctcactgcccgctttccagtcgggaaacctgtcgtgccagctgcattaatgaatcggccaacgcgcggggagaggcggtttgcgtattgggcgctcttccgcttcctcgctcactgactcgctgcgctcggtcgttcggctgcggcgagcggtatcagctcactcaaaggcggtaatacggttatccacagaatcaggggataacgcaggaaagaacatgtgagcaaaaggccagcaaaaggccaggaaccgtaaaaaggccgcgttgctggcgtttttccataggctccgcccccctgacgagcatcacaaaaatcgacgctcaagtcagaggtggcgaaacccgacaggactataaagataccaggcgtttccccctggaagctccctcgtgcgctctcctgttccgaccctgccgcttaccggatacctgtccgcctttctcccttcgggaagcgtggcgctttctcatagctcacgctgtaggtatctcagttcggtgtaggtcgttcgctccaagctgggctgtgtgcacgaaccccccgttcagcccgaccgctgcgccttatccggtaactatcgtcttgagtccaacccggtaagacacgacttatcgccactggcagcagccactggtaacaggattagcagagcgaggtatgtaggcggtgctacagagttcttgaagtggtggcctaactacggctacactagaagaacagtatttggtatctgcgctctgctgaagccagttaccttcggaaaaagagttggtagctcttgatccggcaaacaaaccaccgctggtagcggtggtttttttgtttgcaagcagcagattacgcgcagaaaaaaaggatctcaagaagatcctttgatcttttctacggggtctgacgctcagtggaacgaaaactcacgttaagggattttggtcatgagattatcaaaaaggatcttcacctagatccttttaaattaaaaatgaagttttaaatcaatctaaagtatatatgagtaaacttggtctgacagttaccaatgcttaatcagtgaggcacctatctcagcgatctgtctatttcgttcatccatagttgcctgactccccgtcgtgtagataactacgatacgggagggcttaccatctggccccagtgctgcaatgataccgcgagacccacgctcaccggctccagatttatcagcaataaaccagccagccggaagggccgagcgcagaagtggtcctgcaactttatccgcctccatccagtctattaattgttgccgggaagctagagtaagtagttcgccagttaatagtttgcgcaacgttgttgccattgctacaggcatcgtggtgtcacgctcgtcgtttggtatggcttcattcagctccggttcccaacgatcaaggcgagttacatgatcccccatgttgtgcaaaaaagcggttagctccttcggtcctccgatcgttgtcagaagtaagttggccgcagtgttatcactcatggttatggcagcactgcataattctcttactgtcatgccatccgtaagatgcttttctgtgactggtgagtactcaaccaagtcattctgagaatagtgtatgcggcgaccgagttgctcttgcccggcgtcaatacgggataataccgcgccacatagcagaactttaaaagtgctcatcattggaaaacgttcttcggggcgaaaactctcaaggatcttaccgctgttgagatccagttcgatgtaacccactcgtgcacccaactgatcttcagcatcttttactttcaccagcgtttctgggtgagcaaaaacaggaaggcaaaatgccgcaaaaaagggaataagggcgacacggaaatgttgaatactcatactcttcctttttcaatattattgaagcatttatcagggttattgtctcatgagcggatacatatttgaatgtatttagaaaaataaacaaataggggttccgcgcacatttccccgaaaagtgccacctaaattgtaagcgttaatattttgttaaaattcgcgttaaatttttgttaaatcagctcattttttaaccaataggccgaaatcggcaaaatcccttataaatcaaaagaatagaccgagatagggttgagtgttgttccagtttggaacaagagtccactattaaagaacgtggactccaacgtcaaagggcgaaaaaccgtctatcagggcgatggcccactacgtgaaccatcaccctaatcaagttttttggggtcgaggtgccgtaaagcactaaatcggaaccctaaagggagcccccgatttagagcttgacggggaaagccggcgaacgtggcgagaaaggaagggaagaaagcgaaaggagcgggcgctagggcgctggcaagtgtagcggtcacgctgcgcgtaaccaccacacccgccgcgcttaatgcgccgctacagggcgcgtcccattcgccattcag

SEQ ID NO: 26 - DNA, 7327 bp, synthetic construct
  source 1..7327: mol_type = other DNA
atgccggggttttacgagattgtgattaaggtccccagcgaccttgacgagcatctgcccggcatttctgacagctttgtgaactgggtggccgagaaggaatgggagttgccgccagattctgacatggatctgaatctgattgagcaggcacccctgaccgtggccgagaagctgcagcgcgactttctgacggaatggcgccgtgtgagtaaggccccggaggctcttttctttgtgcaatttgagaagggagagagctacttccacatgcacgtgctcgtggaaaccaccggggtgaaatccatggttttgggacgtttcctgagtcagattcgcgaaaaactgattcagagaatttaccgcgggatcgagccgactttgccaaactggttcgcggtcacaaagaccagaaatggcgccggaggcgggaacaaggtggtggatgagtgctacatccccaattacttgctccccaaaacccagcctgagctccagtgggcgtggactaatatggaacagtatttaagcgcctgtttgaatctcacggagcgtaaacggttggtggcgcagcatctgacgcacgtgtcgcagacgcaggagcagaacaaagagaatcagaatcccaattctgatgcgccggtgatcagatcaaaaacttcagccaggtacatggagctggtcgggtggctcgtggacaaggggattacctcggagaagcagtggatccaggaggaccaggcctcatacatctccttcaatgcggcctccaactcgcggtcccaaatcaaggctgccttggacaatgcgggaaagattatgagcctgactaaaaccgcccccgactacctggtgggccagcagcccgtggaggacatttccagcaatcggatttataaaattttggaactaaacgggtacgatccccaatatgcggcttccgtctttctgggatgggccacgaaaaagttcggcaagaggaacaccatctggctgtttgggcctgcaactaccgggaagaccaacatcgcggaggccatagcccacactgtgcccttctacgggtgcgtaaactggaccaatgagaactttcccttcaacgactgtgtcgacaagatggtgatctggtgggaggaggggaagatgaccgccaaggtcgtggagtcggccaaagccattctcggaggaagcaaggtgcgcgtggaccagaaatgcaagtcctcggcccagatagacccgactcccgtgatcgtcacctccaacaccaacatgtgcgccgtgattgacgggaactcaacgaccttcgaacaccagcagccgttgcaagaccggatgttcaaatttgaactcacccgccgtctggatcatgactttgggaaggtcaccaagcaggaagtcaaagactttttccggtgggcaaaggatcacgtggttgaggtggagcatgaattctacgtcaaaaagggtggagccaagaaaagacccgcccccagtgacgcagatataagtgagcccaaacgggtgcgcgagtcagttgcgcagccatcgacgtcagacgcggaagcttcgatcaactacgcagacaggtaccaaaacaaatgttctcgtcacgtgggcatgaatctgatgctgtttccctgcagacaatgcgagagaatgaatcagaattcaaatatctgcttcactcacggacagaaagactgtttagagtgctttcccgtgtcagaatctcaacccgtttctgtcgtcaaaaaggcgtatcagaaactgtgctacattcatcatatcatgggaaaggtgccagacgcttgcactgcctgcgatctggtcaatgtggatttggatgactgcatctttgaacaataaatgatttaaatcaggtatggctgccgatggttatcttccagattggctcgaggacactctctctgaaggaataagacagtggtggaagctcaaacctggcccaccaccaccaaagcccgcagagcggcataaggacgacagcaggggtcttgtgcttcctgggtacaagtacctcggacccttcaacggactcgacaagggagagccggtcaacgaggcagacgccgcggccctcgagcacgacaaagcctacgaccggcagctcgacagcggagacaacccgtacctcaagtacaaccacgccgacgcggagtttcaggagcgccttaaagaagatacgtcttttgggggcaacctcggacgagcagtcttccaggcgaaaaagagggttcttgaacctctgggcctggttgaggaacctgttaagacggctccgggaaaaaagaggccggtagagcactctcctgtggagccagactcctcctcgggaaccggaaaggcgggccagcagcctgcaagaaaaagattgaattttggtcagactggagacgcagactcagtacctgacccccagcctctcggacagccaccagcagccccctctggtctgggaactaatacgatggctacaggcagtggcgcaccaatggcagacaataacgagggcgccgacggagtgggtaattcctcgggaaattggcattgcgattccacatggatgggcgacagagtcatcaccaccagcacccgaacctgggccctgcccacctacaacaaccacctctacaaacaaatttccagccaatcaggagcctcgaacgacaatcactactttggctacagcaccccttgggggtattttgacttcaacagattccactgccacttttcaccacgtgactggcaaagactcatcaacaacaactggggattccgacccaagagactcaacttcaagctctttaacattcaagtcaaagaggtcacgcagaatgacggtacgacgacgattgccaataaccttaccagcacggttcaggtgtttactgactcggagtaccagctcccgtacgtcctcggctcggcgcatcaaggatgcctcccgccgttcccagcagacgtcttcatggtgccacagtatggatacctcaccctgaacaacgggagtcaggcagtaggacgctcttcattttactgcctggagtactttccttctcagatgctgcgtaccggaaacaactttaccttcagctacacttttgaggacgttcctttccacagcagctacgctcacagccagagtctggaccgtctcatgaatcctctcatcgaccagtacctgtattacttgagcagaacaaacactccaagtggaaccaccacgcagtcaaggcttcagttttctcaggccggagcgagtgacattcgggaccagtctaggaactggcttcctggaccctgttaccgccagcagcgagtatcaaagacatctgcggataacaacaacagtgaatactcgtggactggagctaccaagtaccacctcaatggcagagactctctggtgaatccgggcccggccatggcaagccacaaggacgatgaagaaaagttttttcctcagagcggggttctcatctttgggaagcaaggctcagagaaaacaaatgtggacattgaaaaggtcatgattacagacgaagaggaaatcaggacaaccaatcccgtggctacggagcagtatggttctgtatctaccaacctccagagaggcaacagacaagcagctaccgcagatgtcaacacacaaggcgttcttccaggcatggtctggcaggacagagatgtgtaccttcaggggcccatctgggcaaagattccacacacggacggacattttcacccctctcccctcatgggtggattcggacttaaacaccctcctccacagattctcatcaagaacaccccggtacctgcgaatccttcgaccaccttcagtgcggcaaagtttgcttccttcatcacacagtactccacgggacaggtcagcgtggagatcgagtgggagctgcagaaggaaaacagcaaacgctggaatcccgaaattcagtacacttccaactacaacaagtctgttaatgtggactttactgtggacactaatggcgtgtattcagagcctcgccccattggcaccagatacctgactcgtaatctgtaattgcctgttaatcaataaaccggttgattcgtttcagttgaactttggtctctgcgaagggcgaattcgtttaaacctgcaggactagaggtcctgtattagaggtcacgtgagtgttttgcgacattttgcgacaccatgtggtcacgctgggtatttaagcccgagtgagcacgcagggtctccattttgaagcgggaggtttgaacgcgcagccgccaagccgaattctgcagatatccatcacactggcggccgctcgactagagcggccgccaccgcggtggagctccagcttttgttccctttagtgagggttaattgcgcgcttggcgtaatcatggtcatagctgtttcctgtgtgaaattgttatccgctcacaattccacacaacatacgagccggaagcataaagtgtaaagcctggggtgcctaatgagtgagctaactcacattaattgcgttgcgctcactgcccgctttccagtcgggaaacctgtcgtgccagctgcattaatgaatcggccaacgcgcggggagaggcggtttgcgtattgggcgctcttccgcttcctcgctcactgactcgctgcgctcggtcgttcggctgcggcgagcggtatcagctcactcaaaggcggtaatacggttatccacagaatcaggggataacgcaggaaagaacatgtgagcaaaaggccagcaaaaggccaggaaccgtaaaaaggccgcgttgctggcgtttttccataggctccgcccccctgacgagcatcacaaaaatcgacgctcaagtcagaggtggcgaaacccgacaggactataaagataccaggcgtttccccctggaagctccctcgtgcgctctcctgttccgaccctgccgcttaccggatacctgtccgcctttctcccttcgggaagcgtggcgctttctcatagctcacgctgtaggtatctcagttcggtgtaggtcgttcgctccaagctgggctgtgtgcacgaaccccccgttcagcccgaccgctgcgccttatccggtaactatcgtcttgagtccaacccggtaagacacgacttatcgccactggcagcagccactggtaacaggattagcagagcgaggtatgtaggcggtgctacagagttcttgaagtggtggcctaactacggctacactagaagaacagtatttggtatctgcgctctgctgaagccagttaccttcggaaaaagagttggtagctcttgatccggcaaacaaaccaccgctggtagcggtggtttttttgtttgcaagcagcagattacgcgcagaaaaaaaggatctcaagaagatcctttgatcttttctacggggtctgacgctcagtggaacgaaaactcacgttaagggattttggtcatgagattatcaaaaaggatcttcacctagatccttttaaattaaaaatgaagttttaaatcaatctaaagtatatatgagtaaacttggtctgacagttaccaatgcttaatcagtgaggcacctatctcagcgatctgtctatttcgttcatccatagttgcctgactccccgtcgtgtagataactacgatacgggagggcttaccatctggccccagtgctgcaatgataccgcgagacccacgctcaccggctccagatttatcagcaataaaccagccagccggaagggccgagcgcagaagtggtcctgcaactttatccgcctccatccagtctattaattgttgccgggaagctagagtaagtagttcgccagttaatagtttgcgcaacgttgttgccattgctacaggcatcgtggtgtcacgctcgtcgtttggtatggcttcattcagctccggttcccaacgatcaaggcgagttacatgatcccccatgttgtgcaaaaaagcggttagctccttcggtcctccgatcgttgtcagaagtaagttggccgcagtgttatcactcatggttatggcagcactgcataattctcttactgtcatgccatccgtaagatgcttttctgtgactggtgagtactcaaccaagtcattctgagaatagtgtatgcggcgaccgagttgctcttgcccggcgtcaatacgggataataccgcgccacatagcagaactttaaaagtgctcatcattggaaaacgttcttcggggcgaaaactctcaaggatcttaccgctgttgagatccagttcgatgtaacccactcgtgcacccaactgatcttcagcatcttttactttcaccagcgtttctgggtgagcaaaaacaggaaggcaaaatgccgcaaaaaagggaataagggcgacacggaaatgttgaatactcatactcttcctttttcaatattattgaagcatttatcagggttattgtctcatgagcggatacatatttgaatgtatttagaaaaataaacaaataggggttccgcgcacatttccccgaaaagtgccacctaaattgtaagcgttaatattttgttaaaattcgcgttaaatttttgttaaatcagctcattttttaaccaataggccgaaatcggcaaaatcccttataaatcaaaagaatagaccgagatagggttgagtgttgttccagtttggaacaagagtccactattaaagaacgtggactccaacgtcaaagggcgaaaaaccgtctatcagggcgatggcccactacgtgaaccatcaccctaatcaagttttttggggtcgaggtgccgtaaagcactaaatcggaaccctaaagggagcccccgatttagagcttgacggggaaagccggcgaacgtggcgagaaaggaagggaagaaagcgaaaggagcgggcgctagggcgctggcaagtgtagcggtcacgctgcgcgtaaccaccacacccgccgcgcttaatgcgccgctacagggcgcgtcccattcgccattcaggctgcgcaactgttgggaagggcgatcggtgcgggcctcttcgctattacgccagctggcgaaagggggatgtgctgcaaggcgattaagttgggtaacgccagggttttcccagtcacgacgttgtaaaacgacggccagtgagcgcgcgtaatacgactcactatagggcgaattgggtaccgggccccccctcgatcgaggtcgacggtatcgggggagctcgcagggtctccattttgaagcgggaggtttgaacgcgcagccgcc

SEQ ID NO: 27 - DNA, 7330 bp, synthetic construct
  source 1..7330: mol_type = other DNA
atgccggggttttacgagattgtgattaaggtccccagcgaccttgacgagcatctgcccggcatttctgacagctttgtgaactgggtggccgagaaggaatgggagttgccgccagattctgacatggatctgaatctgattgagcaggcacccctgaccgtggccgagaagctgcagcgcgactttctgacggaatggcgccgtgtgagtaaggccccggaggctcttttctttgtgcaatttgagaagggagagagctacttccacatgcacgtgctcgtggaaaccaccggggtgaaatccatggttttgggacgtttcctgagtcagattcgcgaaaaactgattcagagaatttaccgcgggatcgagccgactttgccaaactggttcgcggtcacaaagaccagaaatggcgccggaggcgggaacaaggtggtggatgagtgctacatccccaattacttgctccccaaaacccagcctgagctccagtgggcgtggactaatatggaacagtatttaagcgcctgtttgaatctcacggagcgtaaacggttggtggcgcagcatctgacgcacgtgtcgcagacgcaggagcagaacaaagagaatcagaatcccaattctgatgcgccggtgatcagatcaaaaacttcagccaggtacatggagctggtcgggtggctcgtggacaaggggattacctcggagaagcagtggatccaggaggaccaggcctcatacatctccttcaatgcggcctccaactcgcggtcccaaatcaaggctgccttggacaatgcgggaaagattatgagcctgactaaaaccgcccccgactacctggtgggccagcagcccgtggaggacatttccagcaatcggatttataaaattttggaactaaacgggtacgatccccaatatgcggcttccgtctttctgggatgggccacgaaaaagttcggcaagaggaacaccatctggctgtttgggcctgcaactaccgggaagaccaacatcgcggaggccatagcccacactgtgcccttctacgggtgcgtaaactggaccaatgagaactttcccttcaacgactgtgtcgacaagatggtgatctggtgggaggaggggaagatgaccgccaaggtcgtggagtcggccaaagccattctcggaggaagcaaggtgcgcgtggaccagaaatgcaagtcctcggcccagatagacccgactcccgtgatcgtcacctccaacaccaacatgtgcgccgtgattgacgggaactcaacgaccttcgaacaccagcagccgttgcaagaccggatgttcaaatttgaactcacccgccgtctggatcatgactttgggaaggtcaccaagcaggaagtcaaagactttttccggtgggcaaaggatcacgtggttgaggtggagcatgaattctacgtcaaaaagggtggagccaagaaaagacccgcccccagtgacgcagatataagtgagcccaaacgggtgcgcgagtcagttgcgcagccatcgacgtcagacgcggaagcttcgatcaactacgcagacaggtaccaaaacaaatgttctcgtcacgtgggcatgaatctgatgctgtttccctgcagacaatgcgagagaatgaatcagaattcaaatatctgcttcactcacggacagaaagactgtttagagtgctttcccgtgtcagaatctcaacccgtttctgtcgtcaaaaaggcgtatcagaaactgtgctacattcatcatatcatgggaaaggtgccagacgcttgcactgcctgcgatctggtcaatgtggatttggatgactgcatctttgaacaataaatgatttaaatcaggtatggctgccgatggttatcttccagattggctcgaggacaacctctctgagggcattcgcgagtggtgggacttgaaacctggagccccgaaacccaaagccaaccagcaaaagcaggacgacggccggggtctggtgcttcctggctacaagtacctcggacccttcaacggactcgacaagggggagcccgtcaacgcggcggatgcagcggccctcgagcacgacaaggcctacgaccagcagctcaaagcgggtgacaatccgtacctgcggtataaccacgccgacgccgagtttcaggagcgtctgcaagaagatacgtcttttgggggcaacctcgggcgagcagtcttccaggccaagaagagggttctcgaaccttttggtctggttgaggaaggtgctaagacggctcctggaaagaaacgtccggtagagcagtcgccacaagagccagactcctcctcgggcattggcaagacaggccagcagcccgctaaaaagagactcaattttggtcagactggcgactcagagtcagtccccgacccacaacctctcggagaacctccagcaacccccgctgctgtgggacctactacaatggcttcaggcggtggcgcaccaatggcagacaataacgaaggcgccgacggagtgggtaatgcctcaggaaattggcattgcgattccacatggctgggcgacagagtcatcaccaccagcacccgaacatgggccttgcccacctataacaaccacctctacaagcaaatctccagtgcttcaacgggggccagcaacgacaaccactacttcggctacagcaccccctgggggtattttgatttcaacagattccactgccatttctcaccacgtgactggcagcgactcatcaacaacaattggggattccggcccaagagactcaacttcaagctcttcaacatccaagtcaaggaggtcacgacgaatgatggcgtcacgaccatcgctaataaccttaccagcacggttcaagtcttctcggactcggagtaccagttgccgtacgtcctcggctctgcgcaccagggctgcctccctccgttcccggcggacgtgttcatgattccgcagtacggctacctaacgctcaacaatggcagccaggcagtgggacggtcatccttttactgcctggaatatttcccatcgcagatgctgagaacgggcaataactttaccttcagctacaccttcgaggacgtgcctttccacagcagctacgcgcacagccagagcctggaccggctgatgaatcctctcatcgaccagtacctgtattacctgaacagaactcagaatcagtccggaagtgcccaaaacaaggacttgctgtttagccgggggtctccagctggcatgtctgttcagcccaaaaactggctacctggaccctgttaccggcagcagcgcgtttctaaaacaaaaacagacaacaacaacagcaactttacctggactggtgcttcaaaatataaccttaatgggcgtgaatctataatcaaccctggcactgctatggcctcacacaaagacgacaaagacaagttctttcccatgagcggtgtcatgatttttggaaaggagagcgccggagcttcaaacactgcattggacaatgtcatgatcacagacgaagaggaaatcaaagccactaaccccgtggccaccgaaagatttgggactgtggcagtcaatctccagagcagcagcacagaccctgcgaccggagatgtgcatgttatgggagccttacctggaatggtgtggcaagacagagacgtatacctgcagggtcctatttgggccaaaattcctcacacggatggacactttcacccgtctcctctcatgggcggctttggacttaagcacccgcctcctcagatcctcatcaaaaacacgcctgttcctgcgaatcctccggcagagttttcggctacaaagtttgcttcattcatcacccagtattccacaggacaagtgagcgtggagattgaatgggagctgcagaaagaaaacagcaaacgctggaatcccgaagtgcagtatacatctaactatgcaaaatctgccaacgttgatttcactgtggacaacaatggactttatactgagcctcgccccattggcacccgttacctcacccgtcccctgtaattgtgtgttaatcaataaaccggttgattcgtttcagttgaactttggtctctgcgaagggcgaattcgtttaaacctgcaggactagaggtcctgtattagaggtcacgtgagtgttttgcgacattttgcgacaccatgtggtcacgctgggtatttaagcccgagtgagcacgcagggtctccattttgaagcgggaggtttgaacgcgcagccgccaagccgaattctgcagatatccatcacactggcggccgctcgactagagcggccgccaccgcggtggagctccagcttttgttccctttagtgagggttaattgcgcgcttggcgtaatcatggtcatagctgtttcctgtgtgaaattgttatccgctcacaattccacacaacatacgagccggaagcataaagtgtaaagcctggggtgcctaatgagtgagctaactcacattaattgcgttgcgctcactgcccgctttccagtcgggaaacctgtcgtgccagctgcattaatgaatcggccaacgcgcggggagaggcggtttgcgtattgggcgctcttccgcttcctcgctcactgactcgctgcgctcggtcgttcggctgcggcgagcggtatcagctcactcaaaggcggtaatacggttatccacagaatcaggggataacgcaggaaagaacatgtgagcaaaaggccagcaaaaggccaggaaccgtaaaaaggccgcgttgctggcgtttttccataggctccgcccccctgacgagcatcacaaaaatcgacgctcaagtcagaggtggcgaaacccgacaggactataaagataccaggcgtttccccctggaagctccctcgtgcgctctcctgttccgaccctgccgcttaccggatacctgtccgcctttctcccttcgggaagcgtggcgctttctcatagctcacgctgtaggtatctcagttcggtgtaggtcgttcgctccaagctgggctgtgtgcacgaaccccccgttcagcccgaccgctgcgccttatccggtaactatcgtcttgagtccaacccggtaagacacgacttatcgccactggcagcagccactggtaacaggattagcagagcgaggtatgtaggcggtgctacagagttcttgaagtggtggcctaactacggctacactagaagaacagtatttggtatctgcgctctgctgaagccagttaccttcggaaaaagagttggtagctcttgatccggcaaacaaaccaccgctggtagcggtggtttttttgtttgcaagcagcagattacgcgcagaaaaaaaggatctcaagaagatcctttgatcttttctacggggtctgacgctcagtggaacgaaaactcacgttaagggattttggtcatgagattatcaaaaaggatcttcacctagatccttttaaattaaaaatgaagttttaaatcaatctaaagtatatatgagtaaacttggtctgacagttaccaatgcttaatcagtgaggcacctatctcagcgatctgtctatttcgttcatccatagttgcctgactccccgtcgtgtagataactacgatacgggagggcttaccatctggccccagtgctgcaatgataccgcgagacccacgctcaccggctccagatttatcagcaataaaccagccagccggaagggccgagcgcagaagtggtcctgcaactttatccgcctccatccagtctattaattgttgccgggaagctagagtaagtagttcgccagttaatagtttgcgcaacgttgttgccattgctacaggcatcgtggtgtcacgctcgtcgtttggtatggcttcattcagctccggttcccaacgatcaaggcgagttacatgatcccccatgttgtgcaaaaaagcggttagctccttcggtcctccgatcgttgtcagaagtaagttggccgcagtgttatcactcatggttatggcagcactgcataattctcttactgtcatgccatccgtaagatgcttttctgtgactggtgagtactcaaccaagtcattctgagaatagtgtatgcggcgaccgagttgctcttgcccggcgtcaatacgggataataccgcgccacatagcagaactttaaaagtgctcatcattggaaaacgttcttcggggcgaaaactctcaaggatcttaccgctgttgagatccagttcgatgtaacccactcgtgcacccaactgatcttcagcatcttttactttcaccagcgtttctgggtgagcaaaaacaggaaggcaaaatgccgcaaaaaagggaataagggcgacacggaaatgttgaatactcatactcttcctttttcaatattattgaagcatttatcagggttattgtctcatgagcggatacatatttgaatgtatttagaaaaataaacaaataggggttccgcgcacatttccccgaaaagtgccacctaaattgtaagcgttaatattttgttaaaattcgcgttaaatttttgttaaatcagctcattttttaaccaataggccgaaatcggcaaaatcccttataaatcaaaagaatagaccgagatagggttgagtgttgttccagtttggaacaagagtccactattaaagaacgtggactccaacgtcaaagggcgaaaaaccgtctatcagggcgatggcccactacgtgaaccatcaccctaatcaagttttttggggtcgaggtgccgtaaagcactaaatcggaaccctaaagggagcccccgatttagagcttgacggggaaagccggcgaacgtggcgagaaaggaagggaagaaagcgaaaggagcgggcgctagggcgctggcaagtgtagcggtcacgctgcgcgtaaccaccacacccgccgcgcttaatgcgccgctacagggcgcgtcccattcgccattcaggctgcgcaactgttgggaagggcgatcggtgcgggcctcttcgctattacgccagctggcgaaagggggatgtgctgcaaggcgattaagttgggtaacgccagggttttcccagtcacgacgttgtaaaacgacggccagtgagcgcgcgtaatacgactcactatagggcgaattgggtaccgggccccccctcgatcgaggtcgacggtatcgggggagctcgcagggtctccattttgaagcgggaggtttgaacgcgcagccgcc

SEQ ID NO: 28 - DNA, 7333 bp, synthetic construct
  source 1..7333: mol_type = other DNA
gtcacgacgttgtaaaacgacggccagtgagcgcgcgtaatacgactcactatagggcgaattgggtaccgggccccccctcgatcgaggtcgacggtatcgggggagctcgcagggtctccattttgaagcgggaggtttgaacgcgcagccgccatgccggggttttacgagattgtgattaaggtccccagcgaccttgacgagcatctgcccggcatttctgacagctttgtgaactgggtggccgagaaggaatgggagttgccgccagattctgacatggatctgaatctgattgagcaggcacccctgaccgtggccgagaagctgcagcgcgactttctgacggaatggcgccgtgtgagtaaggccccggaggctcttttctttgtgcaatttgagaagggagagagctacttccacatgcacgtgctcgtggaaaccaccggggtgaaatccatggttttgggacgtttcctgagtcagattcgcgaaaaactgattcagagaatttaccgcgggatcgagccgactttgccaaactggttcgcggtcacaaagaccagaaatggcgccggaggcgggaacaaggtggtggatgagtgctacatccccaattacttgctccccaaaacccagcctgagctccagtgggcgtggactaatatggaacagtatttaagcgcctgtttgaatctcacggagcgtaaacggttggtggcgcagcatctgacgcacgtgtcgcagacgcaggagcagaacaaagagaatcagaatcccaattctgatgcgccggtgatcagatcaaaaacttcagccaggtacatggagctggtcgggtggctcgtggacaaggggattacctcggagaagcagtggatccaggaggaccaggcctcatacatctccttcaatgcggcctccaactcgcggtcccaaatcaaggctgccttggacaatgcgggaaagattatgagcctgactaaaaccgcccccgactacctggtgggccagcagcccgtggaggacatttccagcaatcggatttataaaattttggaactaaacgggtacgatccccaatatgcggcttccgtctttctgggatgggccacgaaaaagttcggcaagaggaacaccatctggctgtttgggcctgcaactaccgggaagaccaacatcgcggaggccatagcccacactgtgcccttctacgggtgcgtaaactggaccaatgagaactttcccttcaacgactgtgtcgacaagatggtgatctggtgggaggaggggaagatgaccgccaaggtcgtggagtcggccaaagccattctcggaggaagcaaggtgcgcgtggaccagaaatgcaagtcctcggcccagatagacccgactcccgtgatcgtcacctccaacaccaacatgtgcgccgtgattgacgggaactcaacgaccttcgaacaccagcagccgttgcaagaccggatgttcaaatttgaactcacccgccgtctggatcatgactttgggaaggtcaccaagcaggaagtcaaagactttttccggtgggcaaaggatcacgtggttgaggtggagcatgaattctacgtcaaaaagggtggagccaagaaaagacccgcccccagtgacgcagatataagtgagcccaaacgggtgcgcgagtcagttgcgcagccatcgacgtcagacgcggaagcttcgatcaactacgcagacaggtaccaaaacaaatgttctcgtcacgtgggcatgaatctgatgctgtttccctgcagacaatgcgagagaatgaatcagaattcaaatatctgcttcactcacggacagaaagactgtttagagtgctttcccgtgtcagaatctcaacccgtttctgtcgtcaaaaaggcgtatcagaaactgtgctacattcatcatatcatgggaaaggtgccagacgcttgcactgcctgcgatctggtcaatgtggatttggatgactgcatctttgaacaataaatgatttaaatcaggtatggctgccgatggttatcttccagattggctcgaggacaacctctctgagggcattcgcgagtggtgggacctgaaacctggagccccgaaacccaaagccaaccagcaaaagcaggacaacggccggggtctggtgcttcctggctacaagtacctcggacccttcaacggactcgacaagggggagcccgtcaacgcggcggacgcagcggccctcgagcacgacaaggcctacgaccagcagctcaaagcgggtgacaatccgtacctgcggtataaccacgccgacgccgagtttcaggagcgtctgcaagaagatacgtcatttgggggcaacctcgggcgagcagtcttccaggccaagaagcgggttctcgaacctctcggtctggttgaggaaggcgctaagacggctcctgcaaagaagagaccggtagagccgtcacctcagcgttcccccgactcctccacgggcatcggcaagaaaggccagcagcccgccagaaagagactcaatttcggtcagactggcgactcagagtcagtccccgaccctcaacctctcggagaacctccagcagcgccctctagtgtgggatctggtacagtggctgcaggcggtggcgcaccaatggcagacaataacgaaggtgccgacggagtgggtaatgcctcaggaaattggcattgcgattccacatggctgggcgacagagtcattaccaccagcacccgaacctgggccctgcccacctacaacaaccacctctacaagcaaatctccagtgaaactgcaggtagtaccaacgacaacacctacttcggctacagcaccccctgggggtattttgactttaacagattccactgccacttctcaccacgtgactggcagcgactcatcaacaacaactggggattccggcccaagaagctgcggttcaagctcttcaacatccaggtcaaggaggtcacgacgaatgacggcgttacgaccatcgctaataaccttaccagcacgattcaggtattctcggactcggaataccagctgccgtacgtcctcggctctgcgcaccagggctgcctgcctccgttcccggcggacgtcttcatgattcctcagtacggctacctgactctcaacaatggcagtcagtctgtgggacgttcctccttctactgcctggagtacttcccctctcagatgctgagaacgggcaacaactttgagttcagctacagcttcgaggacgtgcctttccacagcagctacgcacacagccagagcctggaccggctgatgaatcccctcatcgaccagtacttgtactacctggccagaacacagagtaacccaggaggcacagctggcaatcgggaactgcagttttaccagggcgggccttcaactatggccgaacaagccaagaattggttacctggaccttgcttccggcaacaaagagtctccaaaacgctggatcaaaacaacaacagcaactttgcttggactggtgccaccaaatatcacctgaacggcagaaactcgttggttaatcccggcgtcgccatggcaactcacaaggacgacgaggaccgctttttcccatccagcggagtcctgatttttggaaaaactggagcaactaacaaaactacattggaaaatgtgttaatgacaaatgaagaagaaattcgtcctactaatcctgtagccacggaagaatacgggatagtcagcagcaacttacaagcggctaatactgcagcccagacacaagttgtcaacaaccagggagccttacctggcatggtctggcagaaccgggacgtgtacctgcagggtcccatctgggccaagattcctcacacggatggcaactttcacccgtctcctttgatgggcggctttggacttaaacatccgcctcctcagatcctgatcaagaacactcccgttcccgctaatcctccggaggtgtttactcctgccaagtttgcttcgttcatcacacagtacagcaccggacaagtcagcgtggaaatcgagtgggagctgcagaaggaaaacagcaagcgctggaacccggagattcagtacacctccaactttgaaaagcagactggtgtggactttgccgttgacagccagggtgtttactctgagcctcgccctattggcactcgttacctcacccgtaatctgtaattgcatgttaatcaataaaccggttgattcgtttcagttgaactttggtctctgcgaagggcgaattcgtttaaacctgcaggactagaggtcctgtattagaggtcacgtgagtgttttgcgacattttgcgacaccatgtggtcacgctgggtatttaagcccgagtgagcacgcagggtctccattttgaagcgggaggtttgaacgcgcagccgccaagccgaattctgcagatatccatcacactggcggccgctcgactagagcggccgccaccgcggtggagctccagcttttgttccctttagtgagggttaattgcgcgcttggcgtaatcatggtcatagctgtttcctgtgtgaaattgttatccgctcacaattccacacaacatacgagccggaagcataaagtgtaaagcctggggtgcctaatgagtgagctaactcacattaattgcgttgcgctcactgcccgctttccagtcgggaaacctgtcgtgccagctgcattaatgaatcggccaacgcgcggggagaggcggtttgcgtattgggcgctcttccgcttcctcgctcactgactcgctgcgctcggtcgttcggctgcggcgagcggtatcagctcactcaaaggcggtaatacggttatccacagaatcaggggataacgcaggaaagaacatgtgagcaaaaggccagcaaaaggccaggaaccgtaaaaaggccgcgttgctggcgtttttccataggctccgcccccctgacgagcatcacaaaaatcgacgctcaagtcagaggtggcgaaacccgacaggactataaagataccaggcgtttccccctggaagctccctcgtgcgctctcctgttccgaccctgccgcttaccggatacctgtccgcctttctcccttcgggaagcgtggcgctttctcatagctcacgctgtaggtatctcagttcggtgtaggtcgttcgctccaagctgggctgtgtgcacgaaccccccgttcagcccgaccgctgcgccttatccggtaactatcgtcttgagtccaacccggtaagacacgacttatcgccactggcagcagccactggtaacaggattagcagagcgaggtatgtaggcggtgctacagagttcttgaagtggtggcctaactacggctacactagaagaacagtatttggtatctgcgctctgctgaagccagttaccttcggaaaaagagttggtagctcttgatccggcaaacaaaccaccgctggtagcggtggtttttttgtttgcaagcagcagattacgcgcagaaaaaaaggatctcaagaagatcctttgatcttttctacggggtctgacgctcagtggaacgaaaactcacgttaagggattttggtcatgagattatcaaaaaggatcttcacctagatccttttaaattaaaaatgaagttttaaatcaatctaaagtatatatgagtaaacttggtctgacagttaccaatgcttaatcagtgaggcacctatctcagcgatctgtctatttcgttcatccatagttgcctgactccccgtcgtgtagataactacgatacgggagggcttaccatctggccccagtgctgcaatgataccgcgagacccacgctcaccggctccagatttatcagcaataaaccagccagccggaagggccgagcgcagaagtggtcctgcaactttatccgcctccatccagtctattaattgttgccgggaagctagagtaagtagttcgccagttaatagtttgcgcaacgttgttgccattgctacaggcatcgtggtgtcacgctcgtcgtttggtatggcttcattcagctccggttcccaacgatcaaggcgagttacatgatcccccatgttgtgcaaaaaagcggttagctccttcggtcctccgatcgttgtcagaagtaagttggccgcagtgttatcactcatggttatggcagcactgcataattctcttactgtcatgccatccgtaagatgcttttctgtgactggtgagtactcaaccaagtcattctgagaatagtgtatgcggcgaccgagttgctcttgcccggcgtcaatacgggataataccgcgccacatagcagaactttaaaagtgctcatcattggaaaacgttcttcggggcgaaaactctcaaggatcttaccgctgttgagatccagttcgatgtaacccactcgtgcacccaactgatcttcagcatcttttactttcaccagcgtttctgggtgagcaaaaacaggaaggcaaaatgccgcaaaaaagggaataagggcgacacggaaatgttgaatactcatactcttcctttttcaatattattgaagcatttatcagggttattgtctcatgagcggatacatatttgaatgtatttagaaaaataaacaaataggggttccgcgcacatttccccgaaaagtgccacctaaattgtaagcgttaatattttgttaaaattcgcgttaaatttttgttaaatcagctcattttttaaccaataggccgaaatcggcaaaatcccttataaatcaaaagaatagaccgagatagggttgagtgttgttccagtttggaacaagagtccactattaaagaacgtggactccaacgtcaaagggcgaaaaaccgtctatcagggcgatggcccactacgtgaaccatcaccctaatcaagttttttggggtcgaggtgccgtaaagcactaaatcggaaccctaaagggagcccccgatttagagcttgacggggaaagccggcgaacgtggcgagaaaggaagggaagaaagcgaaaggagcgggcgctagggcgctggcaagtgtagcggtcacgctgcgcgtaaccaccacacccgccgcgcttaatgcgccgctacagggcgcgtcccattcgccattcaggctgcgcaactgttgggaagggcgatcggtgcgggcctcttcgctattacgccagctggcgaaagggggatgtgctgcaaggcgattaagttgggtaacgccagggttttccca

SEQ ID NO: 29 - DNA, 7341 bp, synthetic construct
  source 1..7341: mol_type = other DNA
atgccgggcttctacgagatcgtgcttaaggtgccgagcgacctggacgagcacctgccgggcatttctgactcgtttgtgaactgggtggcagagaaggaatgggagctgcccccggattctgacatggatcggaatctgattgagcaggcacccctgaccgtggccgagaagctacagcgcgacttcctggtccaatggcgccgcgtgagtaaggccccggaggccctcttctttgttcagttcgagaagggcgagtcctacttccacctccatattctggtagagaccacgggggtcaaatccatggtgctgggccgcttcctgagtcagattcgggacaagctggtgcagaccatctaccgcgggatcgagccgaccctgcccaactggttcgcggtgacaaagacgcgtaatggcgccggaggggggaacaaggtggtggacgagtgctacatccccaactacctgctgcccaagactcagcccgagctgcagtgggcgtggactaacatggaggagtatataagcgcgtgcttgaacctggccgagcgcaaacggctcgtggcgcagcacctgacccacgtcagccagacccaggagcagaacaaggagaatctgaacccgaattctgacgcgcctgtcatccggtcaaaaacctccgcgcgctacatggagctggtcgggtggctggtggaccggggcatcacctccgagaagcagtggatccaggaggaccaggcctcgtacatctccttcaacgccgcctccaactcgcggtctcagatcaaggccgcgctggacaatgccggcaagatcatggcgctgaccaaatccgcgcccgactacctggtaggccccgctctgcccgcggacattaaatccaaccgcatctaccgcatcctggagctgaatggctacgaccctgcctacgccggttccgtctttctcggctgggcccagaaaaagtttggcaaaaggaacaccatctggctgtttgggccggccaccacgggcaagaccaacatcgcggaagccatcgcccacgccgtgcccttctacggctgcgtcaactggaccaatgagaactttcccttcaacgattgcgtcgacaagatggtgatctggtgggaggagggcaagatgacggccaaggtcgtggagtccgccaaggccattctcggcggcagcaaggtgcgcgtggaccaaaagtgcaagtcgtccgcccagatcgatcccacccccgtgatcgtcacctccaacaccaacatgtgcgccgtgattgacgggaacagcaccaccttcgagcaccagcagccgttgcaggaccggatgttcaaatttgaacttacccgccgtctggagcacgactttggcaaggtgacaaagcaggaagtcaaagagttcttccgctgggcgcaggatcacgtgaccgaggtggcgcatgagttctacgtcagaaagggtggagctaacaaaagacccgcccccgatgacgcggatataagcgagcccaagcgggcctgcccctcagtcgcggatccatcgacgtcagacgcggaaggagctccggtggactttgccgacaggtaccaaaacaaatgttctcgtcacgcgggcatgcttcagatgctgtttccctgcaaaacatgcgagagaatgaatcagaatttcaacatttgcttcacgcacgggaccagagactgttcagaatgtttccctggcgtgtcagaatctcaaccggtcgtcagaaaaaagacgtatcggaaactctgtgcgattcatcatctgctggggcgggcacccgagattgcttgctcggcctgcgacctggtcaacgtggacctggatgactgtgtttctgagcaataaatgacttaaaccaggtatggctgccgatggttatcttccagattggctcgaggacaacctctctgagggcattcgcgagtggtgggacctgaaacctggagccccgaaacccaaagccaaccagcaaaagcaggacaacggccggggtctggtgcttcctggctacaagtacctcggacccttcaacggactcgacaagggggagcccgtcaacgcggcggacgcagcggccctcgagcacgacaaggcctacgaccagcagctccaagcgggtgacaatccgtacctgcggtataatcacgccgacgccgagtttcaggagcgtctgcaagaagatacgtcttttgggggcaacctcgggcgcgcagtcttccaggccaaaaagcgggttctcgaacctctgggcctggttgaatcgccggttaagacggctcctggaaagaagagaccggtagagccatcaccccagcgctctccagactcctctacgggcatcggcaagaaaggccagcagcccgcaaaaaagagactcaattttgggcagactggcgactcagagtcagtccccgaccctcaaccaatcggagaaccaccagcaggcccctctggtctgggatctggtacaatggctgcaggcggtggcgctccaatggcagacaataacgaaggcgccgacggagtgggtagttcctcaggaaattggcattgcgattccacatggctgggcgacagagtcatcaccaccagcacccgcacctgggccctgcccacctacaacaaccacctctacaagcaaatctccaacgggacctcgggaggaagcaccaacgacaacacatacttcggctacagcaccccctgggggtattttgacttcaacagattccactgccacttttcaccacgtgactggcagcgactcatcaacaacaactggggattccggcccaagaggctcaacttcaagctcttcaacatccaagtcaaggaggtcacgcagaatgaaggcaccaagaccatcgccaataaccttaccagcacgattcaggtctttacggactcggaataccagctcccgtacgtgctcggctcggcgcaccagggctgcctgcctccgttcccggcggacgtcttcatgattcctcagtacgggtacctgactctgaacaatggcagtcaggctgtgggccggtcgtccttctactgcctggagtactttccttctcaaatgctgagaacgggcaacaactttgaattcagctacaacttcgaggacgtgcccttccacagcagctacgcgcacagccagagcctggaccggctgatgaaccctctcatcgaccagtacttgtactacctgtcccggactcaaagcacgggcggtactgcaggaactcagcagttgctattttctcaggccgggcctaacaacatgtcggctcaggccaagaactggctacccggtccctgctaccggcagcaacgcgtctccacgacactgtcgcagaacaacaacagcaactttgcctggacgggtgccaccaagtatcatctgaatggcagagactctctggtgaatcctggcgttgccatggctacccacaaggacgacgaagagcgattttttccatccagcggagtcttaatgtttgggaaacagggagctggaaaagacaacgtggactatagcagcgtgatgctaaccagcgaggaagaaataaagaccaccaacccagtggccacagaacagtacggcgtggtggccgataacctgcaacagcaaaacgccgctcctattgtaggggccgtcaatagtcaaggagccttacctggcatggtgtggcagaaccgggacgtgtacctgcagggtcccatctgggccaagattcctcatacggacggcaactttcatccctcgccgctgatgggaggctttggactgaagcatccgcctcctcagatcctgattaaaaacacacctgttcccgcggatcctccgaccaccttcaatcaggccaagctggcttctttcatcacgcagtacagtaccggccaggtcagcgtggagatcgagtgggagctgcagaaggagaacagcaaacgctggaacccagagattcagtacacttccaactactacaaatctacaaatgtggactttgctgtcaatactgagggtacttattccgagcctcgccccattggcacccgttacctcacccgtaatctgtaattgcctgttaatcaataaaccggttgattcgtttcagttgaactttggtctctgcgaagggcgaattcgtttaaacctgcaggactagaggtcctgtattagaggtcacgtgagtgttttgcgacattttgcgacaccatgtggtcacgctgggtatttaagcccgagtgagcacgcagggtctccattttgaagcgggaggtttgaacgcgcagccgccaagccgaattctgcagatatctcaccactggcggccgctcgactagagcggccgccaccgcggtggagctccagcttttgttccctttagtgagggttaattgcgcgcttggcgtaatcatggtcatagctgtttcctgtgtgaaattgttatccgctcacaattccacacaacatacgagccggaagcataaagtgtaaagcctggggtgcctaatgagtgagctaactcacattaattgcgttgcgctcactgcccgctttccagtcgggaaacctgtcgtgccagctgcattaatgaatcggccaacgcgcggggagaggcggtttgcgtattgggcgctcttccgcttcctcgctcactgactcgctgcgctcggtcgttcggctgcggcgagcggtatcagctcactcaaaggcggtaatacggttatccacagaatcaggggataacgcaggaaagaacatgtgagcaaaaggccagcaaaaggccaggaaccgtaaaaaggccgcgttgctggcgtttttccataggctccgcccccctgacgagcatcacaaaaatcgacgctcaagtcagaggtggcgaaacccgacaggactataaagataccaggcgtttccccctggaagctccctcgtgcgctctcctgttccgaccctgccgcttaccggatacctgtccgcctttctcccttcgggaagcgtggcgctttctcatagctcacgctgtaggtatctcagttcggtgtaggtcgttcgctccaagctgggctgtgtgcacgaaccccccgttcagcccgaccgctgcgccttatccggtaactatcgtcttgagtccaacccggtaagacacgacttatcgccactggcagcagccactggtaacaggattagcagagcgaggtatgtaggcggtgctacagagttcttgaagtggtggcctaactacggctacactagaagaacagtatttggtatctgcgctctgctgaagccagttaccttcggaaaaagagttggtagctcttgatccggcaaacaaaccaccgctggtagcggtggtttttttgtttgcaagcagcagattacgcgcagaaaaaaaggatctcaagaagatcctttgatcttttctacggggtctgacgctcagtggaacgaaaactcacgttaagggattttggtcatgagattatcaaaaaggatcttcacctagatccttttaaattaaaaatgaagttttaaatcaatctaaagtatatatgagtaaacttggtctgacagttaccaatgcttaatcagtgaggcacctatctcagcgatctgtctatttcgttcatccatagttgcctgactccccgtcgtgtagataactacgatacgggagggcttaccatctggccccagtgctgcaatgataccgcgagacccacgctcaccggctccagatttatcagcaataaaccagccagccggaagggccgagcgcagaagtggtcctgcaactttatccgcctccatccagtctattaattgttgccgggaagctagagtaagtagttcgccagttaatagtttgcgcaacgttgttgccattgctacaggcatcgtggtgtcacgctcgtcgtttggtatggcttcattcagctccggttcccaacgatcaaggcgagttacatgatcccccatgttgtgcaaaaaagcggttagctccttcggtcctccgatcgttgtcagaagtaagttggccgcagtgttatcactcatggttatggcagcactgcataattctcttactgtcatgccatccgtaagatgcttttctgtgactggtgagtactcaaccaagtcattctgagaatagtgtatgcggcgaccgagttgctcttgcccggcgtcaatacgggataataccgcgccacatagcagaactttaaaagtgctcatcattggaaaacgttcttcggggcgaaaactctcaaggatcttaccgctgttgagatccagttcgatgtaacccactcgtgcacccaactgatcttcagcatcttttactttcaccagcgtttctgggtgagcaaaaacaggaaggcaaaatgccgcaaaaaagggaataagggcgacacggaaatgttgaatactcatactcttcctttttcaatattattgaagcatttatcagggttattgtctcatgagcggatacatatttgaatgtatttagaaaaataaacaaataggggttccgcgcacatttccccgaaaagtgccacctaaattgtaagcgttaatattttgttaaaattcgcgttaaatttttgttaaatcagctcattttttaaccaataggccgaaatcggcaaaatcccttataaatcaaaagaatagaccgagatagggttgagtgttgttccagtttggaacaagagtccactattaaagaacgtggactccaacgtcaaagggcgaaaaaccgtctatcagggcgatggcccactacgtgaaccatcaccctaatcaagttttttggggtcgaggtgccgtaaagcactaaatcggaaccctaaagggagcccccgatttagagcttgacggggaaagccggcgaacgtggcgagaaaggaagggaagaaagcgaaaggagcgggcgctagggcgctggcaagtgtagcggtcacgctgcgcgtaaccaccacacccgccgcgcttaatgcgccgctacagggcgcgtcccattcgccattcaggctgcgcaactgttgggaagggcgatcggtgcgggcctcttcgctattacgccagctggcgaaagggggatgtgctgcaaggcgattaagttgggtaacgccagggttttcccagtcacgacgttgtaaaacgacggccagtgagcgcgcgtaatacgactcactatagggcgaattgggtaccgggccccccctcgatcgaggtcgacggtatcgggggagctcgcagggtctccattttgaagcgggaggtttgaacgcgcagccgcc

SEQ ID NO: 30 - DNA, 7336 bp, synthetic construct
  source 1..7336: mol_type = other DNA
atgccggggttttacgagattgtgattaaggtccccagcgaccttgacgagcatctgcccggcatttctgacagctttgtgaactgggtggccgagaaggaatgggagttgccgccagattctgacatggatctgaatctgattgagcaggcacccctgaccgtggccgagaagctgcagcgcgactttctgacggaatggcgccgtgtgagtaaggccccggaggctcttttctttgtgcaatttgagaagggagagagctacttccacatgcacgtgctcgtggaaaccaccggggtgaaatccatggttttgggacgtttcctgagtcagattcgcgaaaaactgattcagagaatttaccgcgggatcgagccgactttgccaaactggttcgcggtcacaaagaccagaaatggcgccggaggcgggaacaaggtggtggatgagtgctacatccccaattacttgctccccaaaacccagcctgagctccagtgggcgtggactaatatggaacagtatttaagcgcctgtttgaatctcacggagcgtaaacggttggtggcgcagcatctgacgcacgtgtcgcagacgcaggagcagaacaaagagaatcagaatcccaattctgatgcgccggtgatcagatcaaaaacttcagccaggtacatggagctggtcgggtggctcgtggacaaggggattacctcggagaagcagtggatccaggaggaccaggcctcatacatctccttcaatgcggcctccaactcgcggtcccaaatcaaggctgccttggacaatgcgggaaagattatgagcctgactaaaaccgcccccgactacctggtgggccagcagcccgtggaggacatttccagcaatcggatttataaaattttggaactaaacgggtacgatccccaatatgcggcttccgtctttctgggatgggccacgaaaaagttcggcaagaggaacaccatctggctgtttgggcctgcaactaccgggaagaccaacatcgcggaggccatagcccacactgtgcccttctacgggtgcgtaaactggaccaatgagaactttcccttcaacgactgtgtcgacaagatggtgatctggtgggaggaggggaagatgaccgccaaggtcgtggagtcggccaaagccattctcggaggaagcaaggtgcgcgtggaccagaaatgcaagtcctcggcccagatagacccgactcccgtgatcgtcacctccaacaccaacatgtgcgccgtgattgacgggaactcaacgaccttcgaacaccagcagccgttgcaagaccggatgttcaaatttgaactcacccgccgtctggatcatgactttgggaaggtcaccaagcaggaagtcaaagactttttccggtgggcaaaggatcacgtggttgaggtggagcatgaattctacgtcaaaaagggtggagccaagaaaagacccgcccccagtgacgcagatataagtgagcccaaacgggtgcgcgagtcagttgcgcagccatcgacgtcagacgcggaagcttcgatcaactacgcagacaggtaccaaaacaaatgttctcgtcacgtgggcatgaatctgatgctgtttccctgcagacaatgcgagagaatgaatcagaattcaaatatctgcttcactcacggacagaaagactgtttagagtgctttcccgtgtcagaatctcaacccgtttctgtcgtcaaaaaggcgtatcagaaactgtgctacattcatcatatcatgggaaaggtgccagacgcttgcactgcctgcgatctggtcaatgtggatttggatgactgcatctttgaacaataaatgatttaaatcaggtatggctgccgatggttatcttccagattggctcgaggacaacctctctgagggcattcgcgagtggtgggcgctgaaacctggagccccgaagcccaaagccaaccagcaaaagcaggacgacggccggggtctggtgcttcctggctacaagtacctcggacccttcaacggactcgacaagggggagcccgtcaacgcggcggacgcagcggccctcgagcacgacaaggcctacgaccagcagctgcaggcgggtgacaatccgtacctgcggtataaccacgccgacgccgagtttcaggagcgtctgcaagaagatacgtcttttgggggcaacctcgggcgagcagtcttccaggccaagaagcgggttctcgaacctctcggtctggttgaggaaggcgctaagacggctcctggaaagaagagaccggtagagccatcaccccagcgttctccagactcctctacgggcatcggcaagaaaggccaacagcccgccagaaaaagactcaattttggtcagactggcgactcagagtcagttccagaccctcaacctctcggagaacctccagcagcgccctctggtgtgggacctaatacaatggctgcaggcggtggcgcaccaatggcagacaataacgaaggcgccgacggagtgggtagttcctcgggaaattggcattgcgattccacatggctgggcgacagagtcatcaccaccagcacccgaacctgggccctgcccacctacaacaaccacctctacaagcaaatctccaacgggacatcgggaggagccaccaacgacaacacctacttcggctacagcaccccctgggggtattttgactttaacagattccactgccacttttcaccacgtgactggcagcgactcatcaacaacaactggggattccggcccaagagactcagcttcaagctcttcaacatccaggtcaaggaggtcacgcagaatgaaggcaccaagaccatcgccaataacctcaccagcaccatccaggtgtttacggactcggagtaccagctgccgtacgttctcggctctgcccaccagggctgcctgcctccgttcccggcggacgtgttcatgattccccagtacggctacctaacactcaacaacggtagtcaggccgtgggacgctcctccttctactgcctggaatactttccttcgcagatgctgagaaccggcaacaacttccagtttacttacaccttcgaggacgtgcctttccacagcagctacgcccacagccagagcttggaccggctgatgaatcctctgattgaccagtacctgtactacttgtctcggactcaaacaacaggaggcacggcaaatacgcagactctgggcttcagccaaggtgggcctaatacaatggccaatcaggcaaagaactggctgccaggaccctgttaccgccaacaacgcgtctcaacgacaaccgggcaaaacaacaatagcaactttgcctggactgctgggaccaaataccatctgaatggaagaaattcattggctaatcctggcatcgctatggcaacacacaaagacgacgaggagcgtttttttcccagtaacgggatcctgatttttggcaaacaaaatgctgccagagacaatgcggattacagcgatgtcatgctcaccagcgaggaagaaatcaaaaccactaaccctgtggctacagaggaatacggtatcgtggcagataacttgcagcagcaaaacacggctcctcaaattggaactgtcaacagccagggggccttacccggtatggtctggcagaaccgggacgtgtacctgcagggtcccatctgggccaagattcctcacacggacggcaacttccacccgtctccgctgatgggcggctttggcctgaaacatcctccgcctcagatcctgatcaagaacacgcctgtacctgcggatcctccgaccaccttcaaccagtcaaagctgaactctttcatcacgcaatacagcaccggacaggtcagcgtggaaattgaatgggagctgcagaaggaaaacagcaagcgctggaaccccgagatccagtacacctccaactactacaaatctacaagtgtggactttgctgttaatacagaaggcgtgtactctgaaccccgccccattggcacccgttacctcacccgtaatctgtaattgcctgttaatcaataaaccggttgattcgtttcagttgaactttggtctctgcgaagggcgaattcgtttaaacctgcaggactagaggtcctgtattagaggtcacgtgagtgttttgcgacattttgcgacaccatgtggtcacgctgggtatttaagcccgagtgagcacgcagggtctccattttgaagcgggaggtttgaacgcgcagccgccaagccgaattctgcagatatccatcacactggcggccgctcgactagagcggccgccaccgcggtggagctccagcttttgttccctttagtgagggttaattgcgcgcttggcgtaatcatggtcatagctgtttcctgtgtgaaattgttatccgctcacaattccacacaacatacgagccggaagcataaagtgtaaagcctggggtgcctaatgagtgagctaactcacattaattgcgttgcgctcactgcccgctttccagtcgggaaacctgtcgtgccagctgcattaatgaatcggccaacgcgcggggagaggcggtttgcgtattgggcgctcttccgcttcctcgctcactgactcgctgcgctcggtcgttcggctgcggcgagcggtatcagctcactcaaaggcggtaatacggttatccacagaatcaggggataacgcaggaaagaacatgtgagcaaaaggccagcaaaaggccaggaaccgtaaaaaggccgcgttgctggcgtttttccataggctccgcccccctgacgagcatcacaaaaatcgacgctcaagtcagaggtggcgaaacccgacaggactataaagataccaggcgtttccccctggaagctccctcgtgcgctctcctgttccgaccctgccgcttaccggatacctgtccgcctttctcccttcgggaagcgtggcgctttctcatagctcacgctgtaggtatctcagttcggtgtaggtcgttcgctccaagctgggctgtgtgcacgaaccccccgttcagcccgaccgctgcgccttatccggtaactatcgtcttgagtccaacccggtaagacacgacttatcgccactggcagcagccactggtaacaggattagcagagcgaggtatgtaggcggtgctacagagttcttgaagtggtggcctaactacggctacactagaagaacagtatttggtatctgcgctctgctgaagccagttaccttcggaaaaagagttggtagctcttgatccggcaaacaaaccaccgctggtagcggtggtttttttgtttgcaagcagcagattacgcgcagaaaaaaaggatctcaagaagatcctttgatcttttctacggggtctgacgctcagtggaacgaaaactcacgttaagggattttggtcatgagattatcaaaaaggatcttcacctagatccttttaaattaaaaatgaagttttaaatcaatctaaagtatatatgagtaaacttggtctgacagttaccaatgcttaatcagtgaggcacctatctcagcgatctgtctatttcgttcatccatagttgcctgactccccgtcgtgtagataactacgatacgggagggcttaccatctggccccagtgctgcaatgataccgcgagacccacgctcaccggctccagatttatcagcaataaaccagccagccggaagggccgagcgcagaagtggtcctgcaactttatccgcctccatccagtctattaattgttgccgggaagctagagtaagtagttcgccagttaatagtttgcgcaacgttgttgccattgctacaggcatcgtggtgtcacgctcgtcgtttggtatggcttcattcagctccggttcccaacgatcaaggcgagttacatgatcccccatgttgtgcaaaaaagcggttagctccttcggtcctccgatcgttgtcagaagtaagttggccgcagtgttatcactcatggttatggcagcactgcataattctcttactgtcatgccatccgtaagatgcttttctgtgactggtgagtactcaaccaagtcattctgagaatagtgtatgcggcgaccgagttgctcttgcccggcgtcaatacgggataataccgcgccacatagcagaactttaaaagtgctcatcattggaaaacgttcttcggggcgaaaactctcaaggatcttaccgctgttgagatccagttcgatgtaacccactcgtgcacccaactgatcttcagcatcttttactttcaccagcgtttctgggtgagcaaaaacaggaaggcaaaatgccgcaaaaaagggaataagggcgacacggaaatgttgaatactcatactcttcctttttcaatattattgaagcatttatcagggttattgtctcatgagcggatacatatttgaatgtatttagaaaaataaacaaataggggttccgcgcacatttccccgaaaagtgccacctaaattgtaagcgttaatattttgttaaaattcgcgttaaatttttgttaaatcagctcattttttaaccaataggccgaaatcggcaaaatcccttataaatcaaaagaatagaccgagatagggttgagtgttgttccagtttggaacaagagtccactattaaagaacgtggactccaacgtcaaagggcgaaaaaccgtctatcagggcgatggcccactacgtgaaccatcaccctaatcaagttttttggggtcgaggtgccgtaaagcactaaatcggaaccctaaagggagcccccgatttagagcttgacggggaaagccggcgaacgtggcgagaaaggaagggaagaaagcgaaaggagcgggcgctagggcgctggcaagtgtagcggtcacgctgcgcgtaaccaccacacccgccgcgcttaatgcgccgctacagggcgcgtcccattcgccattcaggctgcgcaactgttgggaagggcgatcggtgcgggcctcttcgctattacgccagctggcgaaagggggatgtgctgcaaggcgattaagttgggtaacgccagggttttcccagtcacgacgttgtaaaacgacggccagtgagcgcgcgtaatacgactcactatagggcgaattgggtaccgggccccccctcgatcgaggtcgacggtatcgggggagctcgcagggtctccattttgaagcgggaggtttgaacgcgcagccgcc

SEQ ID NO: 31 - DNA, 7331 bp, synthetic construct
  source 1..7331: mol_type = other DNA
cccattcgccattcaggctgcgcaactgttgggaagggcgatcggtgcgggcctcttcgctattacgccagctggcgaaagggggatgtgctgcaaggcgattaagttgggtaacgccagggttttcccagtcacgacgttgtaaaacgacggccagtgagcgcgcgtaatacgactcactatagggcgaattgggtaccgggccccccctcgatcgaggtcgacggtatcgggggagctcgcagggtctccattttgaagcgggaggtttgaacgcgcagccgccatgccggggttttacgagattgtgattaaggtccccagcgaccttgacgagcatctgcccggcatttctgacagctttgtgaactgggtggccgagaaggaatgggagttgccgccagattctgacatggatctgaatctgattgagcaggcacccctgaccgtggccgagaagctgcagcgcgactttctgacggaatggcgccgtgtgagtaaggccccggaggctcttttctttgtgcaatttgagaagggagagagctacttccacatgcacgtgctcgtggaaaccaccggggtgaaatccatggttttgggacgtttcctgagtcagattcgcgaaaaactgattcagagaatttaccgcgggatcgagccgactttgccaaactggttcgcggtcacaaagaccagaaatggcgccggaggcgggaacaaggtggtggatgagtgctacatccccaattacttgctccccaaaacccagcctgagctccagtgggcgtggactaatatggaacagtatttaagcgcctgtttgaatctcacggagcgtaaacggttggtggcgcagcatctgacgcacgtgtcgcagacgcaggagcagaacaaagagaatcagaatcccaattctgatgcgccggtgatcagatcaaaaacttcagccaggtacatggagctggtcgggtggctcgtggacaaggggattacctcggagaagcagtggatccaggaggaccaggcctcatacatctccttcaatgcggcctccaactcgcggtcccaaatcaaggctgccttggacaatgcgggaaagattatgagcctgactaaaaccgcccccgactacctggtgggccagcagcccgtggaggacatttccagcaatcggatttataaaattttggaactaaacgggtacgatccccaatatgcggcttccgtctttctgggatgggccacgaaaaagttcggcaagaggaacaccatctggctgtttgggcctgcaactaccgggaagaccaacatcgcggaggccatagcccacactgtgcccttctacgggtgcgtaaactggaccaatgagaactttcccttcaacgactgtgtcgacaagatggtgatctggtgggaggaggggaagatgaccgccaaggtcgtggagtcggccaaagccattctcggaggaagcaaggtgcgcgtggaccagaaatgcaagtcctcggcccagatagacccgactcccgtgatcgtcacctccaacaccaacatgtgcgccgtgattgacgggaactcaacgaccttcgaacaccagcagccgttgcaagaccggatgttcaaatttgaactcacccgccgtctggatcatgactttgggaaggtcaccaagcaggaagtcaaagactttttccggtgggcaaaggatcacgtggttgaggtggagcatgaattctacgtcaaaaagggtggagccaagaaaagacccgcccccagtgacgcagatataagtgagcccaaacgggtgcgcgagtcagttgcgcagccatcgacgtcagacgcggaagcttcgatcaactacgcggacaggtaccaaaacaaatgttctcgtcacgtgggcatgaatctgatgctgtttccctgcagacaatgcgagagactgaatcagaattcaaatatctgcttcactcacggtgtcaaagactgtttagagtgctttcccgtgtcagaatctcaacccgtttctgtcgtcaaaaaggcgtatcagaaactgtgctacattcatcacatcatgggaaaggtgccagacgcttgcactgcttgcgacctggtcaatgtggacttggatgactgtgtttctgaacaataaatgacttaaaccaggtatggctgccgatggttatcttccagattggctcgaggacaaccttagtgaaggaattcgcgagtggtgggctttgaaacctggagcccctcaacccaaggcaaatcaacaacatcaagacaacgctcgaggtcttgtgcttccgggttacaaataccttggacccggcaacggactcgacaagggggagccggtcaacgcagcagacgcggcggccctcgagcacgacaaggcctacgaccagcagctcaaggccggagacaacccgtacctcaagtacaaccacgccgacgccgagttccaggagcggctcaaagaagatacgtcttttgggggcaacctcgggcgagcagtcttccaggccaaaaagaggcttcttgaacctcttggtctggttgaggaagcggctaagacggctcctggaaagaagaggcctgtagagcagtctcctcaggaaccggactcctccgcgggtattggcaaatcgggtgcacagcccgctaaaaagagactcaatttcggtcagactggcgacacagagtcagtcccagaccctcaaccaatcggagaacctcccgcagccccctcaggtgtgggatctcttacaatggcttcaggtggtggcgcaccagtggcagacaataacgaaggtgccgatggagtgggtagttcctcgggaaattggcattgcgattcccaatggctgggggacagagtcatcaccaccagcacccgaacctgggccctgcccacctacaacaatcacctctacaagcaaatctccaacagcacatctggaggatcttcaaatgacaacgcctacttcggctacagcaccccctgggggtattttgacttcaacagattccactgccacttctcaccacgtgactggcagcgactcatcaacaacaactggggattccggcctaagcgactcaacttcaagctcttcaacattcaggtcaaagaggttacggacaacaatggagtcaagaccatcgccaataaccttaccagcacggtccaggtcttcacggactcagactatcagctcccgtacgtgctcgggtcggctcacgagggctgcctcccgccgttcccagcggacgttttcatgattcctcagtacgggtatctgacgcttaatgatggaagccaggccgtgggtcgttcgtccttttactgcctggaatatttcccgtcgcaaatgctaagaacgggtaacaacttccagttcagctacgagtttgagaacgtacctttccatagcagctacgctcacagccaaagcctggaccgactaatgaatccactcatcgaccaatacttgtactatctctcaaagactattaacggttctggacagaatcaacaaacgctaaaattcagtgtggccggacccagcaacatggctgtccagggaagaaactacatacctggacccagctaccgacaacaacgtgtctcaaccactgtgactcaaaacaacaacagcgaatttgcttggcctggagcttcttcttgggctctcaatggacgtaatagcttgatgaatcctggacctgctatggccagccacaaagaaggagaggaccgtttctttcctttgtctggatctttaatttttggcaaacaaggaactggaagagacaacgtggatgcggacaaagtcatgataaccaacgaagaagaaattaaaactactaacccggtagcaacggagtcctatggacaagtggccacaaaccaccagagtgcccaagcacaggcgcagaccggctgggttcaaaaccaaggaatacttccgggtatggtttggcaggacagagatgtgtacctgcaaggacccatttgggccaaaattcctcacacggacggcaactttcacccttctccgctgatgggagggtttggaatgaagcacccgcctcctcagatcctcatcaaaaacacacctgtacctgcggatcctccaacggccttcaacaaggacaagctgaactctttcatcacccagtattctactggccaagtcagcgtggagatcgagtgggagctgcagaaggaaaacagcaagcgctggaacccggagatccagtacacttccaactattacaagtctaataatgttgaatttgctgttaatactgaaggtgtatatagtgaaccccgccccattggcaccagatacctgactcgtaatctgtaattgcttgttaatcaataaaccgtttaattcgtttcagttgaactttggtctctgcgaagggcgaattcgtttaaacctgcaggactagaggtcctgtattagaggtcacgtgagtgttttgcgacattttgcgacaccatgtggtcacgctgggtatttaagcccgagtgagcacgcagggtctccattttgaagcgggaggtttgaacgcgcagccgccaagccgaattctgcagatatccatcacactggcggccgctcgactagagcggccgccaccgcggtggagctccagcttttgttccctttagtgagggttaattgcgcgcttggcgtaatcatggtcatagctgtttcctgtgtgaaattgttatccgctcacaattccacacaacatacgagccggaagcataaagtgtaaagcctggggtgcctaatgagtgagctaactcacattaattgcgttgcgctcactgcccgctttccagtcgggaaacctgtcgtgccagctgcattaatgaatcggccaacgcgcggggagaggcggtttgcgtattgggcgctcttccgcttcctcgctcactgactcgctgcgctcggtcgttcggctgcggcgagcggtatcagctcactcaaaggcggtaatacggttatccacagaatcaggggataacggcaggaaagaacatgtgagcaaaaggccagcaaaaggccaggaaccgtaaaaaggccgcgttgctggcgtttttccataggctccgcccccctgacgagcatcacaaaaatcgacgctcaagtcagaggtggcgaaacccgacaggactataaagataccaggcgtttccccctggaagctccctcgtgcgctctcctgttccgaccctgccgcttaccggatacctgtccgcctttctcccttcgggaagcgtggcgctttctcatagctcacgctgtaggtatctcagttcggtgtaggtcgttcgctccaagctgggctgtgtgcacgaaccccccgttcagcccgaccgctgcgccttatccggtaactatcgtcttgagtccaacccggtaagacacgacttatcgccactggcagcagccactggtaacaggattagcagagcgaggtatgtaggcggtgctacagagttcttgaagtggtggcctaactacggctacactagaagaacagtatttggtatctgcgctctgctgaagccagttaccttcggaaaaagagttggtagctcttgatccggcaaacaaaccaccgctggtagcggtggtttttttgtttgcaagcagcagattacgcgcagaaaaaaaggatctcaagaagatcctttgatcttttctacggggtctgacgctcagtggaacgaaaactcacgttaagggattttggtcatgagattatcaaaaaggatcttcacctagatccttttaaattaaaaatgaagttttaaatcaatctaaagtatatatgagtaaacttggtctgacagttaccaatgcttaatcagtgaggcacctatctcagcgatctgtctatttcgttcatccatagttgcctgactccccgtcgtgtagataactacgatacgggagggcttaccatctggccccagtgctgcaatgataccgcgagacccacgctcaccggctccagatttatcagcaataaaccagccagccggaagggccgagcgcagaagtggtcctgcaactttatccgcctccatccagtctattaattgttgccgggaagctagagtaagtagttcgccagttaatagtttgcgcaacgttgttgccattgctacaggcatcgtggtgtcacgctcgtcgtttggtatggcttcattcagctccggttcccaacgatcaaggcgagttacatgatcccccatgttgtgcaaaaaagcggttagctccttcggtcctccgatcgttgtcagaagtaagttggccgcagtgttatcactcatggttatggcagcactgcataattctcttactgtcatgccatccgtaagatgcttttctgtgactggtgagtactcaaccaagtcattctgagaatagtgtatgcggcgaccgagttgctcttgcccggcgtcaatacgggataataccgcgccacatagcagaactttaaaagtgctcatcattggaaaacgttcttcggggcgaaaactctcaaggatcttaccgctgttgagatccagttcgatgtaacccactcgtgcacccaactgatcttcagcatcttttactttcaccagcgtttctgggtgagcaaaaacaggaaggcaaaatgccgcaaaaaagggaataagggcgacacggaaatgttgaatactcatactcttcctttttcaatattattgaagcatttatcagggttattgtctcatgagcggatacatatttgaatgtatttagaaaaataaacaaataggggttccgcgcacatttccccgaaaagtgccacctaaattgtaagcgttaatattttgttaaaattcgcgttaaatttttgttaaatcagctcattttttaaccaataggccgaaatcggcaaaatcccttataaatcaaaagaatagaccgagatagggttgagtgttgttccagtttggaacaagagtccactattaaagaacgtggactccaacgtcaaagggcgaaaaaccgtctatcagggcgatggcccactacgtgaaccatcaccctaatcaagttttttggggtcgaggtgccgtaaagcactaaatcggaaccctaaagggagcccccgatttagagcttgacggggaaagccggcgaacgtggcgagaaaggaagggaagaaagcgaaaggagcgggcgctagggcgctggcaagtgtagcggtcacgctgcgcgtaaccaccacacccgccgcgcttaatgcgccgctacagggcgcgt

SEQ ID NO: 32 - DNA, 5550 bp, synthetic construct
  source 1..5550: mol_type = other DNA
acatgtgagcaaaaggccagcaaaaggccaggaaccgtaaaaaggccgcgttgctggcgtttttccataggctccgcccccctgacgagcatcacaaaaatcgacgctcaagtcagaggtggcgaaacccgacaggactataaagataccaggcgtttccccctggaagctccctcgtgcgctctcctgttccgaccctgccgcttaccggatacctgtccgcctttctcccttcgggaagcgtggcgctttctcatagctcacgctgtaggtatctcagttcggtgtaggtcgttcgctccaagctgggctgtgtgcacgaaccccccgttcagcccgaccgctgcgccttatccggtaactatcgtcttgagtccaacccggtaagacacgacttatcgccactggcagcagccactggtaacaggattagcagagcgaggtatgtaggcggtgctacagagttcttgaagtggtggcctaactacggctacactagaaggacagtatttggtatctgcgctctgctgaagccagttaccttcggaaaaagagttggtagctcttgatccggcaaacaaaccaccgctggtagcggtggtttttttgtttgcaagcagcagattacgcgcagaaaaaaaggatctcaagaagatcctttgatcttttctacggggtctgacgctcagtggaacgaaaactcacgttaagggattttggtcatgagattatcaaaaaggatcttcacctagatccttttaaattaaaaatgaagttttaaatcaatctaaagtatatatgagtaaacttggtctgacagttaccaatgcttaatcagtgaggcacctatctcagcgatctgtctatttcgttcatccatagttgcctgactccccgtcgtgtagataactacgatacgggagggcttaccatctggccccagtgctgcaatgataccgcgagacccacgctcaccggctccagatttatcagcaataaaccagccagccggaagggccgagcgcagaagtggtcctgcaactttatccgcctccatccagtctattaattgttgccgggaagctagagtaagtagttcgccagttaatagtttgcgcaacgttgttgccattgctacaggcatcgtggtgtcacgctcgtcgtttggtatggcttcattcagctccggttcccaacgatcaaggcgagttacatgatcccccatgttgtgcaaaaaagcggttagctccttcggtcctccgatcgttgtcagaagtaagttggccgcagtgttatcactcatggttatggcagcactgcataattctcttactgtcatgccatccgtaagatgcttttctgtgactggtgagtactcaaccaagtcattctgagaatagtgtatgcggcgaccgagttgctcttgcccggcgtcaatacgggataataccgcgccacatagcagaactttaaaagtgctcatcattggaaaacgttcttcggggcgaaaactctcaaggatcttaccgctgttgagatccagttcgatgtaacccactcgtgcacccaactgatcttcagcatcttttactttcaccagcgtttctgggtgagcaaaaacaggaaggcaaaatgccgcaaaaaagggaataagggcgacacggaaatgttgaatactcatactcttcctttttcaatattattgaagcatttatcagggttattgtctcatgagcggatacatatttgaatgtatttagaaaaataaacaaataggggttccgcgcacatttccccgaaaagtgccacctgacgtctaagaaaccattattatcatgacattaacctataaaaataggcgtatcacgaggccctttcgtctcgcgcgtttcggtgatgacggtgaaaacctctgacacatgcagctcccggagacggtcacagcttgtctgtaagcggatgccgggagcagacaagcccgtcagggcgcgtcagcgggtgttggcgggtgtcggggctggcttaactatgcggcatcagagcagattgtactgagagtgcaccataaaattgtaaacgttaatattttgttaaaattcgcgttaaatttttgttaaatcagctcattttttaaccaataggccgaaatcggcaaaatcccttataaatcaaaagaatagcccgagatagggttgagtgttgttccagtttggaacaagagtccactattaaagaacgtggactccaacgtcaaagggcgaaaaaccgtctatcagggcgatggcccactacgtgaaccatcacccaaatcaagttttttggggtcgaggtgccgtaaagcactaaatcggaaccctaaagggagcccccgatttagagcttgacggggaaagccggcgaacgtggcgagaaaggaagggaagaaagcgaaaggagcgggcgctagggcgctggcaagtgtagcggtcacgctgcgcgtaaccaccacacccgccgcgcttaatgcgccgctacagggcgcgtactatggttgctttgacgtatgcggtgtgaaataccgcacagatgcgtaaggagaaaataccgcatcaggcgcccctgcaggcagctgcgcgctcgctcgctcactgaggccgcccgggcaaagcccgggcgtcgggcgacctttggtcgcccggcctcagtgagcgagcgagcgcgcagagagggagtggccaactccatcactaggggttcctacgcgtcgttacataacttacggtaaatggcccgcctggctgaccgcccaacgacccccgcccattgacgtcaataatgacgtatgttcccatagtaacgccaatagggactttccattgacgtcaatgggtggagtatttacggtaaactgcccacttggcagtacatcaagtgtatcatatgccaagtacgccccctattgacgtcaatgacggtaaatggcccgcctggcattatgcccagtacatgaccttatgggactttcctacttggcagtacatctacgtattagtcatcgctattaccatggtcgaggtgagccccacgttctgcttcactctccccatctcccccccctccccacccccaattttgtatttatttattttttaattattttgtgcagcgatgggggcggggggggggggggggcgcgcgccaggcggggcggggcggggcgaggggcggggcggggcgaggcggagaggtgcggcggcagccaatcagagcggcgcgctccgaaagtttccttttatggcgaggcggcggcggcggcggccctataaaaagcgaagcgcgcggcgggcgggagtcgctgcgacgctgccttcgccccgtgccccgctccgccgccgcctcgcgccgcccgccccggctctgactgaccgcgttactcccacaggtgagcgggcgggacggcccttctcctccgggctgtaattagctgagcaagaggtaagggtttaagggatggttggttggtggggtattaatgtttaattacctggagcacctgcctgaaatcactttttttcaggttggaccggtgccaccatggccgatgctaagaacattaagaagggccctgctcccttctaccctctggaggatggcaccgctggcgagcagctgcacaaggccatgaagaggtatgccctggtgcctggcaccattgccttcaccgatgcccacattgaggtggacatcacctatgccgagtacttcgagatgtctgtgcgcctggccgaggccatgaagaggtacggcctgaacaccaaccaccgcatcgtggtgtgctctgagaactctctgcagttcttcatgccagtgctgggcgccctgttcatcggagtggccgtggcccctgctaacgacatttacaacgagcgcgagctgctgaacagcatgggcatttctcagcctaccgtggtgttcgtgtctaagaagggcctgcagaagatcctgaacgtgcagaagaagctgcctatcatccagaagatcatcatcatggactctaagaccgactaccagggcttccagagcatgtacacattcgtgacatctcatctgcctcctggcttcaacgagtacgacttcgtgccagagtctttcgacagggacaaaaccattgccctgatcatgaacagctctgggtctaccggcctgcctaagggcgtggccctgcctcatcgcaccgcctgtgtgcgcttctctcacgcccgcgaccctattttcggcaaccagatcatccccgacaccgctattctgagcgtggtgccattccaccacggcttcggcatgttcaccaccctgggctacctgatttgcggctttcgggtggtgctgatgtaccgcttcgaggaggagctgttcctgcgcagcctgcaagactacaaaattcagtctgccctgctggtgccaaccctgttcagcttcttcgctaagagcaccctgatcgacaagtacgacctgtctaacctgcacgagattgcctctggcggcgccccactgtctaaggaggtgggcgaagccgtggccaagcgctttcatctgccaggcatccgccagggctacggcctgaccgagacaaccagcgccattctgattaccccagagggcgacgacaagcctggcgccgtgggcaaggtggtgccattcttcgaggccaaggtggtggacctggacaccggcaagaccctgggagtgaaccagcgcggcgagctgtgtgtgcgcggccctatgattatgtccggctacgtgaataaccctgaggccacaaacgccctgatcgacaaggacggctggctgcactctggcgacattgcctactgggacgaggacgagcacttcttcatcgtggaccgcctgaagtctctgatcaagtacaagggctaccaggtggccccagccgagctggagtctatcctgctgcagcaccctaacattttcgacgccggagtggccggcctgcccgacgacgatgccggcgagctgcctgccgccgtcgtcgtgctggaacacggcaagaccatgaccgagaaggagatcgtggactatgtggccagccaggtgacaaccgccaagaagctgcgcggcggagtggtgttcgtggacgaggtgcccaagggcctgaccggcaagctggacgcccgcaagatccgcgagatcctgatcaaggctaagaaaggcggcaagatcgccgtgtaagtcgacgtttatttgtgaaatttgtgatgctattgctttatttgtaaccatctagctttatttgtgaaatttgtgatgctattgctttatttgtaaccattataagctgcaataaacaagttaacaacaacaattgcattcattttatgtttcaggttcagggggagatgtgggaggttttttaaagtttaaacaggaacccctagtgatggagttggccactccctctctgcgcgctcgctcgctcactgaggccgggcgaccaaaggtcgcccgacgcccgggcggcctcagtgagcgagcgagcgcgcagctgcctgcagg

SEQ ID NO: 33 - DNA, 6004 bp, synthetic construct
  source 1..6004: mol_type = other DNA
acatgtgagcaaaaggccagcaaaaggccaggaaccgtaaaaaggccgcgttgctggcgtttttccataggctccgcccccctgacgagcatcacaaaaatcgacgctcaagtcagaggtggcgaaacccgacaggactataaagataccaggcgtttccccctggaagctccctcgtgcgctctcctgttccgaccctgccgcttaccggatacctgtccgcctttctcccttcgggaagcgtggcgctttctcatagctcacgctgtaggtatctcagttcggtgtaggtcgttcgctccaagctgggctgtgtgcacgaaccccccgttcagcccgaccgctgcgccttatccggtaactatcgtcttgagtccaacccggtaagacacgacttatcgccactggcagcagccactggtaacaggattagcagagcgaggtatgtaggcggtgctacagagttcttgaagtggtggcctaactacggctacactagaaggacagtatttggtatctgcgctctgctgaagccagttaccttcggaaaaagagttggtagctcttgatccggcaaacaaaccaccgctggtagcggtggtttttttgtttgcaagcagcagattacgcgcagaaaaaaaggatctcaagaagatcctttgatcttttctacggggtctgacgctcagtggaacgaaaactcacgttaagggattttggtcatgagattatcaaaaaggatcttcacctagatccttttaaattaaaaatgaagttttaaatcaatctaaagtatatatgagtaaacttggtctgacagttaccaatgcttaatcagtgaggcacctatctcagcgatctgtctatttcgttcatccatagttgcctgactccccgtcgtgtagataactacgatacgggagggcttaccatctggccccagtgctgcaatgataccgcgagacccacgctcaccggctccagatttatcagcaataaaccagccagccggaagggccgagcgcagaagtggtcctgcaactttatccgcctccatccagtctattaattgttgccgggaagctagagtaagtagttcgccagttaatagtttgcgcaacgttgttgccattgctacaggcatcgtggtgtcacgctcgtcgtttggtatggcttcattcagctccggttcccaacgatcaaggcgagttacatgatcccccatgttgtgcaaaaaagcggttagctccttcggtcctccgatcgttgtcagaagtaagttggccgcagtgttatcactcatggttatggcagcactgcataattctcttactgtcatgccatccgtaagatgcttttctgtgactggtgagtactcaaccaagtcattctgagaatagtgtatgcggcgaccgagttgctcttgcccggcgtcaatacgggataataccgcgccacatagcagaactttaaaagtgctcatcattggaaaacgttcttcggggcgaaaactctcaaggatcttaccgctgttgagatccagttcgatgtaacccactcgtgcacccaactgatcttcagcatcttttactttcaccagcgtttctgggtgagcaaaaacaggaaggcaaaatgccgcaaaaaagggaataagggcgacacggaaatgttgaatactcatactcttcctttttcaatattattgaagcatttatcagggttattgtctcatgagcggatacatatttgaatgtatttagaaaaataaacaaataggggttccgcgcacatttccccgaaaagtgccacctgacgtctaagaaaccattattatcatgacattaacctataaaaataggcgtatcacgaggccctttcgtctcgcgcgtttcggtgatgacggtgaaaacctctgacacatgcagctcccggagacggtcacagcttgtctgtaagcggatgccgggagcagacaagcccgtcagggcgcgtcagcgggtgttggcgggtgtcggggctggcttaactatgcggcatcagagcagattgtactgagagtgcaccataaaattgtaaacgttaatattttgttaaaattcgcgttaaatttttgttaaatcagctcattttttaaccaataggccgaaatcggcaaaatcccttataaatcaaaagaatagcccgagatagggttgagtgttgttccagtttggaacaagagtccactattaaagaacgtggactccaacgtcaaagggcgaaaaaccgtctatcagggcgatggcccactacgtgaaccatcacccaaatcaagttttttggggtcgaggtgccgtaaagcactaaatcggaaccctaaagggagcccccgatttagagcttgacggggaaagccggcgaacgtggcgagaaaggaagggaagaaagcgaaaggagcgggcgctagggcgctggcaagtgtagcggtcacgctgcgcgtaaccaccacacccgccgcgcttaatgcgccgctacagggcgcgtactatggttgctttgacgtatgcggtgtgaaataccgcacagatgcgtaaggagaaaataccgcatcaggcgcccctgcaggcagctgcgcgctcgctcgctcactgaggccgcccgggcaaagcccgggcgtcgggcgacctttggtcgcccggcctcagtgagcgagcgagcgcgcagagagggagtggccaactccatcactaggggttcctacgcgtccattgacgtcaataatgacgtatgttcccatagtaacgccaatagggactttccattgacgtcaatgggtggagtatttacggtaaactgcccacttggcagtacatcaagtgtatcatatgccaagtacgccccctattgacgtcaatgacggtaaatggcccgcctggcattatgcccagtacatgaccttatgggactttcctacttggcagtacatctacgtattagtcatcgctattaccatggtcgaggtgagccccacgttctgcttcactctccccatctcccccccctccccacccccaattttgtatttatttattttttaattattttgtgcagcgatgggggcgggggggggggggggcgcgcgccaggcggggcggggcggggcgaggggcggggcggggcgaggcggagaggtgcggcggcagccaatcagagcggcgcgctccgaaagtttccttttatggcgaggcggcggcggcggcggccctataaaaagcgaagcgcgcggcgggcgggagtcgctgcgcgctgccttcgccccgtgccccgctccgccgccgcctcgcgccgcccgccccggctctgactgaccgcgttactcccacaggtgagcgggcgggacggcccttctcctccgggctgtaattagcgcttggtttaatgacggcttgtttcttttctgtggctgcgtgaaagccttgaggggctccgggagggccctttgtgcggggggagcggctcggggctgtccgcggggggacggctgccttcgggggggacggggcagggcggggttcggcttctggcgtgtgaccggcggctctagagcctctgctaaccatgttcatgccttcttctttttcctacagctcctgggcaacgtacacccaagctgtctagagccgccaccaccggtgccaccatgcagcgggtaaatatgatcatggccgagagtcccggactcatcactatatgcctcttgggttacttgcttagcgcagaatgtacagtgtttctggaccatgagaatgccaacaaaatactgaatcggcccaaaaggtacaacagtggtaagctggaagagtttgtccaagggaatctcgagcgggaatgcatggaagaaaaatgcagcttcgaagaggcaagggaggtatttgagaataccgaacgcactactgagttttggaaacaatacgttgacggagaccaatgtgagtctaatccgtgccttaatggaggttcatgtaaagacgatataaacagttacgaatgttggtgccctttcggctttgagggtaaaaactgtgagttggatgtcacctgcaacataaaaaacggacgatgtgaacaattttgcaagaactctgctgataacaaagtagtgtgttcatgtactgaagggtatcgcttggcggaaaaccaaaagagttgcgaaccagcggttccatttccttgcggcagggtctcagtttcccaaacctctaagttgacaagggccgagacggtgtttccggatgtagactatgtgaatagcacggaggcagagactatactcgacaatattacccaaagcacacagtcatttaatgatttcacccgagtggtaggaggggaagacgctaaaccaggacaattcccttggcaggtggttttgaacggcaaggtagatgctttttgtgggggctcaatcgttaacgagaaatggatagtaacggccgcgcattgtgtagaaacgggtgtgaagatcacagtggtagctggtgaacacaacatcgaagagacggagcacacagaacaaaagaggaatgttatccgcattatccctcatcataactacaatgctgctataaacaagtataatcacgacatagcacttcttgaactggacgaacctcttgtcttgaattcctatgtgacacccatctgtatcgctgataaagaatatacaaacatcttccttaaatttggtagtggttacgtatcaggctggggtcgggtcttccacaaaggcagaagtgcattggtattgcagtatcttagagtacccttggtggatagagcgacttgtcttctgagtacgaaatttaccatttacaataatatgttttgcgctggcttccatgagggtggacgggacagttgccaaggagattcaggcggacctcacgtaacggaagtggagggcacgtcattcctgacgggcattattagctggggtgaagagtgtgcaatgaagggaaagtatgggatctatacgaaggtctccaggtatgtgaattggataaaggagaagaccaagctcacgtaggtcacgcgtgacaatcaacctctggattacaaaatttgtgaaagattgactggtattcttaactatgttgctccttttacgctatgtggatacgctgctttaatgcctttgtatcatgctattgcttcccgtatggctttcattttctcctccttgtataaatcctggttgctgtctctttatgaggagttgtggcccgttgtcaggcaacgtggcgtggtgtgcactgtgtttgctgacgcaacccccactggttggggcattgccaccacctgtcagctcctttccgggactttcgctttccccctccctattgccacggcggaactcatcgccgcctgccttgcccgctgctggacaggggctcggctgttgggcactgacaattccgtggtgttgtcggggaagctgacgtcctttccatggctgctcgcctgtgttgccacctggattctgcgcgggacgtccttctgctacgtcccttcggccctcaatccagcggaccttccttcccgcggcctgctgccggctctgcggcctcttccgcgtcttcgccttcgccctcagacgagtcggatctccctttgggccgcctccccgcctggtcgacgtttatttgtgaaatttgtgatgctattgctttatttgtaaccatctagctttatttgtgaaatttgtgatgctattgctttatttgtaaccattataagctgcaataaacaagttaacaacaacaattgcattcattttatgtttcaggttcagggggagatgtgggaggttttttaaagtttaaacaggaacccctagtgatggagttggccactccctctctgcgcgctcgctcgctcactgaggccgggcgaccaaaggtcgcccgacgcccgggctttgcccgggcggcctcagtgagcgagcgagcgcgcagctgcctgcagg

SEQ ID NO: 34 - DNA, 11635 bp, synthetic construct; identical to SEQ ID NO: 10
  source 1..11635: mol_type = other DNA

SEQ ID NO: 35 - DNA, 25 bp, synthetic construct
  source 1..25: mol_type = other DNA
actttccattgacgtcaatgggtgg

SEQ ID NO: 36 - DNA, 29 bp, synthetic construct
  source 1..29: mol_type = other DNA
caagtgtatcatatgccaagtacgccccc

SEQ ID NO: 37 - DNA, 23 bp, synthetic construct
  source 1..23: mol_type = other DNA
aggtcatgtactgggcataatgc